European Patent Application EP 4 589 022 A1, published July 23, 2025. Title: COMPOSITIONS AND METHODS RELATING TO COLORECTAL CANCER. Applicant: Royal College of Surgeons in Ireland. The sequence listing filed with the application follows.

SEQUENCE LISTING (378 sequences)

SEQ ID NO: 1 - DNA, 500 bp, Homo sapiens
  source 1..500: mol_type = genomic DNA
gaaaaggtcattatgaaagccacctttcgtgtgagaggcgaacctgctgaccccactctagctaaacgacccgagcaccgccccttgaggacaaacccacgaaaatgttaggcgccgccttgggcaactgcgtattgctgcctgtgacagatgaaattcgactgcatctggacattcccgcggccccaggaaagtgctagcaaaaggccccggaaagcacctgcgatccctcaggtaagaagactgctgatcgcaataggcccggtctgagggttccccgcttgctcccgaaatgaagacactggagacccataaccgggctacaggatccggattcttcccgcggggtatccagttccagaactaagcgcccatgtgcgggattcgcctggctaacactctccggctcgcagaagcggcagcagccggcgggttttgagcttccgagtcccgggtgcgcaagagtgtggacgccacccctccagggctgccaagcctcc

SEQ ID NO: 2 - DNA, 500 bp, Homo sapiens
  source 1..500: mol_type = genomic DNA
attaaaattaaaaatttttaaaaagcctggcagtgaggcgctccagactcggcctgctgctgcgtgtcccttaaacacaccggcacatgcaactagtgtggccaagaccctcggcttgcgctgacccctctgttcagaacgtgcccacacatgcccatgccctctatcctgctgaaatccaacccccccttcaaaggccactgcagggagccttcccagggcccaaccggattcagtgtctacctgttctgtcctgtacaaagcgccccttttgcccttttcgtgtgtacttagagaattctgattttgactgaatcacctgtgtacttgttttctctcagcctcacccccacatggtgagctcaccggtcttactcatttctgcatgaggtaagggtctcgcccacaccaggtgccaaccagtgcttacggctaccacatggcaacaggggtcactggaggagtgcttaggagcaagggagtccttctcaccccgtgaa

SEQ ID NO: 3 - DNA, 500 bp, Homo sapiens
  source 1..500: mol_type = genomic DNA
atcacaccactgactatgctacgaaataatcacctctcctctggatcccaagagtggaaccgagacaacgggtcggaaaagagcttcagagagctacaaatccctgaggagtgacagcaggaaactgcggctcccaggacccagtgagggagttgagcaaaccccccagcgggcagagacggagacaggcaggcagacgaagaagacaaagagtcagtcagatggaaaagccagggagaaaaacagagacagcagcagagccgcgggtcactagggtcagctcctgaaggcctgtccttaatcaggtgtctctgtctcaggaactgaggctgcgactgcgcccatcaaatggccatatacctgagactggtgataatcgtattcatttgccactaacttgctgcgtaaccttgggcaactccctcccccacggcagggcaggagagttgtacggaatggcccctagagtccgatcccaatcccactctcacattctccag

SEQ ID NO: 4 - DNA, 500 bp, Homo sapiens
  source 1..500: mol_type = genomic DNA
ttaaatttttcattaaaatatgtaaaataaaatttaaaactaggaaattttataggaacagagattaatatcaggaatctgagaactacagctacttaaaactaactataggcctagtataaaataaaatcaaatgaaccatgttttataaacagattcaggctgtgttattcactttgcatgtggttcactaaaatgacaacacaacaatttgaactagccacaaagatgttcacactaatcagttcttttaattatttagatgctttcctgtctctaagctttcactgctattatttctactatttcctataaaaccctctgactcaagctccaaagaatcttaccaatgtgtaaagagccacctcaaataccactttccactaggaggcatttcctgatgcctccttccggcaacctttgttcccccaaagttatggttatttgggtacttatcttccatcaaatcataaatttgaaaaagagggaactaagttgta

SEQ ID NO: 5 - DNA, 500 bp, Homo sapiens
  source 1..500: mol_type = genomic DNA
atggcctgcagttgaaaaattattgaatagaagcaggcaaggaactcaatagccagcggactggatacatcgtcctcatgcacattgctgctgcttggataatggcggaactaaggggagtgaggactaacatgatgatgctaaaaccttcaaaaaatgtgtgtgtgtgtttgtgttgaaaatgggtgttgtagacatttggtagaagacagcaacaagggggaatagaagctgctttacccagacgatgtcaggttccaaagcaatgttttaatgtgaaggtggaagatttgggtttggagaagcaccaaggagtaagaaaaattctttaatctctactcttttcctctaaccctgggctctgtggagcatgggagaatatacagtctctacctgaaaggcataaaaaagagaactcagtttaaataaaggcaaggaagtgagagctattgtttagacaagagtgtgagtgtgttggagtaatttggtgacaataaaga

SEQ ID NO: 6 - DNA, 500 bp, Homo sapiens
  source 1..500: mol_type = genomic DNA
gtagatgctaaatacttgttgaaataaatataaatttgcctcttttgaatttattataccttgaattaattcaaaattatttttgtaaaatattctctaataacatgaattgaaaatgaggtgatgaaagctgtcatcggactcatttcctgggcattgtagtccaacagcaggattatgcgtttttctttgtactgcttccaaaacattgtagaattatccagatcaaggattttttcttggactttggtcatcctttactttcccaaatctaatctttaggtatgtgaatgatacctgcaaagcttaacagatctttgtgaagtagaagcctagataataagtgctttggggaaacatgatgggtttttttctttcaaaaatttttttttatcttctactatcataaaacagatgtggcatttaagaattccttagattcaagcttttaggctttgtaaattaattattattttatccacttgattaatataacaact

SEQ ID NO: 7 - DNA, 500 bp, Homo sapiens
  source 1..500: mol_type = genomic DNA
tgtttaagatgtattaggcacacttctgtgccttttgggggtttaagggaggactctttaaagcgaatgtatgaccacatttgatcaattcatggggagagtggaccatacacatgatggcttcagatatattcttaaatgagatagtacagtataatgcaatctggtctagtgcaagatttggcaatctttcagaagagaggagtgataaattgctgagtactggccttgggggaaacaaggagtttaactagagaaagcaagaggcacaaagaaggtctctttgctaagaaacacctcgctgatttgagtttcatttgcattaaacattctccttgtaaaatacaaatattcctcgaggaggagttactttgatcagctcaatttctggcttgatatggatgagtcggaaactgagaggagttttgctataggactggtggagtgatgggaggaaagatcatttggaacatgagtcactttaaaggcagccagatctg

SEQ ID NO: 8 - DNA, 500 bp, Homo sapiens
  source 1..500: mol_type = genomic DNA
ttaatacttgaaccctgtatactcaatactgtaactcaaattgtttcttctcctctagaagcaaccaaattccaaatgggtgttataaactggatcacgcgtggacacgccctatttccaagaacccttagacagaccccaggaagagccctagctgctgttccccattcaacgtccattttcagcaggaagtagccagaaaaagtcgtcacccaataaccccctaacagcaattaggttgtctccatggggggctggggggaatgtgataggagttactaagaaattattttaggcagatagagaggaaaagcggtccttggaaagttttcatttcttttaaagcagctccagaaaagtttcttgtcaagaaggaaagcccaggcccttagagccaagcaggcaaccttaggtatgcagataccggccattagaaattgggtctacccaacatgatgattcccatggttgtcctcttgcccttgcgctgacatgtgcct

SEQ ID NO: 9 - DNA, 500 bp, Homo sapiens
  source 1..500: mol_type = genomic DNA
cactgtagatatgagaaaatgctatccctgactcacgaaacttatccaaaaagtagagaacaaggctcagccattcaaataaagcctcagttgaatcaaataaaaataagttttaaatatttaatgtgaaagtcttcgagtatgttaagaatggcttaactcagggatagaaattttactgattgaaagaaaatttcaacaaaataccaatctttgaatctaatttgacacccgaaactaggcaatcaaacattagcactattttttcttctatagtttataataaaatttctcatgagaaaaaaagacatttttcttccaagcctgaaaatggatggagaatttttaatatttattgttgctgagaacagtaaatagactatccactttcacaaatgaaggctggctttgagccacagaacatatctgttatatcactctttgacaccatatattaacagaaataataattttcccgcattgagtttcctatttaccat

SEQ ID NO: 10 - DNA, 500 bp, Homo sapiens
  source 1..500: mol_type = genomic DNA
cgtccccagccttttggaactgagctttcccaaaagacaactggggcctcacgggagccttacagggcttcttggaggtcagattgcctgagtattgaggttatgaacctaccgcttatatatatgagtttttagatagcagaaacttttcttcttgaaagattattgtttgaagcctttcaaatatgttcttcctgtttatggaaaaaataccatattaaccaagataccaatcactggatgctaggaataatgggacgatcaggactttgggattgtggggtgtaaaacttgctctacaatgatgtgaccttgttaaaaagcagaatgtttctgcagttgtgtgctggcttttcattgagcttagaataaagccagtctgatcctccttaacaaaacaccacgtggtccggcacctgccaccgtgactcatctcctcccacccttgccccggcctctgtgctcctgcactgtgggcttcctgctcatcttcagaaaga

SEQ ID NO: 11 - DNA, 500 bp, Homo sapiens
  source 1..500: mol_type = genomic DNA
aaaggaataaaagaatggctactccatagccagagcagccctgagggctgcttgactgagtatacttacagttatttcttgattatatactaaataaggggtggattattcatgagtgtttcagaaaggagcaggcaattcccagaactgaatgttcctcccctttttagaccatatagggtaacttccagacattagatgtcatttgtaaactatcatggggctggtgagagtgtcttttagcatgataatgcattataattagcgtataatgagcagtgaggacgaccagaggtcacttttgttgccatcttggtttcagttttggctggcttctttactccgtcctgttttgtcagcgggatctttgtgacctttaccttgtgctgaccttccttgttacgctgtgactaagaatgcctaacctcctgggaatgcagcccagcaggtctcagccttattttactcagtccccattcaactctggtttgaacacctct

SEQ ID NO: 12 - DNA, 500 bp, Homo sapiens
  source 1..500: mol_type = genomic DNA
catcagattgacatggatggtgagtgaaatacaggatgaagccaaatagtgtgtgtgtatgtgtgtgttggtgagtgtgtgttgaggtcaggttgaagagttgcaaagtaaaagtcagtacatatgatttttgttattgtggcaagttattgctctaactgatgtttcactgagtcatctaaatgtgcatagagtaaccgccttaaatacagaatgtattccagtaaaagtgctatagcaaagctccttggcttttttcaaataaggtgttttcaagctgacatgctgttcattgggtttgatggtgcacacaggagatctgtgtgttcccaaatacaccaaccttcttaaccatcactagactgaggctagttcctatgggaaatataaacttctttgttttcaaaaaaacatatgggccaaattagaaagtaaataaatgaatacctctcaagaatccatgataacacttgccgagcagtgggtcaggccagatttaa

SEQ ID NO: 13 - DNA, 500 bp, Homo sapiens
  source 1..500: mol_type = genomic DNA
agtagagaatctgctttggtttcctgactgggttgccttgtttttcagccacagggcaagaaacatgccacagcaatgaaataaaggtgacatgtcataatgagggaaagggagttattccacaggctgagtcaccgctctcctgcaggtacagaatgatacagcctacagaaattcagagcagactgtcagactgtgggattgagtaacaaagagaaacaggtctacagatgacctagcatacgcttattattttgaaatttctgaattgtaaaaaatgagaatggtgaagtcttaggtagatctaagttcattcttgcaacaaaaatcagttccaagtttgcctggaagtgaggcatctaattcataaaatagtggctatagtgacagttatatatttgagggaaacttatctataacttccaactaacatacatcttggtggagtctgagttctacatttttctgctttcttcctcatcaattgtcatggttgacat

SEQ ID NO: 14 - DNA, 500 bp, Homo sapiens
  source 1..500: mol_type = genomic DNA
acacacacataaaaacaaaccactctgaagtgtccatattttagcataaagttaggaattatgcgagtgctgggtgtatcacggtcaattctgtgagcctcgtcacagtttatagccgaagtcagaggcttcaaaatcagacacacattgacctggaatgctttattctgcagtgctcattcttgattctcagaagtatcgctcctgtgaaaaacttatcaccattagggagctgtcatttccctggtaaaattaaacagcaatttcattcacctttgcttctttttggatgaaggctggcaatggtttaaggaacaaataaatgaatgaataaatgagtggagttccctcctcctgactcagaaaggtgctatttcccctcacgcaggagatacaacttccatgcaagccagttctcctactacatagagcccttctgtttttaggaagttctgattcatggattggagaattgaactaaattagtatactgtacagca

SEQ ID NO: 15 - DNA, 500 bp, Homo sapiens
  source 1..500: mol_type = genomic DNA
ttaagaagacacaaggcggctgggcgtggtggctcacgcttgtaatcccagcactttgggaggccgaggcgggcggatcacgaggtcaggagatcgagaccatcctggctaacacggtgaaagcccgtctctactaaaaatacaaaaaaattagccgggcaaggtggcgggcgcctgtagtcccagctactcgggaggctgaggcaggagaatggcgtgaacccgggaggcggagtttgcagtgagacgagatcacgccactgcactccagcctgggcgacagagtgagacgctgtttcagaagaaagacacaaggcaagttggttgtcgatacctggaaaaattgaagttcttatgttttcataccactgaaaatgcttgtatgtaaatatcctctgggacaggaaattgacttaagtgagtattcttaaacatctctaagtgaggaaaggaaatattttttaaagcataattagtgttttaagttgaaaaataacatc

SEQ ID NO: 16 - DNA, 500 bp, Homo sapiens
  source 1..500: mol_type = genomic DNA
atgagactttgtagtgtcatgactgaccgtaaatctcactggcagtagcacagcatatgaaacaccttctgctctagtcattactttatgttcatcacaaacaaatcagaacaaattctgaatgcgaatctcctttcaagttagctgactcaggctgtcggaactcatgtaaaagcgaaccaaatatgacaggaggtgaaagctggccgtagaactggaaacggcagaacgtcattgaagtctgcctaagaactagtcagcatcccacctgcttgctcacagtcacactcaacatctctgtggaatttttagtgctcttttttgtattagtcttttagtcgttaccctagtgactctgatatgcattcctaacttatcagtttactttgaattaacattagaccacttgatatataatgtaagaacttcttacagtgtaatttcatgtacagacttcacaatccttttgttgtagctaaagtttacttctacctagatta

SEQ ID NO: 17 - DNA, 500 bp, Homo sapiens
  source 1..500: mol_type = genomic DNA
gccaccgcacctggcctgtaaacagttttactggaacccagcgatgcccattcatttacgtataggctacggctccttttgtgctataactgcagcgttgagtagtcctgagcgaacatacggcccatgaagccaaacatatcgactatctggccttcttcgggaaagtctgccagcccttgccataaataaatgcagctatacacacatgcatacacagaaaacaaatctgaaattggatatacaccagagtgatgtgtggtcatctctgggtacttttggtctgcttcttagagcttatctgtatttttcagtttttctgtactgaatctgttgacttggcaagcaggcctcctgtaggtcatcatactttgatcagattttattagggctgactgccagaagtcaggagtgtacagggaagacttcctggaggaggggtgcaggagcaggctgggagggtgagaagaacctgagtaagaaggggtggaggagcgggc

SEQ ID NO: 18 - DNA, 500 bp, Homo sapiens
  source 1..500: mol_type = genomic DNA
cctagactctggggaacgaacgcgtgctgagcctccccgccgctttggagacggggctagattttcgttgcctccggctctcgacaggtgcaaaacaatgaattccaagcctcggaagcaaagaagcttaggatccgacggtggccgcaagatctcatcatggatctgacccctgctcagcgcgcgccatttcgtcgttgccaaacgaaatcaagccccgcgtgcgctccaggggcgaaggactctggactcaccccgaccaccgggagagctggcccctacccacctcgggacctcacagcacgccctcaggccgtgtcgaaaggaaggacggcaaaggtcccttactgaaccttttaagagagcctgcgcctggcagttgtcgattgcggacccaggcccgcgcgccctcggacgcgctggcacgagcagcagaactagaggaaagcgagtgatccagcctgggcgctcccacctccgggaacgtctccgagaaggcg

SEQ ID NO: 19 - DNA, 500 bp, Homo sapiens
  source 1..500: mol_type = genomic DNA
gggtcctctttgttagattccatttccattttgctaaagtctatctttaggtgattttccacatagagtgtgtagcactaaacattctgagttctgacatattccttactctgcctttatattgtttggcagtatgtgtggatacgtatcaaattctgacaaagactctctctttgaccaaactttagacaggctcctctgagccttcttttcaactgaaggcaggccctaatctttgggtctgtcctcagcctgcattacccagttttagagcaaccttgctaagtcagtttagagagaatcccctcatccttgaaatctgatcgccaacgatatttgatcatgatcctcattcccctccattgatatctaagttctttgcctgcctctagcaagaatcccgttaggccggtttaccaagaacctccctacccttgatgtctcctcttaataaatttctatcccctgactcatccaatctacctgttggctatgaatcc

SEQ ID NO: 20 - DNA, 500 bp, Homo sapiens
  source 1..500: mol_type = genomic DNA
gaaaaaagttgatcggcctctgctttaagccccacgtcccctgagctagctgcccagcattctcaaagccttccaggcaaaaccacatcctccctaaataaccgaaaaggtatgcatcctattatggaatgttaaatgtaaatggctccttggccatgtgtgggtgtggggccaggatctggaccctggggaaactgacacccctgagaagatacacatttggtggtgagatgggcaataattcaactaagagaacattaatttggtaagattgggcacatgcaaagttcactgtcactctcagcagacacatttaagtcccagctcctccacttgtgtgaccttaaaaaagtcctttcctggctgggcatggtggctcacgcctgtaattccagcactttgggaggctgaggtgggcggatcacctgaggtcaggagttcaagaccagcctgaccaacatggtgaaaccccgtctctactaaaaatacgaaaaattagc

SEQ ID NO: 21 - DNA, 500 bp, Homo sapiens
  source 1..500: mol_type = genomic DNA
gaagcagggcctgcctcccagtcacctgctgtatctcaacagcttattaggaggttgtggatcagaataatactagtactagttctactaataagagctaatacctataagccattacatatcaaacactgttttgagcacttaatatgtttaactcagtttatcctcccatcagtcctataagattggtactattattaaccccactttgccaataaggcaactgaggcataaagagtgcaagcaacttgcccaaggtcagactaccagtaggtagtcaagactcaaatccagacagtccagttttggaatctatgcttttaactactatgctctactgattctcatcagaacagcgtctacctcagcttccctcactttgaaggtccagagtccacattctgggacttgggcacatgcagccaaagcctgttccatcagtcacccaacaaagtggaggaaaggcatgtgtcttgctcaggatcacaagatgaatcaga

SEQ ID NO: 22 - DNA, 500 bp, Homo sapiens
  source 1..500: mol_type = genomic DNA
ggcaccttcacagggcggcaggatgaagtgagtgcaagcaggggaaattccaggcgcttataaaaccatcagatctcatgagcactcactcactatcacgagaacagcatgagggaaaccgctcccatgatccaatgacctccacctggtcccgcccttgattgtggggattattacaattcaaggtgagatttggatggggacacagccaaaccacatcatacaatatgtaaccttttgtgtctggcttctttcacttagcataatgttttttagttcacccacattgtagcgtgcatcagtacttcactcctttttatgatgaattctgtgccacactgcagataggctacgtgctgtttgcctgtccatccactgatggacatttgggttgtttccaccttttggctgctgtgaacattgctgctgtgaacatacatgtacaggtgtctgtttcggtccctgtttttgatcctttgagggacatacctaggcatcaa

SEQ ID NO: 23 - DNA, 500 bp, Homo sapiens
  source 1..500: mol_type = genomic DNA
agtgacagacagagaaggaagaagacacggtcagagacccagatgcagggaacttgagagaggtgagccacacaggcctcttcagctaggatccctgcagctggcaatagtagaaaagaaggaagaggtggaggactgagaccactgtagaaagggtgtcaaaatcaggattagggtgggaagaacacaccagagctggggaagggttgtttggggttcccaagtctctcatcgccttcaccagtggagaagagatgaggctcaaggtgcaaagagtacacgcagtccctctgccagaggcaaggcaaccctctccttgttgagagactgtggaagtggagggaggtcaaacggagtgggccaccttcccaccattttatcaaatggtccaggcaaagtaaggttaggttggatggtataaagggagaaacctctgctgatactgggatgaaggtctctggctggttgcttcgtctacttaaatgtctctgagtttaatt

SEQ ID NO: 24 - DNA, 500 bp, Homo sapiens
  source 1..500: mol_type = genomic DNA
ttgtttattttcacttgaggaagggtgactgtgactgaaggaacatgcacccacacaagtgagcatgtgtgtgtgtgtgtgtgtgtgtgtgtgtgtgcgctgtcagtaaagcactttgtagctatgtgatctcatttacaatgaatatgtcactcccagatattagatcggaggtttacgtaaaagatttattaattggtttttcctctttagaggagaaaattaagtcagcaagaattatgtctgatggtggatagttggatgagatacttccacaactgctatttataggagaagcagcagacccttgtgtgtgtgtgtgtgtgtgtgtgtgtgtgtgtgtgtgtgtgtgtgtgaatttatctgagcatattgcttggtgtctgtgtgttggaggatccatatcaggaaaaggtagaaaaaagagggctggggaacaagagcgagatgtacccttataggggcttctagggatcttggagctccagacccatgactca

SEQ ID NO: 25 - DNA, 500 bp, Homo sapiens
  source 1..500: mol_type = genomic DNA
gaccccagtttctcagtgggccaagaagggtagacctgagccagagaagattgcggtctgaggaccgggagtcagagagaagccactgatgcccagctggccttgaaaaatacccagaaagggaattgctgcgggagctcccaaggctccagatgctgaaggcagagaagaagggagggtatttagagtttggggctcctttaggttgtctttgtggggaacctgttaggagctgggaagggcccatttgggatctggacttcaaggcaaaggatgagggagtttcaggatttgtatggtagaatcctcctggatgttttttaattcctcctgactggaagggcctaatgggtgactcctcccaaactatgggtgcatagggtgggtgttcagtttaaggaggctcactaggcatcctgggaggagaaacaggctatcccatctggaggggctcctgtaggttccgtctgtgcttgggtggagggaactgaggttctgct

SEQ ID NO: 26 - DNA, 500 bp, Homo sapiens
  source 1..500: mol_type = genomic DNA
gccctgcaggccccaacaatcagtgacaataataagaaaatattcagggcataccttcatctctctaaggtgagaaaaaaaagaaggtaggaaatcggcctggggttcagagagtgctgctgagagcgggcagtttaaagggaaagaaaattggcgaatttcactggtcaatttcacttcatttcgttcaatttcgttcaatttcattccttttcatccagcgccgggaggcccgaggccacaaggaaggggagggggtctttccgggcgaatttccctcatcttgtagatttactctctagggctgtgaagaacagccttgattctgaaactttgacgtacgtttttcagccgccgctaagagcagacattttattttattgaagggtatttggtttgggtgatcgaagcacatcggtgagactctccgcacttctctcttgcagcccaattaaagcggttaattcttttcaccgcttattcctccccatctttctttc

SEQ ID NO: 27 - DNA, 500 bp, Homo sapiens
  source 1..500: mol_type = genomic DNA
tttctcctggggctcctcggaccacccaggagccggagttgaggtgggggcggacacttcccctccatatccaatttgctcttgccacagcgggcgcgtcttcgtggttacaaagcgctttttccctgatgacttttttccccttttcaaaaacacttctttctccccccttcaactagcaaccctccccaggcccacccctcctccctctccgctccggtttatttaaacttcgcctcctccagcgccgccgcagcgcgcacttaatgaagttgaaggctcggtgagcccgggtgaagagggtttggaatctgttgaaaggggcgttttgtgacactgattggggcgggggcgggggcagtcgcggaccagacaatgaccgaccaggcgggttttcctgcgcacagggtcaggcgaataaaggcgccgacgctgtttaaacgaaggaccttgtaagagaaagggagaaaagattttgtgtgtggagcgtgcctcgtaag

SEQ ID NO: 28 - DNA, 500 bp, Homo sapiens
  source 1..500: mol_type = genomic DNA
gtttcaccgcgggaagcccgggcattggagatctgtgctcagttctctaggtgttggaaagttgcctcaggctgctttcatctctggggcatttctgtctacgcaggcagaaggatctttggaattgcagttgcatggatcttagttctggaaagggcgaatcattgggggaacaaaaaattcaaatccgtccttttgattcctaaaaatcactgcagacctgaaaagtgcatttcgagttatctgtgtagacactgccggtgtgtgtgtggtggcggagggtggggtaagggccgagggtacaggagtggactttattgttcacattaactcaccggtgcttacagaggaccctcgattcgcgaccccctcccccagcaggtgtctgtgcagttcggactcctgggcttagatgccccatcccgttcagatgcaaatgtgctgggttcgggttgagtgtgaggaatccacctccccacccccaccccggcccacgcctt

SEQ ID NO: 29 - DNA, 500 bp, Homo sapiens
  source 1..500: mol_type = genomic DNA
ccttccccgacgccccttctgggccttttgggttcctgtctcaactttgagttgcctatacatctttttgagataggtctcgcctcctcaacagtcatcatagtcaaagagggcaactagtgaggctattgcgtgaattagccttcgacccagactgcaggagcttgggggttctgaggacagcacggctctactttccactttggagtggaacctacctggcgggggtcacacagcagatagtttgtgcagctgggaagatgagccctggacccgaacggtatgaggatatgtatcctaaggccagctttggtcccagttcactgggtgccggctgccccagccagctatggtctgcagagcccgaaggcaggcaggaggatcgcagatcgaagatctgcaaggactgaggatcgttcctagtgtctgtttggaagcccgtgggtcttgcaatgcgagggcagacaaactacgaagcgggttccggattccgatgagcc

SEQ ID NO: 30 - DNA, 500 bp, Homo sapiens
  source 1..500: mol_type = genomic DNA
aggctaggtcagcgtagatgccttatctactcactctgttcctggaagtctgggctttgtgcattcccataaagggccccagaagagggtgggatctgagcccgtgatggaccatgctgtatgttggtgcagcccaaggggagggaaagctgtgactcagtgtttgtaaaatgttagcttgtggagtgagtaagaccagaccaaggctgactgttttgggaagtggtgagttgggttaattgaaattggagcccaaaagccaaggtcaattcctgccatggtggctctcacttcctagctgtgccctattaccatgtaatttaatctctccaaaccccagtttctttatctgtgaaatggctacattaacacccagcctactcaccccctagcaagatttagaagtgctggagggcacatattttcatatgggtgcatattgaatacatactatatgacacaaacttcatatctgttatttaatcgaattctcagaacag

SEQ ID NO: 31 - DNA, 500 bp, Homo sapiens
  source 1..500: mol_type = genomic DNA
ggacaaaacactttgcctcataggtgcatcctaggaagaatccatcctactaaagttgccatcaactggcagagcactcaactggcagtggtgtgacctgctgtctccctgctctgtgctggagtggagcctctgtgatctgcctctgccacaggcaaagttctcagggaaactagagaaactggactgacttgggggaaccatttatgacaccaggtaaaagaccatggaatccaggctcttcagggccatcgctgtaggggcctacttcctgtcttagttcaggttctagaagcagagcctaagacagggattccggggcatgtgatttctccagggagcgcccttcaggaaaaacctccacgagcattagggaaggacgggccaagcaaggatggatcttgggtaaagccgagctgtgacctgaggcccaagggccgctggggcatttccacagggcagtcacaccgtccttcagagaagggggctggcctttgtgc

SEQ ID NO: 32 - DNA, 500 bp, Homo sapiens
  source 1..500: mol_type = genomic DNA
tttaaaagtcagttaaaaattccagactgccaactgtaacaataagcactatagcagacaccatgaaaaatacaaagaaaagagtaaataattccaggccctatcttcaaaaatctatatctaattggattctaaatacaagaatgtattcatctattcatttaatagatattaattcagctccacaacacgcaaaaactgctcaagggccttgggataaaacaatcaagacaagcttggttccagccatctgcagctaacagaacatattcagaataaaagtgctaagggcaaccagagtgacagtcaaggctatataaaggccctgtactgagtgaaaatcggaaaacttatggaccaagaggtgtaaatacacacaggtgaagagaggaaaattcctgtaggatgtcaataaaactggaattcagcagtacaatggtggactataagccttgcagggaaatcactcaacatataggaagtcctcaatgcaaatgtgt

SEQ ID NO: 33 - DNA, 500 bp, Homo sapiens
  source 1..500: mol_type = genomic DNA
agttctctggaggagaaactgtagagccgtgtggattcttgcctgggtttgtttagagatactacggacttcttgcctaggtttgtttggagaagagtcaagcagtacttgagtgatttgaatttttgttgagaaaaacaaagtgaaaaacattttttcgacatcagatatgttgttttagcctctgtggcagattttatttttctcttttactttttgtttttatccttttgtactatttttaaagaaaggaatgagaagaaattatccccggaccattcctcccggtgaaaaacatgaaatgtgactatccggaaatggagtgtgatcacaggggcacgtacggctgagtcatccaaaacgctgactgtcgtgtagggctccgtggttttggtggttttcttaacttctctgtgccctggttacttcatcaatgtgatggagataataatctcatcggatgttgtgatttactgagatcattcttgtaaacacttaga

SEQ ID NO: 34 - DNA, 500 bp, Homo sapiens
  source 1..500: mol_type = genomic DNA
cgagctggaaaagacagctggtgcgtggcgacgtccctcggaccctaaaaggcccatcggtttagcaacgagctgggatttctcgagctgcgttcggcggcgcccggaaaatcagtcctgctggatgcgcccgagcgggcgcgggagacgccgattccgcgccggcccgcccccgccagtttacaaagcaaactttccccagagaagttccgagatcgaaccacgcgcaaagtgcgccaatcaacacctaaacagacccaaactgtacaaacacggatcgatcagataatttcaaatattataattggctttaattaaacacactgcgttctaattaactctgaaattttagcatgctttgggacactggtgtctgatttgatattgtcagtccagatgtcctaataaaattcaatcctccactcaagacttcaatattcaccaagaacaaaatgcaaattaaatgtaaaacctaaagtattgccaaaggtataatcaag

SEQ ID NO: 35 - DNA, 500 bp, Homo sapiens
  source 1..500: mol_type = genomic DNA
tagttattaaataatgactagtatttgaaacagcactgttacattaagtaaaaaaaaattggcaagaaatgtcaacttagacatttaataagataatagttctgcttagaaaatgaggtgttagttctgcctttaacgtatcaacatattgtaggaaatactgaccttttattctgatcaccacgagtccattaaatttcaaaatgtgggacagccaatacataatatactactaagtaataaatctatgtcatccaaagggagctttgctgtctgagtccaaaaaaaaagaaaacagaagcataatggtaaggttactgaacactcaggtcttgaaataagtcattctgttatgagcatgagtcaccaaaactacttccttagtgataaaagttgcctaagtaacatcaatgcctccctatgctaagaaggatatgggcagtgtgttgggtttcagacccactagtcatagtcatttcctttacttaattgctaactgc

SEQ ID NO: 36 - DNA, 500 bp, Homo sapiens
  source 1..500: mol_type = genomic DNA
tgttccaccggctcaccaggtcctcccttcctggccaactctaacctcagctttgtgcgtgtcacccggccccgggataatcggatcctcccagacccgggaatccatcagaagcgctacccgtacttggcgccctgaaagttccccaagcgcagcggccgcgccctcgagtgcatccactccgcgagccacgggcggcgcctgcccacccgcggctcggctttgcgtgttgtaagccgactattctatcaccattgcaggataagctggcctttaaattttcaaagaacatttaggttattttcaacagttcatgcttttcatatctgtcttttcagactgcagatttccacaaggaaaaatgtatctttcctagacggcaaaaagcagatttattttcctttttaaaaagttgccttaaaacgcctatctcatagtacttggggattaaactgtttcccctaagagaaagttcaacggctaagctcaaacgttagtct

SEQ ID NO: 37 - DNA, 500 bp, Homo sapiens
  source 1..500: mol_type = genomic DNA
caactcaacaaaaaatccagtctcctgccactcagcccccctaggtcgggatcgtttggtttcggtgtcaggaggctccccgggctcagagtcgttctttgtattccgcagtccaacctggaaagcatatgctgcacctctgcgccggttaaaatcacccccagacagattcgagctgccgcctcttcgcctttcattctgtcgcctgcgtccccagcagccccgggtccccagttccctcccctccaccagaggaccctgcctctatccttcccccgcacaactaacgcaatagcctgaggggtttggtaaacagaagcggccccaggagggggtgggattcgccccgggtgtgacccaaaggcacctgcggcggcccaggccctgggcgaggcctgccggccttgtaaaggcctccgcgtctgtgcgcggcaaagcagccctaacggtttcaccgcagcccacgtctctccagtctgcaggcccggccttccctgtgc

SEQ ID NO: 38 - DNA, 500 bp, Homo sapiens
  source 1..500: mol_type = genomic DNA
ctaaaaatgtgaatctgtgtgtattggtgtaaagcaaccctgggaattattgacattttgaaaaacaagaaggggtgagacagtcctgccagttcctcctttttcagtctccatatgtataaataacatgcaaatagtcatataacgcagagaaactggaagtgtattgaatttgcaactttttttttttttttttttttttttttttttgcttgagggcttccatttagtgagcactcctcagtactcacagcagagtattgccagaggaactgtaaaaaattaagtttgctatcaggcaaccagcaattgactaggtatggcatgtatcagtgtatccaccaggcggtactgaggcttcatttctttgcttatttgaaaataaggtggaaaatggcacaacagcctgacctgatttgcaatgtgtcccttagagcttaggctagccattcagtcttttccttttctaggtaactaacagtggctggactatggctttg

SEQ ID NO: 39 - DNA, 500 bp, Homo sapiens
  source 1..500: mol_type = genomic DNA
aatatgggtcacagatgagtaagccttcctcaactggttctgcttcctgttttccatatataggggccccattttttccttttcaagtccacacagcattgcctccaatgggtgtgagcattccttaccagcattcagatgctgaacatttttaacagcctacgggaaacagtgttttaggcagctcttttcaaacactgagtttcttcagctgtggaagagaatgtccttcccaaataagaattaaaaaaaatgcccaatataagcaattgaatagcactggagttatttttaggaaccagggtcactcactacaggaaatgatcgtgttgccaatgcgttaaagctagtgactttaaaaaatattatttattttctcatttaactgcatctcgaggaaagttagcagttgcaattttaagttaggaacttctcaatttcaggccagattcattagggagtaggaaggatacctttcacttaaaaaaaggcatttgggc

SEQ ID NO: 40 - DNA, 500 bp, Homo sapiens
  source 1..500: mol_type = genomic DNA
ctgaacacagaataaatattgtgtgcccatcttttcactcccatatttgacaggtaaaagaaataacttgcaagttaaatatttcccccaatccacaaattgctttaatactgaaatttaatgccaatcttctggaaggtaaatactagtgccatctaatggacttagtcaagcacaaagagtttaaaaattttaagttttaaagaaaatctattctaaggaaagccaaaccctctacttgccttcatttgcttcccaagacaacgtccacacaagtgacccagaataatggagatggagacactttatcctgcggtttgccaggaattccactcattctaccaccacaaggttgctaatcatgaatgagctctcaagatgagtcagcctcaaacaactcaccagctgcgtggccctaggtaacttcttcactcctctgggctcagtagtgataggttttgttttgttttgttttgttttgttttttccccataaatttc

SEQ ID NO: 41 - DNA, 500 bp, Homo sapiens
  source 1..500: mol_type = genomic DNA
cttacatccttcagatattactttttacaagacttcaaacactaataaaatgatacacattagtaaaagagaaaaatccattatataacccttcagaatagactaaaggagcagagtccataaaagctgaatcatcccattgtgtaggtccctaccaaaaacacttgacttatcagctgagccaggaaacctcatcttcagtacacatgagatatcagtagctgtttcacaggttggtcatcaagggaggcatttaggtaaagattcgcattctgactttatcactcactaactggagaattgcagcaagttactcaagcccttaatacctctgttttctcagtattaggaatgcagagtaatgtctattacatagggcagttgtgaaatttgggcaagagagtgtgtgttaaatccagaggctgacacataattaagtattcaactcagtcagcgaatgtgtttactaagtgccaagtcacccactgaaatcaaacctg

SEQ ID NO: 42 - DNA, 500 bp, Homo sapiens
  source 1..500: mol_type = genomic DNA
cagagtttgattgatctgtcaccttgtggaagagcccactttacatgctaacagcttttgagttcttcaggaaggaacggcctgtgactggctgaatcagcactcagctcctgtttactaccaagtacagtaccatttatttaccttggagtaacccttcacccagcatcgcctcttgaaagcttccgaggagaggaaacgtacttcaatatgaagtcttatttctcaacagttctcctggtcgagtttaaaatttaaaaattatcttgccaagctttctgcactgtgatttatgcaagaatggtacaagaatgaaatggattgtcttggcaggctgagtcactgctacgatatcagggagtatcttcctgctgcagaggaaagggaacacgtcatgctctttgagtcacaaaccttctaatcatcacctgtctgaaaggggacctgttgtaactgactcagctgagattcgccaagcaggcacgctgagtgagtacaga

SEQ ID NO: 43 - DNA, 500 bp, Homo sapiens
  source 1..500: mol_type = genomic DNA
cacatattaacgtgtacaattataatgtgtcaatttacaaaaacaaattttcaaaaaagcaaagacctgtaaaaaatttcctttaatttgcacataagcacaggtacacattttgtgcaaatatgcactctgctgttgccctaccagctagtcctgggtccagtcctaaaatgtagccctgtttttcttatatggggctatatcattctagacatacaaaaaataggaaaatggccaacacaaagtccgattttaaaataatttaagtgtttgttctttttcacctctgctactaacatctatcttcttgtaatccctctgttacaccacaaaaatgtaatgccttcacactgccctttggcttttgaaatttttctcagtgcgagtccccttgggcttgcctaacctctaatgtcacatgttccacagttacatcactttttctcttttctgaaaagctccccacttctcatgtggatcataaataggggcttaggaaa

SEQ ID NO: 44 - DNA, 500 bp, Homo sapiens
  source 1..500: mol_type = genomic DNA
gagaagttggggagaaagtttaattctcctctttgcagttgtgttaaacagtaatcattacattagtgaataattattcttgattggcagttatgtttcaaatgtttgtgtccttgcacaccgactgagttcattgcactgagaagaaaagaatgctggttgaatctggcagtgttacttgtcttaattcttcttagtcttcccactgtcttaatagaatttatgagtcacaggacatagtatcctgaagatagtcacagaatgaaggaaaataatgtctgtctccctaggccactttctttgtgcatctgttgcatatatattttagaaaatgctctatacgtatttattgggtgccactcatttgaaaggaattgagccagatgatgagtcaggagttggcaaatacatagtaatgaacctcaaaaaagcgtttagaaaaatatgcggaaattttaaggagggaatgggattagtttttgaagacttgccaataaagt

SEQ ID NO: 45 - DNA, 500 bp, Homo sapiens
  source 1..500: mol_type = genomic DNA
tcttgaatgtcaagtttatatgtgtcccagtctcagaaagacagacacaccaggggcagaagccaagtgtcatgtgctgcggaaaaatgaatgctttttcagaacactgaatttgcaggctatgcctcagtgaagccagcagttacatccaactggtgaaagtccattccagacaacattcactaatcagatcagcagataaaatttaaaacctcagtggttttccattttattttagcggcatgttgaatgccccacccatcttcccataggaaatctttatctgaagcagatacaggcaaagcagctttgaaataggagtggaaatccagccattgagcttcctggtggcagcctgttaggttcttctgtggatagagttctacactcatcagttttcccagaacttcttctaaaatttcttctcggatatactgtgtgtacccaagaggctctattaatggaactccacagggaaaatgcataattcctgctcataa

SEQ ID NO: 46 - DNA, 500 bp, Homo sapiens
  source 1..500: mol_type = genomic DNA
ttcttgcagagcaccattttgcttggttgaactttgttttataagtgtacaaaggcttaaatcatcctgtgggcatctctgcatgtgtcacattcaccaggcaacttgtctaactctgtgaatatgtttcttttgaaggacttggctgattcattgtttgaagaaaagcaaataaacaacttaaatactgaaaaatgtatgagttaatatctctgacctgggctgagccaaaggcagaattataaagtataagcatttccctatagagtgtgctttcacaattcaaactgaccattttacaaattaatgataatgagattgatgaattaggaaacacaccttgcatcaaccagcctatcttccctcccagaagataagctcctgacggtcacagactatctctgattttttttcattttgaattttctgtgtctggtccagtgtctgtcacatgaatgaatgaatgaattcttataggacttaaatacttatatacagct

SEQ ID NO: 47 - DNA, 500 bp, Homo sapiens
  source 1..500: mol_type = genomic DNA
attttgtcctagactcagtatcagtgggttgtatctcactgccgtcatttcatggaataactaggagttactcaacacagtctatagctggtttttttaaccttttgataaccttgtatcaaaataatgcctcttttgatgctatatctaagatgcatccaaaaatgtcaacaaattactatggaggaaattaggttcaaagacaagctgggtgcagccacatggaaagtcacacagacaaagccactgcctaaggaattagttgcacaaaaatgaatatgaacaggttgttcagcactttttttcctctgggtgaccaaaatctgaggaatttggaaatgaaagtttattttattaccatttaatgtcctgtctacttagtcattttactagaaatatgaatcatgtatgtttttcaaggaaatagcttcacggatagagtcaagcattattatgaattaatctagtaactcagcatctttaccggcagtggaatattg

SEQ ID NO: 48 - DNA, 500 bp, Homo sapiens
  source 1..500: mol_type = genomic DNA
gcagagagttcaaaacttgagcttaaaggagagatgcccggggcaagccagccacagatcccagagacatttctgtcggggtacaactgacacactcctcccatctgaggtccccaggcagatgcatcagccgaactctaaaacttgattctagaaatcgactgcaggggagaccaaaacgcctcatccataaaatatgtgttttccattctcatctgtaaccattacagaatgttaagaagggtgagcttgagcaatcaaagtttccaaaatcccactgagaatcatatctggaaatgtcacagaaatgcaagcagctcatcagcccaccgcagaattttactggaactgtggagactctagtccaagggacgagctcaaggtgattgtggtgaaaaagcaggaagggtgagaagcctctgcttccagtgtctgcttgggaactgtgggagggtttggtttccttgcataagtttaagaaggcatcttggcagccacca

SEQ ID NO: 49 - DNA, 500 bp, Homo sapiens
  source 1..500: mol_type = genomic DNA
agtatacacgtggctgtgagtattaatctacagacagcaatggagagtattactaacagagagacaggagaaagagaagacagaaaagaaagaacattcatgtctgctgggcctgcctgaacttgactcatctccacatttacttgaggggcttgaagaaccgaagcttatgcttttaaaatgtcactatgtggctatcacagactccgaaaatagctaatgcctcttcccatcgccactttattagataaatacatctcacatgatataaaattgtgaaagatgaggcacaggggagaacaagttctcattaattaatacaacaaaattaaaatgtacttggtgaggattttcatgtaaaaacaaaaaaggcagtgaaatcatccttatgcagaaaccaaattcttttttcattgaggtagggtctctgccacccgggctgaagtgcaatgatgcaatcaaggcttgctgcaacctccgcctcccaggctccagcaata

SEQ ID NO: 50 - DNA, 500 bp, Homo sapiens
  source 1..500: mol_type = genomic DNA
tgtaagatggacatactaacaacatcctctttacaaagctgctgtgtaatcaagatgatatatagaaaatccatctataacttgaactctgctatacaaagtttagtcattactgctatattggaaaataaaaacatacaaacaaaaagaattcctttgaatgtaattcaaattttagtttcctgaacaggaatgttgaataaatttggagttcacgttcatcatctgtcttccagggttcaaaaagacaaaggtggctggagtcatttcctgaccccaaatccaatgatcaatttgttcttttatggatcatatttttggtgttatacctaagaaatcttcacctaatcccaagccataaagatttattttctatgttttcttttagaagttttgtaattttaggttttatatttaggcctgtgattcactttgagttaatttttatacattgtgagataaagatcacagttcagcttttcattttttattctataatt

SEQ ID NO: 51 - DNA, 500 bp, Homo sapiens
  source 1..500: mol_type = genomic DNA
tcctgaataaagctcctgtggatcaggcaagttcatttttgggtcactggcacttatgtatccaccattatcttggcccaatctcattatattatgccaactttgagggaagaactgagtcatcaccttcctttgtaatttcctagacaatgctccactcataatgggttttcagaaacatatctacctgatcaaagtcactcgcccactcattcaccacaaacctctgatgatgagatttgttttattccttgtgattcatcttggtgaatgtaccatgcggttttgaaataaatgtgttataatgcagatgttgggtctactgttccctaacttttagatcaagatagctgatagtgttgttcaagttgtctgtttttactgatgtttttgtctagttgttttatcaaatggagtattgaaatctctaactatggtgatataattatctttttccttttaattctttcaatttttgcttcatgtaaacaagcttttct

SEQ ID NO: 52 - DNA, 500 bp, Homo sapiens
  source 1..500: mol_type = genomic DNA
catcttgcatgtgctaaaacttgaaaacactaaaagagaaaataaacagataaacatagatggtgcaagaaccacgaaacaatgttaggtatattccccatgtgactgcaaccaggaataactatcctatagctaggaatcactttaagtcctatataatggcacactaaccatgcaataagtgaaatattcacctttgacgaagttaccaacataacactaatgagcaatctgtttcctctggcactcatatccatctcaatgaacctaacatcccccttcgtgaccttcatgccctttccgtgatacccatatctacagtagcttgacctttaaagcttaggagtagcacttttgttccttcattcacttccatctcccatttacagcccccaattgcattagagtgattcatatatcgctttcgaaatgccaacggacacacagtgactcacgttccctgctttcatcctcatatttccttatggaaatactgaggt

SEQ ID NO: 53 - DNA, 500 bp, Homo sapiens
  source 1..500: mol_type = genomic DNA
gaaaatacagagagtaagagggatagagagaagagaattatgttttacatagattgctcagggaaggcatcgctaactgggtcacatacagttagagagaagagtgttaaagagtgttatatacttcttcaataaatatgaatcgggcagaaagaaccacatgagcaaagactttagagaggaagagtgttctgggtaagcaagaggaactgcaagaatgcccatggacctggagtagagtaaatgatgggaaaagtagcaagaggtaactacagacaataagtgggatggtagatcattagcgacttgtaagtgacagttgaaatgttcggaatttgggtaaaaattagaaatccacttgtgggtctttattgtagatgagaaatatgtcatcatgaagtgtatcttctagaagtatctctgtttgctcaagataaaagggtttatgactgacacataaatgaaagtttggaaatgcttagtggttaatgactcagcca

SEQ ID NO: 54 - DNA, 500 bp, Homo sapiens
  source 1..500: mol_type = genomic DNA
atgccggcggccaacatgatggagaaccggccgctgcccgccctgcaggtgcccgagccgcagggtgcgcccgagggcagcccggtctggtccagttcgtcgacccccacgcttcgccgccggcgcttcaagatgcgccgcatgaagaacgtacaggagcagagcctggaggccgggctggcccgggacctgcccgccgtcttggcccccggcaaggagttcctgcagctgccgtccatcgagatcacgccctccagcgacgaggacaccccgtggtccaactgctccacacccagcgcgtccccgcgccgaaaacgcttcctcctccgcaagtggctgagggtgagggagcggaaggagtgcagtgaaagcaggtacgtccccgttccgcccgtctccttcccttccctcccgtcctctccagagccgtccagggccccggggcattctgggggaaacgtcctgggggagaacaggagcccgtcaccagaggcgcttct

SEQ ID NO: 55 - DNA, 500 bp, Homo sapiens
  source 1..500: mol_type = genomic DNA
gttataccagcattttaaggcaagcattgctatccttgctttacagttgaggaaatccaagtcctcaaggccagtaagtagtagagtcaggatttaattccagggtggccaggctgcaaagcctctgctgtcctgtctcccaccaggtatagaacaccacattagcactgggctgagtagggcagctctttatatcacagggctatctttggaccctactgggtcataaatttgttgagagtacagaccatgccttataattgttttatgacacagtctcattacctgtgaaaaacagagctaatctttctgtttattctccagtgagtcaaaccaaataatgtccatgtgagcctttgaaatatggtggagaaagtgggattagggcctcaggcatgaagaagagcccatgcagctcctctggaaacctaccctctgtcttctcaatgccctattagaactcgctcagttcttctgcagattccttctggcgttcggtg

SEQ ID NO: 56 - DNA, 500 bp, Homo sapiens
  source 1..500: mol_type = genomic DNA
agctctcgggctcaattgctcctgaagaaataaagaattaataagtcaccttttttcgcctctgtggacacccttttgaaattttttcttccaattgacttggatctcctctggattttttttccctctttcccccgtcggactcttaaataaaagtgagcaagtccaaagcgtggtccggagagcgtggacaaggtaacctgttttggatgtccgggagaagggagtccggccgaaagggcccagcccctcgaggctgctccaactggggcgcgcggcggcccaggagggaggcggggaggtctccgggttgggccggggaacgccggcctccaggctgggtagggaggacggtccagagcgcgggcctccgggtctcaccccgggaaaagtctgggtctgctctgcgctgttgcgtgctgcgctcctgggacctgctgactgtcctagagggaacgtcccgcggtagtgtcagttccctggggaccaggaagggcgac

SEQ ID NO: 57 - DNA, 500 bp, Homo sapiens
  source 1..500: mol_type = genomic DNA
catgttacaaaacacagactatgactgctgaaggtggaggtgactgaattatacggggcaagaatggaggcagagagaagcattgagagtctatagctgtaggctatgggagagataatgatgggttggaggaaggtgggaggagacctggtgagaagagaaatttgactggggatttttctttaaggtatactgacagggcttgatgccttgtgtgtgggggctaagggcaagcaagtcaaggatgaccctgggttatgtagctggagcacttggtgaaggctcatgccatgtccgtagaagtcagcagtggaaatttaagacaagggaaaagtcaaaagtccttagttggccatattacaattttttgtcatgatcattaaagtattttaaaaaacagcttgagatataattcacataccatacaatccacccatttaaagtatacaattcaatggtttttactatattgtgaatatatgtgagagttttacatccat

SEQ ID NO: 58 - DNA, 500 bp, Homo sapiens
  source 1..500: mol_type = genomic DNA
cagggcctaaagagcagcatagttcaggccactcatatgactcgtatatttttagatgtttcttagcatgtcagttcttttgctggtttagttttactgcccattattgagacctgtgttcttattaggtatcttagcctacttttttttattgctataacagaataccacagcctgggtaatttataaagaaaatatttcgcttttggttctggagtctggaaagtccaagagcatggtattggcatctgacaaggacctttgtgctgcctcttaacatgttggaaggtcaagggagcacattagaccaagagataaatgtgtccaaacttatcctttcattaggaacccaattctaatgtaactgttgcactcccatgagaatggcatgaattcattcatgaggatggagccctcatgacgtaatcacctcttcaaggctctacctcctaataccattacaatgacagttaaatttcaccatgagttttggagggata

SEQ ID NO: 59 - DNA, 500 bp, Homo sapiens
  source 1..500: mol_type = genomic DNA
catggctgggcagggactctcgggtagatgcagcgctgactgggtgcccccgggaagaatacctcgcatttctcctgaggtggtgaaataggcggaaactggttcccatccaaatcctggaaaccaccatgggtgaggtcatgtccacacatgtcaaggccttgatgagatagttatctgcatagtccagaaaaatcacttttccaccaaacattctaaatgattgatggagaaacaaattttccaattacgctaactttcattgttattactaaagaattaagtgctacaccacacacacacacacacacacacacacacacacagtcacacaatattcagataaaaagaaagcctaattattttatattcagaaaaaaatgaattggcctttctgaacaaccacaacgatgaaaaaggaaaagaaatctgttaaaactttaattttagttttccttttagattttaaaataattgtgaaatatttcaaacatagaaaa

SEQ ID NO: 60 - DNA, 500 bp, Homo sapiens
  source 1..500: mol_type = genomic DNA
ggctctgacaccctctttgggactctgtggttctggtgtctccaagctttcgggcgccactgtgttctcgttcagatgcggatgcccgcagcagaagctgtgtgcggtacatctggtccagccgcagcctcgcatggagcttggcatctctgccagtgcctggagctgcccgccccactgcagcagctggcatctgtgcctggctcactgttgacaggtgtgggatccgggccggtagcacgagccaagcaccgcctgcagggacaagtggacagaatgagcccagtgggcaagcaatactcaggtagaaggtgccgccggccacagacgtttctggctggtgaagtgacaccccagagatcccgtgacaatagtttagttagggagttacccatgtacatgattatcttcatttaatataagaccatacattatgagtgccatataaagtttaatgctttaggtagtataaaaatatctttcacttggataactttata

SEQ ID NO: 61 - DNA, 500 bp, Homo sapiens
  source 1..500: mol_type = genomic DNA
agtctatacaagaagttagagaggccaggaaaaggttgttagaaattaggggacaacttttggaaagagcttttggtgtgctatcagtcctactctttcccccaccgaggagcaggtaaaaggtaattcctcctccatctcaaatctgggtgaaaggtcttcagagagatttctcagatggttcagtatgtgtcccctgcagtctgggcattcaggtctagtttatgactcatccctgagaaatctagggagtaagtggctgaggagctaaccgcactgacagcagaacacagaagaggtggctgctgccctgggctgggcctgcactcccgagtttgtcagggcaaagaatggaggagtgtttcttgtcaacttgttatgagagagagttggggaacagtcatgtgaaatcttgctggagacagctgactagggtgttgggggccggtgataggtccccaacagaaaaacagggattttgtatgtgtgggaggggagtg

SEQ ID NO: 62 - DNA, 500 bp, Homo sapiens
  source 1..500: mol_type = genomic DNA
ttaaaataagaacaatccagtcccctgtgaatgtttgtgcatgtatgagatgcacaatgatcacgtatgaccttcaaccagcaatttgcgaagtcacgactggtttccattcatccagacacaccttactacctagtatcccctcctcccacatcaaataagggtatagtaggggcagtttgtggtctcaaccctaccgaggtaagagggcacaaagaaaattgatatgcatgagacctcgggcattcttcaggtaaaaagatggcttaattggaacattcggaggcttaagagaaaatcgggagtggtggaaggaagcaatcaagcagggtaatatttcccaaatgcctaccggccacgtgccagacacaatgttaggctctatctgtgatgtcttatttaactgaagagggagaagaatgtgaataaatggctggattcttgaattgcataaaaagagaagccaatacactttttcctttatttcgtttaaacaagta

SEQ ID NO: 63 - DNA, 500 bp, Homo sapiens
  source 1..500: mol_type = genomic DNA
attaatctcggtaaacaacttgttttgatgaaagctgaaagccagatgaaacaacgaaaattcatggttatcagaaaacaaaacatgatccctttctcctcccacctcttcctgcacttttctgtgacatctaagcctttgataatttgggccccataaagggagggcggaagtcaggctgtttgcctcaaagaacatgccggtagaccgttccagaaccttttgagagtggacatttgcagagccgggtcagagtctagggcctgggaggagtcctggagagctacaggttttgtgattttttttttttcccctcggaagaaagcattcctgaaggcaattattatgccttgttatttaaccccagctggttgtctccggggaacagagctgacatccattgtgatcatcctcagcttttcgggtgaaacatggttccttagaggctccaggatctaagggggtgtgataaaccaggaacacatacactaatggaaaat

SEQ ID NO: 64 - DNA, 500 bp, Homo sapiens
  source 1..500: mol_type = genomic DNA
atatatttgtatcaagttacttataaagtctattttactatttaggttcccagcaactcccttttcatgtttcactataaactattgacagagacaggagacaaccaaatgctgcccaggtgattgtgcacaggaggcttgcctaaacatgcccatggtgaaaaattctgtagtttaacacatgagattaagggagataaagcaatgtggagtggctcaaactaaggacccgcctgctcactgggataatggggtggaaccaccggaaatttgtgccttttgcagcggggaggagcctggcctcttcagctcatgtgtggcagcctggtattcaatcttgaagtgggagcctgttggcaggaccccctctttttttgccgagagctttcttttaataaattccgctttcctcacctttcaacatgtccacatgattactttttcctgttcatgagacaagaacccatattttagctgagctaaggagcaaaaacatcctg

SEQ ID NO: 65 - DNA, 500 bp, Homo sapiens
  source 1..500: mol_type = genomic DNA
atatagcacaagctgcatgagctgcaatgcagagctgtaattctttgctggagcagtttcctcaactctttatctggtcccctcttctggtaaactaatctgaccatgtgtgaccattaggactccttttccttttctccactaagctgtagagccacgtctaagcattattttcaaatctctttcccctaggccctcagtctcacttcacttaacacatctgagctaggctgggcatagtggctcacacctgtaattccagcactttgggaggctgagggaggtggatcacgaggtcaggagatcaagatcatcctggccaacatggttaaaccctgtctctactaaaaatacaaaaattagcttggtgtggtggtgcatgcctataatcccagctactcaagagaactgaggcaggagaatcgcttgaaccagggcagaggttgcagtgagtcgagatcgcgccactgcactccagcctggtgacagagtgaggctcc

SEQ ID NO: 66 - DNA, 500 bp, Homo sapiens
  source 1..500: mol_type = genomic DNA
ttttttttttttcagacagggtctcactcttgcccaggctggagatcagtggtgcaatctcagctcactgcagcctcaacctcccaggctcaagcgatcctaccatctcagcctcccaagtagctgggattacaggtgcatgccatcatgccagactaatttttgtttttttttttgtagagacagggttttgccatgttaccaagtctggttttgaactcctgagctcaagcaatctgcccaccttggcctcccaaagtgctgggattataggcgtgagccaccacacccaacctcaaactaaaaataacttgttaagtatcagggagcgagcactgttagacactgatcaggatataaactggtgagtggtaagttttctgttcaataaaaaaattccatgagaaaaaccataaactcctgtgcaatcaaaacctaaagtcatgagttagattataagtattacagaaatacagaaaagtaaaaataaaatcattgtg

SEQ ID NO: 67 - DNA, 500 bp, Homo sapiens
  source 1..500: mol_type = genomic DNA
cagcgaggcaggagtgcagaaagggactacttaacctgtttagctaaaatgactggaacactggatcagcatttccttgctttcttttgcttggaagaaaaaggattgcaaataaactccaaattgcctaagaatgtagtaattttcttcctgtttcttgataatgtgagattttgcttttcttctatgaacgctaaagtgacctgagaagtgaagagggtgagtgcaagataaatctggaatgcaatagggactccagtgttatggttataaagctgcgtatttccacagaaattaagtggacacattgcagctgagctaggtgtgcagtttccacaggagtactctatctaatgcaggcaggaaatctccaggaaactttgatgtttaaaggctttaatatttcttcaatgcaaagagctttgtttttaaggacttcactaaatacgtaaactttacaagaattttagactcccaataaatttatgaaatcatgtcaa

SEQ ID NO: 68 - DNA, 500 bp, Homo sapiens
  source 1..500: mol_type = genomic DNA
aactcctaatattttatatatactagcactttaagaaagctttccaggcgggagaaatgaaagtacaggttccatggtcaccaggaaaccctgtttacaagagccataatttgaactttgtaatttgcagaaatatactacagaaattgaagtaattagtgctgcgctggtaaatcttaaaatggttttctacttggaaaaggtctctcccaaaataaaaacaattgctcaggttataaaagcagtttaaaaataaagtttaaacgtaacaggtacaaactgaaaagttatttatcttttttttaaaaaaagtgtctgtattaacaacaaggaggctattccaatataacacagaagactacataaattattcaagttcttagtacttttaaagaaaatcctttcatatctatttttgtgaatttgggggtataagagaaggttatgtcttctatatgggggggtgatataaattattacagttcattctttccataaag

SEQ ID NO: 69 - DNA, 500 bp, Homo sapiens
  source 1..500: mol_type = genomic DNA
ccatatcattttcccttttggaaaattggggcccttgcccatcttcaggctttacttactttccagcaatttctcctgggtcctctttcactgtctcctggccaaccatgaattcaattctctctttagaacgtctcttcctcccgtgggattggaaagaacatttgtcctcagcggcaaaggcagggcttcatcaaagacgagtgactcagtgcttttcctgctgtctggccacatgatccacatgcccgcaaaggggacgtgtcttgaacatgtcatgatttcccctgaatttcttatgttattcttttaaaattcacctggggaacttactcctttttttttttttttttttgagacagtggctctctcagtcacccaggctggtgtgcagtgcagtggtgccatcctagctcactgcagccttgaccttctgggtttcgagtgatcctcccacctcagcctcccaaataactgggaccacagcacctgctaccata

SEQ ID NO: 70 - DNA, 500 bp, Homo sapiens
  source 1..500: mol_type = genomic DNA
cacacacacctcagagcccaggcacacaccccagagaactatgcacacaccccagagcccaggcacacaccccagagaactatgcacacaccctagagcctcttgtggttgccctttgcctggagctctctgattggatagttgtaacagtatgttttgggctgcaagtaacagaaaacttaactcaaaaatggctttaaccaggggtcaacaaactgctgcttatggtctggctccttgtttttgttaatgaaggtctataggaatgcagttacgcccacccatttctattgccgatggctgctttcatgcaacaacggcaagctgagtcattgcaatagagaccatgtgatctggaaagcctaaaattatatttaatgtctgccctttacagaaaattttcaccgacctctggcttaagcaataaggaagacgtattacttcatatgatgaatgctcagaatgaaggtggcgtattcgttatctctgactacacaaca

SEQ ID NO: 71 - DNA, 500 bp, Homo sapiens
  source 1..500: mol_type = genomic DNA
cgtttttctctatttaaatactgtaatattttcagaccatgattggccacacgtaactgagactgcagaatgcaaaatatcagataaagtaggtactgctacatataaattgtggtttgttcatacatgaaatagtatataacaataagaaataacaaattatatttacagacaacaagaataaaattcacacacatgtattaaagaaaagacccatactcaaatgtatatctcgtgttaaagcatttttgataaagttagaaaacaatcatggtgaggtaattcaggatgacggttatgtctggagagtgaagtaactgggaaggagcatgactgtgcacttttctgtttgtagattgtaattattttttaaaggattttttaaagtaaattaaatgcatagaaattacaaatgcattaaaaaatgagtaaaacaaatccttgactcagtaaacattgcatcaaaatattgcaaaacatcagattctgagttgttgaaa

SEQ ID NO: 72 - DNA, 500 bp, Homo sapiens
  source 1..500: mol_type = genomic DNA
ccatttaggggtaggaggaagggagactgggagaggaatgtaggacgtagaggtcacatgaaattatggctgctccaaggggaacacagtattcaaggcatcacgggaagtacaggagcacaggccctcagccaggatccctctcctcccagcctcacggactctgatcgggcagcctgggggctaactggtctgctgggagttggatagtcagtgaaagcactctgctctcctcccccagcctgcctctaggtaaatgtgtgtatttaactaaaccacaaccacaaaggctcatgaaattttcctggaagccaattaaagcaaggagagtcatagtagtagatagtattaagccatgtaccaattctttttggcttacaagtgccggaattgcttgtttatacattaagagcaaaaaaaaaaaaaaaaatagactgtagtcttttctcttaattgctgtaattatacttgtgccacccacaagagaggccattgatctc

SEQ ID NO: 73 - DNA, 500 bp, Homo sapiens
  source 1..500: mol_type = genomic DNA
gtagtaggtctctgtaggtctctgtaaaaaaaaaaaatctactgctgactgtagtcaatacgtttgaaagtcactgccttggtaacattattttacccacttactgtcatatgacatttaaatgccaatggttttgaaaagtgtatctataggctagatttttatcttgaactcagacccatattttcaactatctaccagatattagcacttggatgttccacacgtcccacaaattgagtaatagaatgattaaaataatgggctttgtagccagatttgagtttgaattgtgggatttctcagcctgttttctcattcttaaagtcggaataattaaaacctcaaaatagtgctgtaagaatttatgtccttagaacagtgcctggctcacacaaaaataaataaatatcgcttgagcaccaaccacgttccaggtattgttctaggcactagagattgatgagaaaattcagcccccccaccatatgagacaatgc

SEQ ID NO: 74 - DNA, 500 bp, Homo sapiens
  source 1..500: mol_type = genomic DNA
atataattcaggcataattattttcatgttggttttatgaaaacttatagtacattataactaatcatgttccagaaaatgcaaataagataatagttgagaaggaatagacatcaaatgcttctttaataaaccacagccattttctctaagcagggaaaatgctttaattgaatttcatcttattagaaagacattatttcctccagagtcataaagtatatacaaggaagattaggaattgtgcctgttggggctattttgtaagcaccacaatctactgtggtgctactgtggctagcgtaggtagaaaaatgaatttattgaaagatattagacagctcagagaactgttgggtgggctgaggaatagtctcaagattagcccctccggaaccattcctcagaaccacaccaaagaactggcctgagcaggaagttaccatggccaccaccacccccacattagcaaaaggaatgaatcatccccagtttgtttc

SEQ ID NO: 75 - DNA, 500 bp, Homo sapiens
  source 1..500: mol_type = genomic DNA
ttgctacagttcacctccacggttaagtctcacttccgcctctaacttacaaaaccatagttacacatctgcagcttagccacaagggagtctgagaatgcagattttttttttttcttttcaaattacccttggaaaatggagctcacaatgtggagaagtatcaaatgaatagagggtgttgaaggcatgtggaaaatttggtaggcaaaattctaagatcttccactatctccactccctgatgttatacccaagattagttatatggcaacagggattttgtagatgtaattaagggccctaaatagtttactttgagttcatcaaaagggtgattatccttggtgggcttgacctaaccaggtgaacccttagaagagaatgtgccctttctgagaggagatttgaagcataagagaattttcctgctggtcttaaagacacaaagtccacaagatcgacagctgcagggaaacaaattctgccaatgaccccat

SEQ ID NO: 76 - DNA, 500 bp, Homo sapiens
  source 1..500: mol_type = genomic DNA
taccttgctatagaagggaatctgcattctggaaaagtggggtgtgataggttttcatttgttgagcaaatatttattgaacagctactatgtagcaggcattgttctaggctgggaaacaatacagcaagtgacaaaacagataaatccctgcctcttggaacagactatctaatggctacttatttcctcctggtcattttttcttccatttactggctcctgacatggactcttcagagatgtaagaatggtgtgaaggatccgcagggaaggtctgtgtgtgttgtggatttaaactgatgttatgtactctgatcctagcacatattcagagctgactcattttcttatgggtgtgtctcgaattcattagaaccttccctgctgggattctctaaccacagctcgcctgaagtattttgcctttccctctggctaacagtttcccctcagcccttggttttttggttgtctgtgccacagactttctctatctg

SEQ ID NO: 77 - DNA, 500 bp, Homo sapiens
  source 1..500: mol_type = genomic DNA
gacatgacaagctctgaggcattatttatactccagagatgccctgcagcatcaggcccaggctgagactttccttaaaatctcaccacttcttggcttccttcccttcgctttactgcttctcctactcttttgtggggttaaactgtaagcattcttttaaatgaatcacttgtacacatgatttaaaacagccatttcatgactgggcagcaacttagcatagtgataatgaggaaagataaggtactatcaccctcttcttgatcctaacctcccttccaagagaaataatcattgtataagtttaaagtcactgggataattctcttttccagtagctatgcttctgaaggtttatactatagaaatattgactttccttatgcaaaacaagcagaagttctgcctaccctgcgttcatcctccctcagccttaaaatgaggcattcagatagccatgcagacattgttactcttattagaatttttccaataaa

SEQ ID NO: 78 - DNA, 500 bp, Homo sapiens
  source 1..500: mol_type = genomic DNA
acattccagcaaggaggggtgtggggtctttcacgtagattgcagagagtccacctggtatacattctggttggaaggggtggtaaaatacagctgctgtgctggaaccctgttgtcacatgggctgctgagtcccagcgtcctctcgaagtccagcagctgacccatgaagttgaagttaggggatatgttggattttttcattttgacaatgtcataggcgtcgttcatcgacagattgagcttctgcataaggtaagccacagtcacagtgactgagcggctaatgccagccaagcaatgtaccaagacaccacagttcttgccccgggcttcatctgtgaacacaaaaagaaaagcaagatctcagcagactgaaaaccaccctttgtgaatgatcagtctaaaaactgaacttgaaaacataataataataatagttgtgtgtggcagttgagccctacaagcagcagaaaatgtatcactgaaatgaaacatgt

SEQ ID NO: 79 - DNA, 500 bp, Homo sapiens
  source 1..500: mol_type = genomic DNA
agtcatgattcgtatctttgtttcatcttgtcgttaatattatatctggtaattttcttgaaaacataaggacttattttacaaatttgtatgctttcataagtacttcattgtaactttaatagtaaataaactttggctttattaaggtgtaggagagaaaaccctacgaacagaaataaaacaattgtgatgaatcattcattaatccctgggagaagcagagtgggcgtactgtgggcttaggctcactaagaaggacctggattcacatcctagctttgtccattgtatgtggccttgggcaggtctcataagccacactcctttgcaaaatgaagataacaatatctacttctgagagctgttttcagaggatgaaagtgcataataagtgccttatcttacacatggcccagtcttggctcaaaaatgttacttttctttcttgaatatccccacttcctcttgaacagcctcccccaaggcagttagttgct

SEQ ID NO: 80 - DNA, 500 bp, Homo sapiens
  source 1..500: mol_type = genomic DNA
tgtactaaaggtgggtggaaattccactcttagatccaggcaccctcaggcgtcagccctgagccctgtgctttgcaaacttctcaagctattattatgtaaaaatagatatcttgggatattattcaaatgcactctgtgattccttagagctggggttggggcctgagaagttgcatttccataagttcccaaatgatgctgatgttgctgcaggtccatggaccacgctttaagaacaactgacttagtaattcccattctgtctcttttagacaggcccttcccccacaggctgcagttcatgtgacttagggaacctgccaactcagaacctgtgtccttttttcctaagccgcactttggttatccaagaccccagaattacctgtccagacagcctcccaaaactgtgcatacctgtccccagtctgtccttgcaatagaagactccaccagtgtgtacacacctgtatctaagtgtggccagaaaatcagct

SEQ ID NO: 81 - DNA, 500 bp, Homo sapiens
  source 1..500: mol_type = genomic DNA
agttttattccctccagaaacctttccatgcccctcttccttggccctatagcaccttggtccacctacacagaattgttcaccacatcataattgatcctgtcttttgtctttcctgctaattccttgaaggaagaactcttcttcacccctgtatctccagcatcaacagttcaaacacagcagcactttttaagtgtttactaagttttgttttttgtttttttgagattgtagttactgaaaaagtgataaaaagcacgtggacctaaaagaaataattcataaatttcagagttgtaataaactctgaaaataatctttttcaacttcttaatttacaaatgaggtttataaaaaagatttaagaaagatttttcccaatagcatggatatgagagaaggaaaaataaactagtgaagataccctcccctaccccgaaaatcttaaaactgtctaaggaaaaggtatctggggaatataatggataaatggaatg

SEQ ID NO: 82 - DNA, 500 bp, Homo sapiens
  source 1..500: mol_type = genomic DNA
catatacaccatggaatactatgcagccataaaaaatgatgagtttatgtcctttgtagggacatggatgaaattggaaatcatcattctcagtaaactatcacaagaacaaaaaaccaaacaccgcatattctccctcataggtgggaattgaacaatgagaacacatggatacaggaaggggaacatcccatacccctaatcttatccatttgttcatggcagaacccagacctcaccttgagtcttttttctccattttttactcccttttccatccagcgaatcaccaatccaactgagttttcctctgtataactgcttatttctgcctttagtgcaatttctgtaacataggtcactatgatattggccagatttaaagcaacagagcctgcatgtactttcctctcctccagcctcctgtttcctgtccacaacactgctagggaactttctaaacagcaagcccagacatgttagactactgctcaaaatgt

SEQ ID NO: 83 - DNA, 500 bp, Homo sapiens
  source 1..500: mol_type = genomic DNA
tcattatcctttctttcctgcttaccatacatcgtttaccaaccctttgaaaatttaaactaccaggttcatctagctctggcactgctagaaccgagactacagaagatgtctgagtcttccaagctatttgggtcaaacaaaacaaacaaaaccacacacagccaccgagttgggttattttaaggacttagagctacagaaggcaatctgtcagcatccgaggctgtttcaaaaccacctcctccctccgtgcttgagtcaagagctgcagtctttctatcgcccatagccatgctgcagcacttcctcaatcaccctcttctcgctgcacgcattgactttcggtttcttcacagagtcactgacagcttgcagctttggcttatcgatagccccgtggttctctccatccatgacctaccagatggcattttagtttagttcccaccactcactgccttatttaattggtatttcttgccccacatttccaaagc

SEQ ID NO: 84 - DNA, 500 bp, Homo sapiens
  source 1..500: mol_type = genomic DNA
aagcccggtctggattctgtttggttcagccatctcatgggtctccagctgcttccctgtcctgtaggcggcctgcgtgaggcgcagttcctacttccaaggtattgtggggcagtggctatttttgcaggctattgtgaggcagcagaggtaaagtatgagttgaaacatacaaacaaaatatggcccctcagcattgtagaacttttgcagataatgaattttagaaccaaatagagcaggacatttgttttcacagtgagtcttatggctctacttagaatcttgtcactctgttttgcagtcacctctccaagtcattgtcttttattgtacccttgagaaacaatactgtttccattccaaccactttactgagtatttttactcagtggtcaggtcacaaataatctgttaagttttaaattcagttgtcttgtattgctgatttctctgtcttatttaatgtattattcacttcttaaactatttctcttgtg

SEQ ID NO: 85 - DNA, 500 bp, Homo sapiens
  source 1..500: mol_type = genomic DNA
gccatgagcccactttgacttgactcattattaataattttggtaaaaaggaaatatgctgtttgagattttaagaacataatttttaagttaatgctggcgatgtttcttttgcattttttaaaaatgttgctgactgagaacccaactctcaccaacccctcccttctcaccgtactatattcctggaattcacactgcaaaggcgggtgctttcaaaattcactttttcccacaagcggattcagaaatgcggaggttgcctgccgccttttctaccggacaacattcccgagttattggtgagctggaatgtgactgacttgcattccagggtttcttaaagtcaaaggttgactaaccagcagattccctcagggaaaagaggcagtaaatgtatctttttcaaggtaacattgcatgaacttgtcaaaagacaaaaaggatagaggggtttgtattaaaagaaatgattccaaggtacctagaaataaaagtaa

SEQ ID NO: 86 - DNA, 500 bp, Homo sapiens
  source 1..500: mol_type = genomic DNA
tccagctctatccatgcaagggaatactctctatttgctgatatggagcactgtccaagatgtatggcatgggaaaacaaatctagttgcagaacagtgttaaatacatgcactcacgctaggaggatatttttggcaggtcaccccaatacctgtgttgggggagtgggaagttaaggagcagggatgggaagaaaggtgtactgtttgattatttttgttaaatctcatgtgtgtaatagtttttcagtatacgaatgataaaaagaaaagaaatgatctcggccagggtggtgacacaagtttgtgaaggcagtgtcaatctgtgctaaccaatgtcaccatgggttggaggctgtcgagcttccctttcagctgttttccctctttcttttgttcttggtaattatttattgaacttaatggggaagatttcaaggcattttaaccacccagctttactgaatgaaatgaaaacatcaaagcagacatttatattg

SEQ ID NO: 87 - DNA, 500 bp, Homo sapiens
  source 1..500: mol_type = genomic DNA
tgtgattggttcatttcatttagcgtaaggtcctcaaggttcatccatgttgtagcatgtgtctgaatctccttccttttaaggctaatattctattgtatgtatacaccacatttttttaatccattcatccaccactggacacctgggttgtttctgtcttttggcttttgtgaataatgctgccatgactatgttgcgtacaaatatctgttaaagatcctgctttcagttcttttccgcatacacccaggggtaaaattgttgaatcatatcatttcccatatttttaaaagacattcctgcacagcatttgcagttgtagttccttgctaggaatctaatgtgccttttcaactgcctatgtcttttgattacgatcgttactattgttagggctctggtgatgaagtcctcagggttcaaggggtctcagtcctactttcatgagccccgttgtcttttgtgcacaatttcacagaacacaaggcttttttgtt

SEQ ID NO: 88 - DNA, 500 bp, Homo sapiens
  source 1..500: mol_type = genomic DNA
ttaaaaaattaattagctgggcatgttggcacatgcctgtggtaatttgctactgttttatgtaagacttcacatctatgttaaaaggtgagtctggtctacagttttctgttttggaattttgtggaaataaatctttattgaattttttaagtttatttttatgggtctattaaagttcctattttgtccagttaataaagatttttctatttataagcacttaaaagcatttactatgagatataatcttttaaaactgcatacttaatgatcccttccttcatttgacaaatgttgattgcttgcatttgactttatagatttaattcgtagtaaggtgtctgccacatcacattttaaggatttaatcactgtggctggagctgattttgctgctggtaacacagttgtgaacacgactggaaaaatcctggaaaccacagacgaagtcaacaaatggattacagacggtggaggtgggcaggtgtggctgcctg

SEQ ID NO: 89 - DNA, 500 bp, Homo sapiens
  source 1..500: mol_type = genomic DNA
ttcatgtaggaccatgtggtctctcaatattgagatgtgggaaccacaggagaaaactaggctatgaaggccaaaaaaaaaaaaaaaaaaggtaacatttaactaaaatgttaaatacaagttaagctaatgtacaatttgtgacccacatagacatgctatgacctagtgatttttttaaagcttttatcagagttggcaaattcccacaaatattagtctcagacaatttggcttcatatttcagaataatgcgtctgtgattaacaccctgggcttcttcacagtattgattctctgggcctgatgtggtaagcaagcacaccagggatcacaaggtcattttctaacttgccctgagcctgtggcttttgtggttattgccatctgccgctgttgttattgctattgttgttactggatctcatacacagtctggagctaaacgtaaagcctcatcctgcaggcatcatttcacgcgactgccacagtcttctccc

SEQ ID NO: 90 - DNA, 500 bp, Homo sapiens
  source 1..500: mol_type = genomic DNA
cttgggcttgaaatattttatcacctgtcctacagagttgttgtgaggattcaaatttccaagcacataatagatattaaataaatgtccattgtccagttttaccttatcaccttatctcctaaagttgatgtttgtttatatttatttagagtacagcctgcagttatattcatatgtgcttaaatcatgatatgtgtataatggggcagtgacacttggtctcttttaagggctcacatttaaatgctaactcacttgaatattttgaaaaataaatgctttttttgaaaggacaacttaatgtgttttttcctgtgattttacatttcattttgaatgaaaggttctgggaaatgtatgattttgtaaatttctcataatattgcaggttaagatttacctaaaagtagtgatacattaaataaaatcacgctaattttgtctcagacttttgaaaattgtgtggttgtgaatcataagttataatattactattg

SEQ ID NO: 91 - DNA, 500 bp, Homo sapiens
  source 1..500: mol_type = genomic DNA
ttttagtgaagtgatacaattaaataagaactgttggactgtgcatgtgttaggggatccatttgatttcattgtctccttgtcagcatctcttttgatgctacttttttccccttgtctgattaaatggcattttttgtaagaggtatttaattataagaatgcttacattaaaatctcttggcctataaattctcatgtgagttctagttgcttgttactgcttcctttaagatctcgggggcggtgggtggttggaaactcactagatttacttccgtctttactcactgggttttggtattacttcaggtgatttgtaatctctaggccacaggaaatgggataatgtaggcttttgatgcaatggattggactttgtaaaggtgaagcttcaagctatctacttagggtgcctggggactttgaagagttatagaactatgatgcagctgcagtggcctttctgtaaatgtactactttctgttcacacatctca

SEQ ID NO: 92 - DNA, 500 bp, Homo sapiens
  source 1..500: mol_type = genomic DNA
ctccaggtcatcatttaagttgccaatgaggaaacatcctcaaataggacatgtcttgttcaaattaaatattgctacataaaggtcacaatgccttttatttttggtgaggcatgtcttgcctgatattgggcagatctgactcagtctgacatcccctcaatccaatcccatggttgggggtggtggggcagcagcgggggggttacagccctacctgatcgaggcagttgctgcgtagatatctcagtgcttgctgaatactttgaggcaggggctgtcccgttctttggacgtggactatgagaggaacgccaaagacagccttgtctttgtagtcgggaactttcatcctcttcatgaactttggaactgacctagaatttacagaaaccaggtcatgcaagcctcctgggtcacactgtggggtgaggctctggaagcaagcatgagggaagccaggcttttgttggaatacccaacagatgcggggtgaattc

SEQ ID NO: 93 - DNA, 500 bp, Homo sapiens
  source 1..500: mol_type = genomic DNA
aaataactagtccagaccacttacacacagtagaaaacataaaaacaaatgcgcccccaaaagactctacttagggttcccacgacaagtcttccaaaatcaacagtgcagtctgtctgaatgttatcaatgctcactaaccatgcattcccatgacatgactcagtgactccatttcctgcctacacttccgctagctctgggcctcactttgagcttgtctgtcaagtatagtaatgccagatacttctagctcctacatgtacaccataaaaatacttcagaaaatacacaacacatgagaataatatcagaaaccaatttacttcccaatttcatccattcttgtgattgtacctgtcaattaaaaaactattcagaactctatcacattaggttttcttagacatcacttaagccaattatcatcttaaccattttaagtggacagctcagtggaaatgtggaattttgaacttgtcttttacattagagacttg

SEQ ID NO: 94 - DNA, 500 bp, Homo sapiens
  source 1..500: mol_type = genomic DNA
atagccatggtacaattctactaaagccaaaatacataattatcccttgatccccttcccaaaatatgttatgtgcctcatagactgaactgagaaaaagcattgtgcccagtgcgaactcaggcagccttgcctggaaggtgctactctctctccccaacgcagagcaggaagtgagaaggaactcagctggacaggataaaaatgctaggcagctttccagctccttcagagcaagtcttgacagtggacttcattagttttattagagcatcatcaattccctaaatgtcacatggagctctattcaaataccagcaaagaaatataatccaaagacaaacataccttgtttggtgattattcagtgtttataaatattcacatcctggctcttctccagggaaaatatgaaaagcgtggagagctgatgattcttgatcctgatcagtcatattgggaactcgatttccttatgttaaaaagaagggagatgttat

SEQ ID NO: 95 - DNA, 500 bp, Homo sapiens
  source 1..500: mol_type = genomic DNA
cctgtgtgattcctggtataagaacacttgagacaaaaaatagcttgaaacctttcaaggtttcagtgatttcttaaagtaattatttcatcttttaatatcagatttatttcaaagtcaagcagaggattgaggtcactgtttgcacaatttagaccctattttatttcttcaactagaacattttgagaatcgtggttaattttttagaattgtttattcttcacttgactgataaaggcctttgcctcagttttcttcatcaccctagttcacaatcatatagtcacatttgtagtgaagagtactttttttctctacagtgttgcttaataagcttgatattggtattaataggtttttgaaaagaaaattttgagattaaaaatggaagttgggagtatacttgtaagaattgaccaccgctgcttgatttgcagacttgaagtaatactggataactagccaaaacttttcttttggtagaaaaagaaatttaa

SEQ ID NO: 96 - DNA, 500 bp, Homo sapiens
  source 1..500: mol_type = genomic DNA
caaaatgaaactagatctctcatttgtctgtatgggcaagatatggtaaacctcatgatcaaaacacatgccagttagaaacttgatcacagaaatgatgctcagtgttgaaacccaacaataaacaaacaaacaaaaacccccactctaaccagaggcatttaagcctctccactgaagttcctgtttcccaccagtttacgacccttaatgttactgcatgtatggttgcatatttgagatgattaaaaataaaagactggcttaaaagcacctcctcctctagtgtgtaattacatacaaactaaagattccttctgacgtcctaggaaccccatttgttaccgtttcatgtgtaagcaccattgaaccaatttttaaagcacatttgcagttatcaaatgtttagtgtgtcctcaagtttcattgatttgtttgcctttaagcaagaaaagagtaaagtgtattattttcccctgcttcttttcatatctgaattg

SEQ ID NO: 97 - DNA, 500 bp, Homo sapiens
  source 1..500: mol_type = genomic DNA
tcaaaaaatgttaattttggaagtgcttttaatcactattttccccaacagactagaatggctccatgaaatttgacaattaagtaaggaaatctttatccccaaaagaagcacgtatcttaccctctaaactgcatgcaaagtaagggtctgtgtgagagtattttccccaaactcctaatggacatggcagacaatgtgtagaaaaatctgagttttgaactgaccaacttcaagtcttttaaaatctttgggcaaaaaaaaatatcatgtagcagttaaaaaaattattgacttacaaattatagaaaagatatgttatctacaatatatgccaggtgacccattaaatttaaaaaatgtgtgcgaatgagtaactacattaaaactaccatcttggatcttggtgctttccaaaattctgaaatcactattaaggagggaccataccagatttttttgttgttcttttccttggagaatggggaagaagttggaaa

SEQ ID NO: 98 - DNA, 500 bp, Homo sapiens
  source 1..500: mol_type = genomic DNA
aaaaataaagtaagctaaaacaagattcccagataaatgcattggcaatagatcttaactggtaaataaatgagactatattcaatacaacgctaatcttttgatgttgatatcgtatgaggcagccagacttttccactggggtaagggcacgtgggatggggccactcccctagataaattatagaattgaatagagccgtggtccagcattatttgccatgctcttagatttaacatacaccaactttcagtcccattttttgcccagagtgctgtgaaaaccaacaaggaatcaaatatgtggatctgagcaaaaatgttaaaactttcgtttcaaaaagctgggaattcttaagatcaagacaaatgtgcagtcatggatgaaaaatcaaccacacataatctcagctttcaactgagtcatgtaaaaatacttgtcacgaagaaaacacacctttgtgatgatgcaagtgttaagaataacaagaaagaatgta

SEQ ID NO: 99 - DNA, 500 bp, Homo sapiens
  source 1..500: mol_type = genomic DNA
aatagtaaaggaaaatcttgcagcagggtagggcatccctgtatttccaattatttatatccaggcaacccatacttttcgccctgcctaccagtctgcttttgatgagtcgttaccaccctgtcattcccccaaggcctgaaattatttcggttttctggccttgaaaatgctttctgtgtttgatgaagtattactttgaagacccaaggtttccaaatattgaagcttctgtttattctcagccatatattattctattttaattttgaaaattacagttgtttgcaaaggctatttttgttgaggaggtgttaattattttctgggcctaaattgtgatagctggcctagttattgcaggtccaacagtgaactcggtttattattgctttgatttagctccactgagggactgacctaaaatgtcttttctttctaaagccagagaatttaatactgtgattggattgttgtaatggcttcctaaccagtctccc

SEQ ID NO: 100 - DNA, 500 bp, Homo sapiens
  source 1..500: mol_type = genomic DNA
gctagtctgtaacttaaggtccagaaagaaatatttacctattagccatcgtttcactcaagggattgtgaaatgcaaaagcacacatcaatttattcattagttgtcaagtgaggaggtaaacccctctttcagcatctctctgcatatcttagtttggatggtgaatgaagaaggaaactctctaaaatgtcaaataaggaaaagaccacctagaaatgagtgacagtaattcacagggatactaaaaataagaatcaagttgtaatatctgtactcagtgacacaaggtatcaacacaccttcccaatctaatcattttatcgtgtctacatggatcttccttatagcatgcttttttcataaattgtggaatattttttgagaaaagagagtgtaggtcactgaggccatttgttcttgtagctctctggctggcggggatccaagtgtgtatgaagatgagtgacagtgtgtggccagctttttcgctgctggtc

SEQ ID NO: 101 - DNA, 500 bp, Homo sapiens
  source 1..500: mol_type = genomic DNA
agaacactgctcaagtccactatcccagttccataactcaaattaacagaatagtttataatcaacataaatctgaatatttatttagtttaaaatatgttgttgacaatgtaatatgaacacaggcgataaaaaagatctattgacaaaaagaaaaaggaataaatgtttctagtatattctgcttggaaaactgccttttagtacatctaagattttcacctgcaagcagtaatctgaaccagtgttaggcttcgtttgatgaaatatctttttctgtttgaattgcttactacacctttgtaaacgaaagtaacatgtattcactgggaaacactaaaaaattcaaaaaagaaaataaagtgtaattccaccactcagggtaagccctattaacaccttggtacataccctttaagtgtgggtggttttaataacacgacatcattgtcaccaagacacttcatccactgtttcatttctgtgatcacagtaacatg

SEQ ID NO: 102 - DNA, 500 bp, Homo sapiens
  source 1..500: mol_type = genomic DNA
ttttatttccagaagagcaaattcaggcacaaagaggacagataaactgtcaacagtcaccagggaagccagcagaagggctgagagcaacactcttgcctctagcatcaagtgtgttatttacctgctgaaccctcgagggtctgagctggcaggctttcctgagggtgtggcggcagggcctgcattcttgtctctattgtcctgtactgtttacttgcaggatgtggaagcacagcatgtaatgtaataccagatgttctacgtgggaggaatttcataactcatacattttagcatgcttttttctaactgcgcccatctcctttcatgcagcacaaaaatgtaaatctgtttcccaaactactaccaggtcctggaatctaaaaggaaatactggtggttctttggtatttttcacttttagttgaagcacacatgtggatgtctagggtaacatcatgtggattcttcttattttttaaatggctcctattgta

SEQ ID NO: 103 - DNA, 500 bp, Homo sapiens
  source 1..500: mol_type = genomic DNA
tgtaatcccagctactcaggaggctgaagcaggagaatcgcctaaacccgggaggcagaggttgcagtgagccaagatcgcaccactgcactctagcctgggcgaaggagcgagactttgtctcaggaaaaaaaaaaagaattcaagtctgactgactaaagcctaagctcatcataaaacccaccacctaggagaaaatattaaatgatgcatgtcttggagaatcaacgtagttagcagaggagagctttcctaacacaatagaaaaatgcctttggacggtgtcggtagtcccctcagtaaagtgtctcacacttcctgaatctgatcactggtaataatgatgataaaaaaagatttcctttttttagcattggaaaaaaccctacccaaataatttttggaagcttgagattacattatttatctggttcaggttttaaaaatatttctgatttttttctgccaaaatccaagccctctttcctcatacagaaca

SEQ ID NO: 104 - DNA, 500 bp, Homo sapiens
  source 1..500: mol_type = genomic DNA
aaggttaaatcctactgtttcctggattttcaggttccccagtgaggatgcatgttcagaggcagactccccctctcacactttgggcacttaacggtttttctgctgtctcatggagtctgcaatggcaagctgctgctttcaaagggtctgtgaattcttttggttttcctgatatgtttctggagtagttcttggagcaaaagttcacggtgtgagtctccacatgctgtttctgcacgtccgagtgggagctggaagttagtccagcttcctctccaccgtttttttctttttgttgtttttaaaggttacaaggcctttgtttttccttctgtaaaataagtctttagaagtagtctattaattttattattaaaaactcaagtttttattacattattattgaatgaaaaagtaaaatatatgtgacagaacttctgatgtgctctaggagttgaagattgaatgagatatccttcagtgagctcatatattta

SEQ ID NO: 105 - DNA, 500 bp, Homo sapiens
  source 1..500: mol_type = genomic DNA
tcccctctgccttatgtcatttagctgaatcggaagaccaggtttgctccagtcacactcatctgacaggcctgctcttttcctctaagtagctggcaggagcatagctctgttccaggagggggacctgtcctcatgggaacatggcagttatggtccaagtccagctggccaagaactcagactgtcctctcctgaaggttcccccacagaaatcaataagagcccacctccagacagtggctggcctcagatctcagaggaactcaccatcctcttcctctccatcatcctctctaagcttccctgtctttgcctcagccaaagtccaacccatcagggacagaagagtaattgatgaaggccttaagggatatcaaagcgctattgagcaaaaccacaactcaacagccgtgcaggtgcttcctgcggcagggagggaaagaagtgtctttagaaagccctaaataactctaggcagggatgtcagcttgacaaat

SEQ ID NO: 106 - DNA, 500 bp, Homo sapiens
  source 1..500: mol_type = genomic DNA
gactggtgagaaatagccctgttgttctctggtgtgtgattcatccaaggctgtgctggggtggggggacaaggcccagccgtgagtcccaccgttggtcacttggggccgctcttcagcttggctccaagatggataagaaggcacttttgttggtgctcttggcctctgtcactttgaccttgttttccagtggttttatttagcggatttgtgctgatttggtttgagccgcattcagaggaggatagcaactgtggggagactctttctaagcatccgaaggcctctctccctttgatgttagctcccagtgcttcttgccatcataacatcaaagaccaggggctgctcagggcagaggcccatttcatctccctgttcccagctcctcaaagagctggcttattgaaatgcttgtcacgtgttgaatggataagtgaaaatatcccgagaccaagggatatgacatgacagctagtttctagacttagcgctgg

SEQ ID NO: 107 - DNA, 500 bp, Homo sapiens
  source 1..500: mol_type = genomic DNA
gttattgtgtataaagctgctatgaacatgaatgtaccttattttgtttttcactgaattggctggttcttttggttctaccatattaacacctgcattttccagatttcccatctccatttaagcctggaaagatgtgcctttaggatctggtgcttttttctccagtgtataactttatatgccctctgactacagacatgggcgcaaagctgcatgggtgatgaactgtaacgggctggactccagcacatcccgcaggaatgtgtaacatgacttagacaacaatgtttgattctacttcccagcagaggaaaactaagtggggcgggttctataggatcattcttagccaccaagtcagggtttcacctcagtgtgaaccatcctgttgtgctctcaggaggagactgccatgaagctactggaagcaccttcccttaccagctccccttccagggatctcaaaaatgctgccgtggaagctgcctctcttacaa

SEQ ID NO: 108 - DNA, 500 bp, Homo sapiens
  source 1..500: mol_type = genomic DNA
gtgaggaaggcaccccaaaattagctgtcattcccttgtggtacctttactgtgagtgacgcactgacgtgtgctataccttttatggaggctcatgcagagtactgccacctaatagcaggtgcacacacaccaacatgcacacacacacaccccaacatgcacacacacacacacacatgccccacagaaatctagcagcctgctgacctgaaacccatcctccgagactcagggccatgcaaaagctcccttaacacgactctattttctatcagtcaaagaaaataaactctcctggggcatatttcttcctcccaggtggtttcatgaaaagagagggtgaatctctcccaaaccacacaagaacttgtgttttcacaagaaggggaaaccgcaggggggtcttctctctgggtccctagcggccccgggagacccaggttttcccaagagccaacagctcttccctgcatgcagagctggtcctgggcagatga

SEQ ID NO: 109 - DNA, 500 bp, Homo sapiens
  source 1..500: mol_type = genomic DNA
aactctagttttgcttattccaaggtttcccatgctagactctacccatgccccttacgtgtgtattttttaaccacttaagagatgtgccaaagcatgtatcaatttttatttttcagacaattgaatcagaacttagtcatccaaatagatgttgccactttgaaaatattcatcttgggggattaatcacttccttcaatgcaaccactgcccatcataatttagggattcctctttgtggtttgccctcagtgtatgcatcacccactgttgaacacggtagcctacagcaatgtctcagaggttttagaacatcattcagaaccatgactggtgattgcaggttactaagagcacatacatagatattttgtagttccacaatttacacatctccagctgtcccttgttgagtgaaaccctttctctcattatgctgctctaaatccaaccaattccagtgatggcaaatggttgctctgtgaaagtgacttttc

SEQ ID NO: 110 - DNA, 500 bp, Homo sapiens
  source 1..500: mol_type = genomic DNA
ttcttaattttatttaaaaaaaaaatgctctgcaaacacaacttcaagacatattccagccactgtccaccctgccccacttcttagcagattgttgtccctaaggtcctcctatatagatactctgtagcggtcaccatctgtgctagtttctcagctgtaaacttggaataatagtaacaccgacctctctctcccagtagtagtggtgtggggattgactaattaagccctgtgaaatgccttgaaaagtagacaataggattctctccctgtcagaaagaattcacactattcccccaacgcctgacccgagggtggcggctgtagctcatgtcaccctttgctgatattttgtcacacttggacaaagggctctggagtcaaagggcagcttaaaccacacacccaatatcatgcttagaggaattcctgggaactggtttggtgttgacaattgcccactgctctgaatcacttcctttcttcctgcagattga

SEQ ID NO: 111 - DNA, 500 bp, Homo sapiens
  source 1..500: mol_type = genomic DNA
ctcttttcctgatttttgctcccagacaaactgggtgtgcatgtctgttgcgggagagggaccatggctctggccccaggcttgtatttccagatgacatgaggcctgcaatgcttctttctaatgtgcaccaggtagagataccttcagagcttcctcttcctgcccctcacctatttcctaatcttggctcaggtttcattgtgatattgatcaaccttaaggaaatccttgactagtaagcagttccaccaagatgaagctggagaaaccagagtggctcagtgctcaccacctacataattacccaggaatgttgtgtgattaataagttgctgtggtcttggtgcaaacaggtccctgaaaacatctgggctttccgcagatggtttactaatccacatacatcactgacaataagctctttacaaaaccctcttaaagtatattggatgtgacaggtttccagaatttttagaagcagagatcctaggtttaac

SEQ ID NO: 112 - DNA, 500 bp, Homo sapiens
  source 1..500: mol_type = genomic DNA
ctttaagatatctgtcttctgattatatggaggtggtgtaggccaagactcggaaacatgcagtattgattttggtacaagaaacaactctaggtactctgaggagtttggcacagaggttcaaaaaatgagccttagttctcagtaagtcttcacactacagcttttcttttttaatatttgttttactgtgccagactctacagctctgtcctcaaagagcacataatctttagggaaacttacaggagaacagcaaggtcaggagaactacaagtagttccttatatcttgatgacagacccagatacagattttattcctgccatttactagctatttgataccggagatgacgtttaactttctttgctgcttcatctacaaaaggggggtaattatactaatacctatgaaagaggggcattttcaggcctaaataacatagcatatgtaaagcccttagagttttgtcaatgctcctacaggaatactgtagt

SEQ ID NO: 113 - DNA, 500 bp, Homo sapiens
  source 1..500: mol_type = genomic DNA
atcctatccatagtgaggttttttcctaccttaaaatatttatttcataaacatgttttcatctagagtaaagtttaaattagagtagatggtaatatgttaggacatgtccaagttctaaggatgtacatgaagtgaaaccacaaaaggaatggttttattttactagaaagaaaatgaccccatttacataagatgcagggctagcccgcgtttccatggatagcagtacttgcactgaaccatgaagctattgtgctagggatgtacctttggcttctttcttagatgtacttctgagcttagcacacaggcctacagattcatcaacatttaatggtaacagacatactctggatccagcaattgcattttgcccagtacctgcttctccaagggagggaagaattagaaagccaatgtaagtgggctttctgcctcaggaaaaaaaaaatgtgatttttggtagagaagatttgcattcatgtttgattattaga

SEQ ID NO: 114 - DNA, 500 bp, Homo sapiens
  source 1..500: mol_type = genomic DNA
tactatgaaaagatacattaaatgtagaataaactgctacttacaaacaagtgcaaagactgtgttttatttcaattttctttttttttaatttatcttttattttaggttcagtggtacatgttcaggcttgttatagaggcgaactcatgactcgagggttttgtgtacaggttattttgtcacccaggtacaagcataatactaaatagcttttttttggcggggggaacctctccttcctcccatcctacaccctcaagttggccccagtgtctgttgttctgtttctgtccatgttctcgcattacttagctgctacttataagtgagaatgtgtggtggtgtttggttttctcctcctgcgttagtttgctaagaataatggcctacagttccttccatgttcctgcaaggacatgacctcattctttttcatggttgcatactattaaatggtgtatatgtaccacattgtctttatccagcctatggttgtt

SEQ ID NO: 115 - DNA, 500 bp, Homo sapiens
  source 1..500: mol_type = genomic DNA
catcttaaattcccagtttttgtggaagggacctggtaggaggtaattgaatcataggggcaggtctttcccatgctcttcttgtgatagtgaataagtctcatgagatctgatggtttaaaaattggagcttccctgaatgatctctcttctcttgtctgtgccacgtgagacacacctttcaccttccaccatgattgtgaggcctcctcagccacgtggaactataagtccaaaaagcctctttcttttatcaattgcccagtcttgggtatgtctttatcagcagcacgaaaatggactaatacataaaatataaattattcatccattcctctacctgagcatttccataaatttgatgtttgttcttgcttcaattttagcagaattcatgttgttctcatagggactctttttaaagctgatgttttagtcttatcagtgtcacaaactcagtcttgttgaggcatgttataacaagttagtacaagtttatt

SEQ ID NO: 116 - DNA, 500 bp, Homo sapiens
  source 1..500: mol_type = genomic DNA
tggccgctcagctcacccgatgccccgtgagccagccccgcgccagaagccgcggtggcaggaaggtttgatcaaacattaaataacgtaatgtttgcgacaaggcttatctcacaagtggaaaagaggacctcgcgagaattagaattcggctgctattttaaaaaatcaattaagcttgcggtcttttttgaaacagctcgaaaggactgcgtggctatcatcgtggcgctaagactgagatggcaataacaccgatggcagaactgtaccagtattaattgtcatcacctttatcatcccgctggccaccaaggccgttcgaatggggtgggaaaggctagttttagccaggatcagaagccccagttccaacttcacggacgaaaaactgcgaaagcctatcaacttgaaagatgagtagggatacttcacgcaggtgccaggtgctatcaggagaggccggggcggcggggcagaggcagagggcagggatcgct

SEQ ID NO: 117 - DNA, 500 bp, Homo sapiens
  source 1..500: mol_type = genomic DNA
cactgggggccatcccgggcagtggcctgccctccgaggcccgcgggacccagcccagagctgaggttggagttctccgggccacgttccgggtcgcttaggctcggagatttcccggagaccgtcgtcctccctttctgcttggcactgcggagctccctcggcctctctcctcctctggtccctaaggcccggagtggttggcggtactggggcccgtcgtcatctctgcttctaaggcattcagactgggctccagctgggaccggcagaggaggttctcaaggaaactggtgggaaatatagttttctttcgtctggtcgtttaatttaaatgcaacttcccttggggacattttcctggacgttaaccagaccaccttgagatgtcgttgatgacctagagacccagatgatgcgtcccaggaaagttcactgctgactattgtcactcttggcgttatatctatagatatagacctatgtacatatctccaccc

SEQ ID NO: 118 - DNA, 500 bp, Homo sapiens
  source 1..500: mol_type = genomic DNA
aagtgtgagaggtggaaagtctgcctctgaacatacatcctcacgagggagcctgaaaaatccagatcacatgggagggatttaaccttacctagagctgaaatgaatttagggagtcgagcaaaatataaaagtagaaaaatcagtggaaagagccctggaggcactcccggtccccagggaagccatttctgactttatcttacaggggtttttggggagaattgccagtagaattggagaaagaccacagggaagaggaaacttccaagtgaactttgtaataattttgaccaagcgtgaattttccagggcagaatctaggagtgggagggcaaacagtaagtatagataaaagcaaagaagtcacagcagaaagcaggtgaagccttgaaagtcctccttcctttctcagtggggaggctattagtctgggacaagttcccagccctgctcaccagctgcctggatataaactcggctgctgggggagcacagtg

SEQ ID NO: 119 - DNA, 500 bp, Homo sapiens
  source 1..500: mol_type = genomic DNA
aaagtgagactggcctttccagctttgtgggagctgggtgaggcctgtctctgccagcttttctccacttccttggtgacctgtaggacatagaagaggcatccataatcccctgggaaaaactccattgtcctgaaaaagacacctccatcccccacagtggctgcaacaagccccgcccaatgagagtctgagcccagacacacctaaacctgctcccacctgatggtctttctctacctgcgctggtagccagagacaaaagatagactctcttgggagctctagggccctgcccaacacctgattctccttatactactgcagctgatgctctcttgaaggttccaccttttggctagtggccagccaacacaaaccattacagtgactcataatagaacaacctgccccaagaaaggagtaaacaacagctaactccaccgcttgtaacattctggctaacaagaagtcctcagtctgtccacatgacaacttta

SEQ ID NO: 120 - DNA, 500 bp, Homo sapiens
  source 1..500: mol_type = genomic DNA
gggcagtggaaagaatcatgacatgtgaaattccttgaataaaaatttattgactttaagtaaaaaaaaaaactgccagcttgggacatggattttttttaatcaatttttttttttaaatattggaactactatttgtgaagctgggtggaaccttggaatgcctgttagtaggcttgctgggaaattggttatagcaaccagcatagtaaagaactcatagtcagacgtaataaatatttgctgctgatgagtcattcgtactggaaaaagtgaagcagacaggaatatctccgccaaatgctgcaggttatcagagtggccttaaccaaaatttccatgagtaatgttgcaatcttcttaccatggcttggtaagacctccaggaatgataatgccttatacgagtgttctgttttaagtcctccaaatcttccatagacagtatgtagatagaatctcaggacaacctggtagagaggaggaaactgaagttttga

SEQ ID NO: 121 - DNA, 500 bp, Homo sapiens
  source 1..500: mol_type = genomic DNA
tttctttaaccagatcttttttttttttttttttggtctttttctcatttgatctccttgaaaacaatggtttttttccccccataatcttggcttcatgatctatatcaaatgtttaaaggaagtgttacagaacaagaacatcaaggtatagaagatactagaatactttcatagtctttagaaatctgataagagctttcactgtaatttgtatctgtggaaaatattttcatttcattgtacaattgcatgtgcgtactttttaacaatcatagtatgaagtggaaacaaatgagaacaatcaaaaagtagaaagtagaaaatcagtgtcaaaattaatttattgaatacagtgtcgcaaataaagctctgaagaagaaacccggtgtgctctaccaacccgagctttggggttttcaagaagcattgtcagcttgattatttccttgtttgtgaagctgtgatggtagcgtcaccatttgctaaatggtttgctg

SEQ ID NO: 122 - DNA, 500 bp, Homo sapiens
  source 1..500: mol_type = genomic DNA
tgaagactactagagtactactgtccaggttacatttgaaaagcttctttgccaatcctcagcgaatgtcaattgctccctgctgggctccaggtctgtggtaggagaatgattttcagttttctatctgtactacctgtcacttttcttttactctcacggcttttgatgtagttttattctacagcttcctgtgtcaccatgtgtcgcttggccttttgatccactgattaatactcataacattccttatcccacgcactctaaccggatactggcgtcacttcagaatgccttcctccctccccttttaacctttagcatttcctctcacttctccagtctgctgtcatgtgttatcaatggctcatctggggcgttttcttaccacttttacaaccgtttctcatgaaatctttttattctccatctctcaacccccgtaccgttacacgccccctgatcctacctgatatccatgtaaccaaatagcccgtttc

SEQ ID NO: 123 - DNA, 500 bp, Homo sapiens
  source 1..500: mol_type = genomic DNA
aagtgtaatttggagaagatttgcaaagacaggcacgtagtgaaataatttgatttgttcagtaaacttggtttcagttattcctttccatgagttgttttagaaccccttcaatttctttgtgatttgacaacagctttcagcccaatgaagatatgactcttaggcattgccaggaattcagaattggtttataatattgtcgcttaataagaaaatgcgttcattggcaggatataaaatttatgggcttcaaatggatttctgtttgtagttttagccctctgtgctcctgccattctcgaggctatgagtaaggttttttaattaagtcaaattgaattgaatgagcttttattgaacgcccactctgtgccagacaccagctccttaacccttgcactgccctgtaggtggctatggggagctgagccagaggaggttttgccccatgctcacgatcattcagctggcaaacctgggaggtgggatttgaagtt

SEQ ID NO: 124 - DNA, 500 bp, Homo sapiens
  source 1..500: mol_type = genomic DNA
gacagggtttctccatgttggtcagcctggtcttgaactcctggcctcgtgatccactcgcctcggcctcccaaagtgctgggattacaggtgtgagccaccgtgcccagacctaggctttcttattagagagttccctggctcagcttcatcattgaccttggaaatgttctgagttcaatttccttgtctgaaaaatagagataaaaggagtatctactttacagggtgttgtaaagattaagtgaagcaatatatgaaaagagcttagttcaatgcctggcacatatcaagtttgacaaatattagctatcactattattaatgggtgccagaaaaaggacgaggtggggagtgttgtcttgccccaggaacccagctgggctctgtgccacccctggccctttactcaccagtaggttatctttggtccaggcacagccagtgacccagtcacggtgacaggcagggaaggagtggatcaaaacaggggttttggg

SEQ ID NO: 125 - DNA, 500 bp, Homo sapiens
  source 1..500: mol_type = genomic DNA
aaggaagagttgggtgaatcttccacagcccctaggtcctgtcttctcggccttcgtcccttggcagcttttcaacctctcagcaggccacaggcgcacgtggctggcagctccccggcctccggctctgacagtccgggggcaaccaggcctgcagttctcgaggaaacccccagccccccacgtctcgttctggaccaggaaccccctccccaacaaccgcgcagcaagtggcgactctgggagctgaactggagtggagctcgaagtggctggggcgggcaaagactcccgcttcactctgggacacaactgggacggcgcttcaacctctgcctgcaggcgtgcttctcgcgcgcaccagcaagctctctatccacctcgcctgggcctttgcagcgccctgccgcccaggctccagcgcctctactaccctagccccttctcaacacgcggctctgccttcttccccagtaccactgcactgccgaaaataagcc

SEQ ID NO: 126 - DNA, 500 bp, Homo sapiens
  source 1..500: mol_type = genomic DNA
tcccgtaagtaaacaggaaaacccaggtcatctggagcagactatttcctgagtagcttttatcatttgattcagaccttaaaatagtctcttgaattttttcatgctttttgtgggatatgaaaggacactatagttgttctagaatatatcccaagtgttgcagacaactgtactcttttgcaagactttccctgatcccttatgaagcacagaatagtgatggagtgatttttttaaaaatatgtgtcttaagccctggtgatatgccaggcattgtttggggaatgagtctacagtggtgaacaagaagggcaaagcccttgctctcaaaggcttgcatcctgatggggaaagcaggaattatcatgaagaaatatgataattacagttggcaagcagattaggaaggactttttttatggtcaagaaggttgagggcagggagagtgtctcctttagtgcaggtggtaaggcagggctttgctgcggagagactt

SEQ ID NO: 127 - DNA, 500 bp, Homo sapiens
  source 1..500: mol_type = genomic DNA
ttacccccatgctgtttgtaaaaccaccctttcaaaagaaatttatgctgctgcttcccttattaataaccagttgtgactctcattggcctaatcaaatttctgttggtctccttggcattcaaagccttccataaaccagccttatcatatttattcaaccataaaccttaacagatatacctattttacttaaactggttgtttatactttagacctgttaaaagacaatccttaaccaaattaaatataactcagtttaattgagcaaatctggcggcttcttgaacccgagtagtctgagagagactccattgcagccacgtgctggaagatttatggacagaaaaaggaaagtgacgtacagaaaacaaaatagaggtacagaaacagctggattggttacagctccgcatttgccttatttgaacgtagtttgaacagttggccccctttggccaaaactcagtgattgtcacaagagcagattacagtctgt

SEQ ID NO: 128 - DNA, 500 bp, Homo sapiens
  source 1..500: mol_type = genomic DNA
ctattatcccatgttgacattaattcttggcaaaggtggggctgtggtcttatgaagctggtcttacgaagctgggtgtaggtgtgagtatacgtgagaacgtggcactgtttgcaatcgtttgagctgaagctgctttacaacagtatgcattctttggggttagtgtgttgaaaatgtcagctgagtgacttccaccaccagctgcgcccctaacaccgtgtggcaccgggcttgggaaccacagctgtggcccgtcgtgctgtcatcgcttgtggctctgggtccttccccacctgttgctgtgtccgtcggtgtggcagggaccgccgactggctggaacatatatgctatttctgtgcataggatgtgagtaagtacatgccatagtaagtcagaccaggatatgagtcagatcatattataaagtgatacaaagaactgatcttcaaagcattctggaagcattaatccacgtgtcaacactattgtaagggag

SEQ ID NO: 129 - DNA, 500 bp, Homo sapiens
  source 1..500: mol_type = genomic DNA
ctacagtttgaaagacacgattactaagcaaaggagagacgctgcaagactcaggtgaacagaactggctaaaggcctaccaatgaaaacaaatgcatatggtgggagccaaaatccggaggccttaaaatttagaggtaaaaagaaagagttagcaggaccacatatttctccagcatattcagtcagaaatggagaagcagtgaaacacgggcagctcagaatagctgtggaacatgggcctgctttattatccatactatctgcagagcaacctttctggggctaaattaatggtcctcaactgactcttaaaaaaaaaaattgattggcactgaggtgtaaagacacacataaaaagacgaccatccacagcactatttgtaagcataaaaactgattaaccatcatgatgtccacaaatcagcaaaatgaactatattatgtcactttcatggaacccaagtagctattaaaaggaatgaaataatctgaatata

SEQ ID NO: 130 - DNA, 500 bp, Homo sapiens
  source 1..500: mol_type = genomic DNA
acaggaggcaggtccctaattggtttgaatttaatactcaaagtacatgcgcagagaagttatagtataagattcagaacaaatgggctaagtaagagaaaaaaatgtagcaattggaagatgaagaagagaggaatattcaaaaagatagcattgtgctcctttcttggtggagtgaacaggtgaggattatactgtctttatggattataggtacattggaaaatagtttacagttattatttgaaattcctctatagtgaaggaagtagtcaagataaaatgtgttttgtgacttttgatataggaaagtcagtaatagccatctcaataaagtatatgctcagctatttcatctttatacttagagattcctcaagaggatggttacacattagctctggatcagtgagagtaagaccaaggccctggaacagtaaggctttctcttgtaaagctcagttcccatggttctttgatgctttttctgtgttagaata

SEQ ID NO: 131 - DNA, 500 bp, Homo sapiens
  source 1..500: mol_type = genomic DNA
gaggattgcttgagcccaggagttcaagaccagtcctggtaacatagcaagactctatctctataaaaaatttaaaaaggagccgggagtggtggcatgagcctgtagtcccagctactcaggaggctgaggtgggaggattgcttgagcctgggagattgaggctgcactgagccatggtcataccactgcattccagcctgggcgacagaggaagaccttgtctccatcaatcaatcaatgaaatagtttctggcacatagaaagtcccgaataatatatagtagctacttctttggaacgtatgactgcagaatttatttttctcctttttttccttttaaatacgtaaccacttcagaaaactcaatttacaaaaacccaaattttggaagcgagaataagccagtgggtaataattctagttataaaatgactcactaaccattgttaggctctttacatttttacttgatgtcttaaaagcagtgatccatcca

SEQ ID NO: 132 - DNA, 500 bp, Homo sapiens
  source 1..500: mol_type = genomic DNA
agtcttttttttttgagacagagtctcactccgtcacccaggttggagcgcagtggcgtgatcttggctcactgcaacattcacttcccaagttcaagcaattctcttgcctcagcctcccaggtagctggaattacaggcatgcaccaccacaggctggtctcaaactcctgacctcaagcgatccgcccaccttggcctcccaaagtgctgagattacaggcatgagccactatgcccagctgagagtctttctgacaagtggtgctgggacaactggatatccacatgtagaagaatgaagttggatctctacctcacatcatatacaaaggttgactcatacaactcttagaaggaaacaacagcataaatcttcatgaccttggatctgacaattgttttataaatatgaaaacaaatgcacaagcaataaaataagaaataaataaattggacttcatcagaatggaaaacttttgtgcgcccaaggacactat

SEQ ID NO: 133 - DNA, 500 bp, Homo sapiens
  source 1..500: mol_type = genomic DNA
tgctgctttgatcactgtttgcactcaatctagtctttttctgcttgactttgaggtctttgtgcgcaaggtctgggttttcgccactctgagtccccagggccaggttcctgttgcagcctggagccggaaaagaatctgggaggaagaggttgggtgttggggccagcagactaggggacgacagatcctgccctgccactcatttgctgtgcaactctcagcaaagcacccaacctctccgagccctcgcttccccatctgtgaagtggggatcataaggcccatcctgcaaggtggtttccgcggtgaaaatagaaaacgaggcctgttcctacagcctgtgtgtcttgggaggaactgctcatcatctgtgatccttttttacctgattacgggaaaggggagtgatctgctcactgacccccggctgggcttttccctgccagtgaaatcatttgaaattgtccaaggaaatcaggaacctgagccgacgcaga

SEQ ID NO: 134 - DNA, 500 bp, Homo sapiens
  source 1..500: mol_type = genomic DNA
gggttgaaaaactacctattgggtactatgctcactacgtgggcaatgggttcagtcatacccaaaactcagcatcaagccacatacccatgtaacaaacttgcacgtgtatcccctaaatctaaaataaacgttttttgtgttttttttgagactgaatctcactctgtcccccaggctggagtgcagtggcgcaactgcaacctccacctccctagttcaagcaattctcctgcctcagcctcctgagtaactgggattacaggcgcatgccaccacacctggctaatttttgtgtttttgtttttagtagagactgggtttcaccatgttggccaggctggtcttgagcttttgacctcaagtgatccacctgcctcagcttcccaaagtgctgggattacaagcgtgagccaccatgcctggccaaattaaaaaaaaaaaaaaagaataaaacaaaaacatataacaattacttttaaaatactatataaggccgg

SEQ ID NO: 135 - DNA, 500 bp, Homo sapiens
  source 1..500: mol_type = genomic DNA
ggggagttcctttagcaattcctttccagtctgaataattatctcctaatttatcagtttcataaatctacattttcataaatcattctgcctaaggaggggcacccgtggactgccagtctcagatcctggatagctggatgccgtgactgttaacgtggcatcagaaggcagggagagaagttgaggcaggctgtctgcctgggtgatcagattccccactctgccccgccacaggcctcccaggacctaggctcctgctccctccctggagactgacggtgcctacattgtcccttgattgtttgctcttgcaagcgtagctattgctgtgtttggaaattgtctcttagttacttgtgtttttcttccgttttatgttgttgcccaacaatcaggcatctcccaggcttccaaggctggcaagagataagcagcctgtaataaatgttcctgccacaattggtgaaaagatgaatgtatcagctgctaaagaaaca

SEQ ID NO: 136 - DNA, 500 bp, Homo sapiens
  source 1..500: mol_type = genomic DNA
ttttcatcaccactcccccgccccccactgaacagatcacagtcccccatgtttctatagagtcttcataatgataacatctgtgtaatagcagcttccacttctctggtgttggacatttgggttgcttccagagttttgttattactgaacactgactatcttcttgcccagagttcatatgcttaggaacaatttgccggaatgtgcttactgggcaaagaccaaacatatggcattttctatattttcatactacttctgagaaggttctatgaattaccagcgatgtctaagtttgccagtttcaacatcatcttgctagctttacaagttgtcttcgttttggtgtagactctggagccaaattgcctaagtttgcattctacccctgccacatactataatagctatgtgaccttgggcaagttctttaacctttctatgccttatactccttatctactaaatggagataataaaagtgattatggccaggc

SEQ ID NO: 137 - DNA, 500 bp, Homo sapiens
  source 1..500: mol_type = genomic DNA
tgcagccccagcccacatagccatggcacactaagagcttctggggtcgggtcctctcattccaagtcccactcagtgcttcctggcaggtggccatcgtcaccctcttctggaatgggcaatggaacaatgccagcagcccgtggctgtgccctgcagctcggccctgtcattgaatatatatctcagggcaaggaaagcagattttatgtgcaggattacaacaaagataagcttcatcccttttggccagggcctgcctttcttctttaacctatgctcagccttccttgtgcttatagaatggtttaaaaaggcacagggtcttaagagtccctcaggagcatggggtgtcatcatgggtgcttgggggagctgttggctgcagggatttgagagccgaggtctttccacacccagggtggagtgtggaggactgcggttcctgccagggcaccgcttatgtaacacaaacccaatctgttgccagaatttaccag

SEQ ID NO: 138 - DNA, 500 bp, Homo sapiens
  source 1..500: mol_type = genomic DNA
gagcagaaaagcgcaaacaaatgcagctgcaggttggtttgatttaatattctccagaggatgctattactgtgtgttttagaggagataaaatgagagtttataggaaatatagctcggcctggtagacaaggcttgttaatagtgttttgtgtatgggaatctgaagaagaaaagttaaatgtgggcagctaatccaaccagggcttatttagaacagaagaaaggaagggactagaaaaaggggagtctcttttattgggcaatgtgctgcctgtgaaatcctcatgctagcatttatgggctcctttccccctaacttggtgattctgtaagtgtcagctgggccagaggagagggatgggagaggtgaagtgaggacgtggaggctgcaccaccactacagcagtgcacagaaggcagcacacagatgcctctacttgtgacagctgccatttattgaatgccgcaggtatcaggcacgtataggcaccctgtgg

SEQ ID NO: 139 - DNA, 500 bp, Homo sapiens
  source 1..500: mol_type = genomic DNA
aagcctggctctccctacccccaaacccaaatgctctccattgcaccacccgcccaccccagtctgtcagctgactcggatcaagtccagtgtctctctagcctgagctccaggaaggccacagctcttaggcgcatgacccacaccaggaggtttcagtctagacaggagctgggaagaacttaagcccctgggccaatcagcaggggaggaggcccagcctgtggttccaaacaccaggtcttactcagtgtccccaaccacaagccacaggtgagtcagcatgccacttcccgagctgggtcccactccacgccctcacttctgttcttagaaaaggacgaccaggcaatcttgtaaaacctttgcttcccattactcggcccacacagtcacctgtgtggcctctttagctacatgaatcttgctcaccaccttcagcttttcatgccagccagctgcctgccccttacacgttcctgtctttggccagacgcaat

SEQ ID NO: 140 - DNA, 500 bp, Homo sapiens
  source 1..500: mol_type = genomic DNA
attcacacttgttccctgtgtccaggatgtgattttgtacagcatctcaggtcagtagacttgggccagagggacctctcttctctgagtgatgttcctttgggcttaggggtcttataggaagagcccaagttgttgattgtgctcttacaacattttcagagaagggaacccagaactcccttcatacaaagcagagcaaagcagagttgcttgggttgaagccaggagggaggagtacacacttgtacacatatgcgccttcccaaggcagcaggctttggattcagactccctggtttgagatcccggctctgctgcttgttagctgtatatccttgggaaatcacttaacctttctgagcacaacattccttgtttagaaattaagataatttctactttatagggttgtcccagggcttttatgagattgtgaatataaatccttggcacagtgcctggcatgtagtattctttctctctcttttttttttttt

SEQ ID NO: 141 - DNA, 500 bp, Homo sapiens
  source 1..500: mol_type = genomic DNA
ttaattagggtcagaaccgtactggggatttcctataccctaagtttgttaagtgattacatcggtctggggaaaagggatctgctcagagtgattcagtcaactttcttagtatcgggtggtgaatcgcatttcctctctgctaccctgtatactgactaatgggtggcgtatggggggtctccaagaggtgtgtttactccaattcagaagctataggatttcagtaggccttggcctgttgggcaatgtgaggtttcaatctttctctctcaaatgagtggggctcttatcagttatgaagggacttcccttgggacttgtcacgacaccatacagcagagatggcaatttgagggcagtttcttgttctgctttgccatcttggggtggctctgaaaagctttctgaacctccgacaaaagaaaaatgttcacaggattgattactacacacaattcagtgaagacaactgggcaacctgaatcaaatgttgagat

SEQ ID NO: 142 - DNA, 500 bp, Homo sapiens
  source 1..500: mol_type = genomic DNA
tctcccctgagccatgctggaggccccagaaaccagccaaacactaaacaggcctggatccagggaaatactaagccctttgggacaggaaggagcagagagagggccaggccccagaaactcccttgtggtctggcaacccgaacccaggactcacactgctccctagagcacccaagagaggtgggaaccgaggaggccggggttctctcctctccctttactttcccacacagcctcattccctttggttgctgccatcttttcttgtgtagcctagggactccacacaggcccacagaaactttcacttccccctgaaactcaggttccaattcactgcctgcatcaaatcgctggtgctttgtgtttaactgaacttgggtaggaacaaaggttggggaaacctgacttacagggcaggggagattccatattctactaatgtcccttgcaaacaaaaaggaagcctgcaaagaagacaggaaggagggggcgtg

SEQ ID NO: 143 - DNA, 500 bp, Homo sapiens
  source 1..500: mol_type = genomic DNA
aagttaaaaggacaaaagtctttcctgtgtttcatacttgggcggtgagtcactaggaaaggatttggtttttagaaaaaaaacttctgatccctgggctaaaacagagagccccaaagagctatgttgatcccagacaagcacgtgcgtggattcttcaaagttcaggtcaactcaggcccctcctccttgcagtcagccctgtactcaaggttgctggagacatggcgcctctatttcctgcccaaagaagcccccttaactgggggccacgggttgagtggtgaaggaggcaactcacacctgaattatagtgggcttgtaaacctgaacagggcaagtcacaactttgggaggctgaggcaggaggatcacttgaggccaggagttcaagaacagccctgacaacatagtgagaccctgtctacaaatgaaaaaactagccaggtgtggtggtgcatgcctgtgctacttggaagactgaggcaggaggatcactt

SEQ ID NO: 144 - DNA, 500 bp, Homo sapiens
  source 1..500: mol_type = genomic DNA
ggtcacactggagtagagtgggcccttaatccaatatggctagtatcctgattagaagaggtgaagagaaatggaccccggaggggagaacgctacatgagggaagtgatgcagagccagccgcagcagcgagggaaatccctggaaggcaggaagaagcatggcaggctgccccctgcggctttcagcagcagcaggaccttgccgacaccttgcctttagacttccgttctccagaactgtgaaaaaataaatgcatggtgttttcagctgcccagtatgtggtcctttgtgatgacagctctaggaaattaatgccagatccttgctatgatgacgtaatggaagtggcactttacctctaggatcttcctccccaaaacccacaactccattctaatcatgagaaaaacatcggatacatttcaatagaaaagcatcctacaaaatacctatctagtaatccctcaaaactgtcagagctgggctgggcgcggcag

SEQ ID NO: 145 - DNA, 500 bp, Homo sapiens
  source 1..500: mol_type = genomic DNA
aggtctcctccccaaatgccggctccttttctttttttgcaaatctcacccacagcctctaccctagggcagaagagacaggcccaaggcaagtggagtgggaggaaaacaggaatggggtcgagacccagggacaccatcctggccttgacattcgccaaaagccgacagcacttcataggcaaatcactcagctgcccgctacctaaactgagtcagctgcaaagtacgaaaaacaggacggacagtaccccccaccccgatccccggccagcgtggaaggaggggtagagcaggtgagggatgaaaggctcctagccctggcatgtggcccaggacatgtgagagcgcccgtctctccccctatccgtggctcagagcagggactgtgtctgatttccttctgggtcccactcagatgggaacggcctctgcccatgcacatgcccgtggtgcccgtctggcctgaggtggcagctccggcctctgtctccacgcca

SEQ ID NO: 146 - DNA, 500 bp, Homo sapiens
  source 1..500: mol_type = genomic DNA
cctcagcctcctgagtagctgggattaccggcatgcaccaccacgcctggctaatttttttttgtatttttagtagagatggggtttcaccatgttggtcaggcttgcctcgtactactgacctcaggtgatccacctgcctcggcctcccaaagtgctgggattacaggtgtgagccaccatgcccggccttggaattatttaaataatgcttagaatgatgtttctcaaacttttctgattatgaaccacaggaagaaatacattttatgccaggacccagttcacgtaatacatgtataactgaatgcttatcctcactgcttgggctacactaatattttctatcccattctgtattgcatttaaaaaaatgctggctgtgactcactaaatggactataggctggcagttgggaaaaaggtctagacaacaagatagatgcctgcaaattcaggagagtagggacttaattcacttgtactcactgctgtccccc

SEQ ID NO: 147 - DNA, 500 bp, Homo sapiens
  source 1..500: mol_type = genomic DNA
aagttttgaccacatgcatacaaccagcaaatggttttacattctcttatacgaagaagacacttaaaaaaaaaaacaaaactgcaagccttcgagtggctaactcccctctttactgtgcagcttataatcatatattttttaaaaccatgaatggcatgggggatattttgctctccataggaggaaggcatcctacttctaggataaactgaaaatggcactgctgcatcagttcaatcttagcttgagtccagtgagattcctcaaccctaattttgtagctcggagcagattttagtgtggatgatatatatcaaggtccacctgggcccagcactgaaccagaaagaaaggaagaaggtattgatggaaacgacatgtgtctaggtttaaatatagggaataggaatgcccttctgcaaagcaccttacagtttatgagaccctttcaccattattattccattttatccttgcagccgtgtggtaggcagggc

SEQ ID NO: 148 - DNA, 500 bp, Homo sapiens
  source 1..500: mol_type = genomic DNA
ttatattgttatatcctatttactcgaggtcatacatgcccaggctggattgagactccgtcccaaggtttctgaatcccagttccatgctctttccacattttcatcctgcagcctgagatagtacgcagttaactactgaccggaggtactctgcccactcagatgagagagaaattattgatttaaaagaggtcattctgggagttctgcattccacttgcctagtgtaagttgctacttgtctggaggaagtaaatcatcaagctgtaagttacacaatgcatgtgtctttgatgtgggcatcaggcattattgactcattgatatgcgatacataccctaagaactgaaaaatgctttattgagtagaattgtgggcctgatcacaggaaatcatgtttttttttctcctaaaagttaaacactattaaaactccaaaatcatgactggataactaaattcatgaagaaagaattttaaaatgagataattacaa

SEQ ID NO: 149 - DNA, 500 bp, Homo sapiens
  source 1..500: mol_type = genomic DNA
ggacgttatctgtgttcctgattccatacacacaggaatgatgtatataggccattccaaaaaatggcaggtaaatgatgctccagatatgcccgtgtagaccctggcgacgaggcggcctgttctgcactgttctcccggcagagccacccggaagagcccagcctggtaattaaaatgcactggatcaaagaaactccacacacacgggcttcctccttctccccttcaggcccctccttcaagtaccggtttcttaaattctcacttataggattttggagatcaaaaagaggcctttaaacttaatgaattctccgcttcgtcccggatggagccgttccgcacctttcagctgttcccgggaatgatagggcagctcagtgccgagctcgctaggtaattctcgctttctagaactcctgtgaaagcaaagcagcccgcatttggaggcttccaattatacttcacatggtgaactgtgtaattagtttggaaga

SEQ ID NO: 150 - DNA, 500 bp, Homo sapiens
  source 1..500: mol_type = genomic DNA
ggggttctcctgaccccacactctgcctggcatctttctatggtgattcacaggtcaggagtgcactcgtaagcaaatggaagaaggtaaggagaacaagagctaattatctgagctgcttttgaaataaagtgatatcagagaagaaagtatatttggcactaatcatagacaggagaaaaatcccagccacccaagaagtagaacttttatatcattatattctcacatggaaacagggtttgacctgactcagtcagaatgacctctaactacaaaggtactagaaagctactcatgaagttagaagcaaagaagagggagcccgtcaaatatcattttagttacatcagggatctttagaagcaaggccatgaaatagaataccaagttctgaggcctgtgaagatcaagaccttaaaagataacccagtcatgtgttctggactccttttctccaccaggtgaggaactcagggctcaaccatccaaaaatcata

SEQ ID NO: 151 - DNA, 500 bp, Homo sapiens
  source 1..500: mol_type = genomic DNA
catacacagcctaatgtagaggacagcatataacttagcacaaaatgctctcacaagaaactttggcaacaatggatgtcattcatgctcttttatccatatgtgaatataataatcattattaccttgtgtttccttgaagcttcacttggatatggttgtttcattctcttgtcctaacttgctggttaatgttgctattatggagcagctggtgacccaccctgtgtagtggggcataggccctggtgttaaaagactcttctttgggttatctaccttgaggaggagatacatttgacattacaggtgacccttaaacaacacaggtttgaactgcgtggattgtcttctgcctctgacacccctgaaacggtaagaacaacccctcatcttcctccttaacctagtaaggtgaagacaaggaggatgaagacctttatgatgatccactttcacttaatgaatagtaaatacattttcttgggccaggcacggtg

SEQ ID NO: 152 - DNA, 500 bp, Homo sapiens
  source 1..500: mol_type = genomic DNA
tgtgagagagagagagagattggagggaggaagggagagggagagagatttcttttaattaaagaactctgaagtttttaagtttaaaaattactagcctgatcatttggaataatttaactttttcctccaccactatgcggtattgttctttttcgtaactttgcctagtgtgtcatttcttcccatctgcatgtctactttttcagttttcttacctttcaatttatgtgctgctggcttctttgtgaactattttatgattcccttcctacccctacctcacccccttcactcctctcaaattgtctctgaattcctatctcagcccagctatgtctttcttgtgtcacttatcacattctaccttcttttaaaactatttatagacttttcttatctctccaggagtctaaactccttaagaagggggcttaaaaatgtttgtattttcaacaatgcctgcctactgttacacatactactcatgcagtggatac

SEQ ID NO: 153 - DNA, 500 bp, Homo sapiens
  source 1..500: mol_type = genomic DNA
gcctgggcaacagagcaagacaccatctcgcaaaaaaaaaaaaaaaaaaaaaaaaaaagtgagcatctgatacacatgcaagaatttcacaacattgcattcactcctccagaaacaaagatatattttaaaatgctttcttagcatatgtgctctggttttctagcagatactctgtcaaacttttgataagtgaaaaatttaccgaagaatttaaaaccaaaaacagttttttaactttcccacctgaaaatattgaccattttctaatttattttcattataaagaatattggttatcatggttgctcatgcctgtaattctagcactttggtaggccaaggcaggcaaatcactcctgagcccaggagttcgagaccagcctggacaacataatgagacctccctacaaaatatttaaaagttagccaagtgtgacagtatgtgcctatagtcccaggctgaggtggatcacctcattagtgagccgtgattgtgt

SEQ ID NO: 154 - DNA, 500 bp, Homo sapiens
  source 1..500: mol_type = genomic DNA
gcccggggtcgtacctgcttcacgatctcctaccgcggcgggccgcgtacctcctggatggcctcttagacgttctctgagtcgctgcgcgacaggggcagcaggcacacccaggagcccgctacgctgcaggccttgaagctgccgctgcttccgaggttgccggcgggaggcgagacgacggcgcgcgtcaggtcgtccagggactgcgcgggccgcacgggcgccgtgggccgcaggtacaggcaggcgggcaggccgggcgccaggctgctgcgctggctcgcggcgccgcgctgcgcagggccgcacagggagctggccccgcctcggggctccgctggggggccgttgggggccgctgccacagccgcgctcacgaaccggtagtcgtaggcgagcggctcaggggctgcgggtcccgatggggggacctggcggcgcgtcagcggcagggttgcccagcgcaggcagctcgcgcacgtactgcgcgggcaggt

SEQ ID NO: 155 - DNA, 500 bp, Homo sapiens
  source 1..500: mol_type = genomic DNA
agaaggggcggccgccgggcttgcgccgcacgtgccaccaatgctcagtgctctgtgctgcgccgcagcggccggtagcgctcattgggcgggatggccacgcggcgcccgtccttgccggtgtactcgaaggggtgctccaccagtacgtacacgtccccctccacatccgccgccattgcggccgcggcattttcctgcaggcaacaaggaagagggccgcggaagtcaagaccactgagcccggaatagcccagcactcgaggagagacttgggttcgagtcccgatgctgcacttgccgttcgccttcgggcctcagttttcccatttctaaaatgaggacttgaataaaatcacatgcaaggcttccattcttacactcagtgctggaattaggacaacctcttcattccgtggggttgattctaagatttcagcctcgcttcagtcctgcggtggggagattgtgggtagtcttggtccaaatcgactgcgagg

SEQ ID NO: 156 - DNA, 500 bp, Homo sapiens
  source 1..500: mol_type = genomic DNA
cccgcactagagattacagcgtatgtacttgtccctggtttctgcgcatgctctgaagtattgccccaaacggcactgctgggatcataattagattggacagcgggttgcgattaagggctacgcggtgaataaaacagctcttaaaagttgcataggaagtcctcacaggagaaaaaaatcaagtggtttgccaaaccactcattatacccctcccctttagccctcaacttcctcagaattcaattagtagataagagcccctgacttgcttttaacctctgacaacttatttagcccataaatactggggttgctgactcatctctgcacacttctacaaatgaatgttgggtgggtgcatggctgaaacctagatttgctaatccccgtagggaaaacacagagcttcaatacttaaagaccattgctcattgtagattttactgaatctattccactgggctcacaagagtcactcacaaagggctaagaaaaa

SEQ ID NO: 157 - DNA, 500 bp, Homo sapiens
  source 1..500: mol_type = genomic DNA
cgggcgtggtagcaggcgcctgtagtcccagctaccggggaggctgagacaggagaatggcgtgaacctggaaggcggagcttgcagtgagctgagaccgcgccactgcactccagcctgggtgacagagcaagactccacctcaaaaaaaaaaaaaaaaaaaaaaaaaaaaacacagaaaatgctcacatactctaataattagaaagatacaaaatagcacaagatatcacttcacacttcttagactgaaaaataaaataaaaggtctagtaatacttattactggagatgatatgagggaaatcacagcactcacacaccattttgaggggaaaattagtgcattaactaaaagaacaatttgctcttttccctccaggaatcctctctcaaatgtcttttgacttaactcctcaggaatcatcttctaagacgttctcactcatctcccagatgatatttgcattataaagtccacctgcaacttttgtgcattt

SEQ ID NO: 158 - DNA, 500 bp, Homo sapiens
  source 1..500: mol_type = genomic DNA
acccagctagtgtgtgtgtgtatacacacacacacatatatagtagagacagcatcttgagatgttgctcaggctggtctcaaactcctggcctcaaacagtcctcccaccttggcctcccaaagtgttgggattacaggcatgagccaccgtgcctggccttagcctgtgttttgtgaggtggtgagttccctgtccccagaaggatttcagcagggatagcattcctcacgggactgagtccctgtggtgcaatcagagaaaagagtcactcacagctggagttggtcatttcaggttcaagtccaggcgtgtctgtgtgaactcaggagcagggtattaaacctctctcctcatctctgaaatgggatttgggtctccctcaaaggcagttctgaggtcaccctcaaaggcagttctgaggtctccctcaaaggcgagactgtgtgcagaatgtgtgcagacattttcatgccccagtctgactcatggccctgtgc

SEQ ID NO: 159 - DNA, 500 bp, Homo sapiens
  source 1..500: mol_type = genomic DNA
gcttacactggggctgagtcacccgacaggaagttcctacaaaccttactggcatcattgaaaacagacagctccatggtaccttcaaagtcctgttgcaaaacagacctcaaacattcgtccagccacggttcagcgttgtggactgggaggataatagactggaattcaaaagaaatggattaacagaagtgtgaaaacttagttccctttccatggctctaatttacctccccttcaccacccgcacatatgccgtgacaaacaaaaggtgtccactccttttctccaggctcttaacatgcttgtaagattctttacgtcttagctttccctgaactgccttctacatgtttttgaaagtgaaaaaaaaactgaaaggactttgggaggccgaggtgggtggattacaaggtcaggagattgagaccatcctggctaacatggtgaaaccccatctctactaaaaatacaaaaaattagccaggcgtggtggcagg

SEQ ID NO: 160 - DNA, 500 bp, Homo sapiens
  source 1..500: mol_type = genomic DNA
aaaaaaaaaaaacttgaggttctcgatttttcatttatttgaagatagcatggaattctattaaataaaaaaatgatttgtagaagaaagatctcttccaattgaaaagtgatttttgagtacataatttatattcagttctgtgctaagtatcatgtggggtggtctattacgtggaccagtggactaggtattatgtggatctgtaaacagatgtgcaaaaggaatcaaaatctcaaacctcaagggttttggctgaaattcaagcacggcatgctgagccatctccaaagaagaacccaagtaaatttctgtgaatgtttttcttatcagctcttctaaaaagatgtaactctaaaacctaaggaaacattcatgatgtcagggagtttccctgagaagcagagatttacctcacagagttctgctgatggcaagccttgctgatatcttgacttctgctgttggaaatgcattgcaagtgatgcttagcttccaga

SEQ ID NO: 161 - DNA, 500 bp, Homo sapiens
  source 1..500: mol_type = genomic DNA
ccctctttgtcacctagccaatttctaatattccccaatctcttgccaatgcaccggtcactcatatcagctcatggtcagcctcggcacagtcattcaacatcatccacctactgggcgtctaggtgccttgcagtgcaccaggcaccaggaagtgtggtgatgtcataagataatcatgggaaaattataagacttgctggcatctccaccaaaaatctcttgtggaaaagatgctggagttgtacaaaaatcagaatgtgtagaatctgcaaattcctgtgtataaatcctatttgtttgcaaattaaattgaatttgcttggcggtgttttttgttgttgttgttgttttttaagaaaatgtcatagaaagtagcctgttagtgtttctgatgaggaaagaaatttgcccataatcctggaaatggtctcctgctcaggcaggcaaagcctggctagaggcagagatgccttccatcccttccgcacacttttcta

SEQ ID NO: 162 - DNA, 500 bp, Homo sapiens
  source 1..500: mol_type = genomic DNA
tgtccaaggcctttcccattgccccagttgtgatttatagaaagtcataaatatagagcagatgaaaccccagagccctcagagcccagctggttcaccccctgcctaccccacccccaaccagctccatgaacctccatccagccacgcttggacccacccatgtgctccatatctctgccgccaaagtcctcctccatggccaggaaggaggagggataaagagaaagagagaatcgatattcgttgggaaattggattgcagatacagaagtactgaaatattgcagtacttcccttggcatttcctcttgaccagagaaggaaataccagaaatctcataagcgaaccaatttgggcaatttttttatactcagtattcatacatttcacattttttttctccaaacctttgagtactaattcaaaccgtccagcctccaggccccctggagattcacctatcactaaatattgttgatttgcaaaacacacggat

SEQ ID NO: 163 - DNA, 500 bp, Homo sapiens
  source 1..500: mol_type = genomic DNA
tctaatttcagatgatgaatgccagctgtcaatgaacctataccgactgtgtttttgataaaactaatagtccaagcacctagaactgttacccctttaattgttgatccctcattttttaaatcataaatatgagtggctacctgcctccttcacaaggtcgtggtgagaagcaaattgatgccagtgccattttttccacctcaattccttgggttgcacaattttgtgggaatttcctgggaaaacttcaaagcaatttaaatagatctgtcccaaccatgcaattacaggagctgatgacgtttcagaaacagtgacaaagttcagaatcccattcttccatcctagatgggaaacatcaactttcctgatggtgagtttgtcagagtccattcccaagagtgggggtggggaggtgggggtggaggctgttgacaggcaatgatttctgtggagtagaagagaggaaaagagaaaaagaatttgttagttgtaac

SEQ ID NO: 164 - DNA, 500 bp, Homo sapiens
  source 1..500: mol_type = genomic DNA
tgtttgtttacttactacttttttgagacagggtctcactctgtctcccaggcttgggtgcagtgcatgatcatggctcgctgcaacctcaacctcttgggcgcaagcgatgctcccacctcagcctctcaagtggctgggactacaggcatgtgccaccatgcctggctaacttttgtattttttgtagagacagggtttcaccatgttgcccacgctgatatcaaacccctggcttcaagcgatctatggggcttggctttccaaagttctgggattatgggtgtgagccaccgtgtctggccagcttcttttattttataaacattatctcagcccttcttatacaactttgaagaggtcgacttcggactttgaaattaagttgctcaaatgttatgctagtgtgtatacgttcaggttttttgcaggaatagaagagaagggtggcaaggattaaaaaaagattaaataacttgcatctttctctcttaacagga

SEQ ID NO: 165 - DNA, 500 bp, Homo sapiens
  source 1..500: mol_type = genomic DNA
gctgggtggaggccaagcctgggcctttccagctgggttgtcagccccttggcacttcccacggacggtccgtcgagatttcctgacgatcaggatcccagaacatcaaggaccagagcaagactgactgtggtcagaggttccagtccagagctttcgtcttctgggaaaggaaactgggtccctgcatactgtgtgcttaaggtcatctgtctcccaagatgtggttgatttcaaagaaaacattcaggaacagggattatggtgtttacagaaccaaggcactatattcctgtgagcttcaggaaagaaaccaaaccagccttgctgcagccgcttttccagtccacccatcagcccttgggcatgcaggagtgtgagacctgccgggagggctagacagtgcccttcttggtcccacaccgtcttgccttcccaacgcagttaaattgacatccagaaatcttcctaaattgcagagattaagtaaaagctttcag

SEQ ID NO: 166 - DNA, 500 bp, Homo sapiens
  source 1..500: mol_type = genomic DNA
tggatcacgaggtaaggagatcgagaccatcctggctaacacagtgaaaccctgtctctactaaaaacacaaaaaattagtcgggcatggtggcgggcgcctgtagtcccagctactcagaaagctgaggcaggagaatggcgtgaacctgggaagcagagcttgcagtgagccgagacagcaccattgcactccagcctgggcgacagagtgaggctccatctcaaaaaaaaaaagaagtgagcttgctgctaagctcggttgtgtgtgagggggtggggtttggagctctgttgggtggtgacctcagtcctgtttacccctgcagaagaaggacccagcccagttcctgcaggtacatggccgagcttgcaaggtgcacctggattctgcagtcgccctggccgctgagagccctgttaatatgtaagactgatatggaaggcaggggagtgtctgaagtctgggagtcaaaacggacctggggtggtgtagagtgt

SEQ ID NO: 167 - DNA, 500 bp, Homo sapiens
  source 1..500: mol_type = genomic DNA
ggagcagagactgaagtatggacagacctttggggactcagaggcagggaaggtgtgacccgcatatgaaggtgatagtcacagggtgtaagaacaatgagcaggggttggggtggaggccccagagtagcagtcatggttggaggacttagaaatgggtggagccagggccagaggcccagaggaagcagagagtaggttgccagacccgagctggctcagggtgcctggggcccgcccctcaaataccctctaggacctggttcaagttccccactattgcttggttgtgagaaatggggccctggtgtccccaggggcagtcagatgactggcctgtttcaggtcccaggagcctgaatgtggattcagggaggcttgcaacagaagggactgagagctgggggttgaggtgagggtcatggcatggggaccaaagcaggctgagggccaggcttctaagcctcagctggcagggagcaggtgctttgtgtcctggg

SEQ ID NO: 168 - DNA, 500 bp, Homo sapiens
  source 1..500: mol_type = genomic DNA
ggacagctgaggccccaggttgtcctcaaacatgggcactggcaggttgacgcggcggcgggcaggcggcgcgctgggctgcttctcctgtcgccggaggaaggcctcgaccagttcctcatcatcctcactctccaggtcgcttcccaggaacttgctgcccaggtagctgacgggcattttgcgcaccttcttgccccgccgcgggccctggcggctcttgtctctggaggtctcgaagtcgctgaactcgctgtcgctggcgttgctgctgtcgtacgtgcccacgaccagccggggcggaggagtcaccatctgctgcactctcctcctcactcggggctccttgggctttttggggggctggggcgggtgcggggtgctcttctccatgatgcgggccacgtcctccagggtgcggccctcttcttccaggaactgggtcagccgctcccgaaattctgcttccttggtggcgggcttagagatgactctccaga

SEQ ID NO: 169 - DNA, 500 bp, Homo sapiens
  source 1..500: mol_type = genomic DNA
ttggtaaaggaaaaaaacaatctttttgaataattttaaaaagctcccaaagttccccatgaatgaccacaaaaaggcttgcgtgagagcatccaactccttccgtctcaattaactaggacacaaagagaagtgatgtaaggaggaaacatcacgagcccaggccccaaaaggttagccacaaatggagctatctctgcggaaaggcccgcagctgcccaagcgggagccaatgtattaggcgtgcttgcctgaaggttccagggcatgtggcagactcctcctcccaggaccctccactgtcctttcgcttatgtccctccctttgtctgccttggggctgctacccaaacatcaaggagcgcctcaagagcagctttttctatgaactctcactcccagttcaaaggggatgggttctatttcaaacccaagtggcccagccccacagatacccctgggcagaggtcaagggcaactctcaaaacagaatgcaggac

SEQ ID NO: 170 - DNA, 500 bp, Homo sapiens
  source 1..500: mol_type = genomic DNA
gttgcatacccatgaattctaaaacttcatcctcttttgtccctttcgagttaacattacagccacagtgacctttcaaaaatgcaaattaagttactcttaaaactctagttaaaatacttgatgtacataaagtgcttagcaaaatgaccaactcatactaagtgcttagtaaatgttagataagtattctccagaattgatgtaaattatttttaaacagtgcattcttgaaagcagtatggcagtcataaaaattttggaaccaaaacagtatctttttttaagctaaaaaaaaagttttaaatggtgtctttctatgttgcccagggtggtctcaaactcctgtgctcaagtgaccctcccacctcattctcaagtggctgcaattacaggcaaccagcctgacttaaaacagtatcttaaggtagatggtgattagcacatgtagtatgcttaacatttaatattataataagacatcacagcggctgtctcat

SEQ ID NO: 171 - DNA, 500 bp, Homo sapiens
  source 1..500: mol_type = genomic DNA
tgttttctgaaatatttgtcccagatagagcattcaaatcagaaggaagactgatttttttcagacacagaattaatcatgaattttttttttttttagtttgtgaggcaaatatgacttaaaccaaagacacagaactatgggagaaagtagcctctcgtttgtttttatgcatcctgtatacataaaaccagaccctgagaccatggcgagggagggagggaggtttttaaagccatgaatggcaaagcaattcagattccatgcaacccctgcccctcctggaaaggcattcactttaacgtcactacccacagcgttccagcacagaaccaagtcaggtaacatctgcacatagcagagaagtcctcggggaccaacctctccctgtggaatggcagcaacagacacacacacacaggaggaatgccatccttccagacaaagtccatgtcatgccattctacttttagccaatggtgaggaaacacatccaccat

SEQ ID NO: 172 - DNA, 500 bp, Homo sapiens
  source 1..500: mol_type = genomic DNA
caagcctcagatggaaaggttatttccaggttatgataacattattggatccaaagtcattgtcatcatttcattccacagaaagttattttgcactttcccctgggagcaggaattgaattggtggggagcagggcagggggagatctgaaacagcttccagctttttcaaaaagattttcatttcatcccacttcttcacagcacatgaaaagagccctcaaatgccctacatagcacctgctgtctgctcctcccacaagacttctttttctactcctctcttcttccttctcttttctttgctataatggaggccataaagaggacaggatcatttcagggggatggatgagaagaggaaggagagtcaggatcagaggacaggacccgttctgagggcattcccagggcagcacctgggaggctgcagggcagcagtaagttggataggggttgctgctcggatggaggttgtcagggccaagggtaggggaccc

SEQ ID NO: 173 - DNA, 500 bp, Homo sapiens
  source 1..500: mol_type = genomic DNA
tcctcacatctaagaactaagtaagaggacaaaagtacaagacacggtgcatgtgtggcgagtgaagtggagcagtgcattcgtgtcatcacccacccgaccccggctgcgctcctccgaccccgccgcctactcccgccgaggaggaggagcacgtgcggtcggtggggcgcagggccggggagccaggggggtgccggggctcgaggccgcggggccgcgggggccgcgctctgctctccgcccaggctgggccactggagcgcgggagccctggagcccggcgctgcccggcgctacccgccgccctcgggacagtcaccgtgagcaaaagagtcggtgtcatgtgcgtaaacgaagctcttaggagccgaggatagatttcacaggaacgtagtgccttgttctgaaagacgcgctttggttgatattaggaagtatttttaaaaaattggggaggtcgtttcccttgcagctccgccaccatctgctgcgtggac

SEQ ID NO: 174 - DNA, 500 bp, Homo sapiens
  source 1..500: mol_type = genomic DNA
gctcctcctcccttgggaagagccatccggaagcggctcttgttcaggacgtggacgcaaccagggccggctgggagcggcgttgtcaacacacacccttggccctcggcaggtatcagatacacaatgggatgaaggaggttttttcacatttggttcacaactaggcagtatgtgtgcaagtgacagctgaaagcaaacctgtttctaaatgtggcttatgaatgttctaatcaggtgtggaaggagctgacacacggagagtcacaggctatacagctgcttcgagcagcgggaatgtttgtcttgggattagatgctgacgtgtggtgaaatgttacagagagcccagaggaaggaggagttcagaggttcccagggaagaggccgggggcttgcactgcacccccagacagtgtccctgtgaacgctctcatcaaaggttctgttccgtttgccaaacaccaattttctttttaaacatagcttgtgatggaacc

SEQ ID NO: 175 - DNA, 500 bp, Homo sapiens
  source 1..500: mol_type = genomic DNA
caggcagcaggttggagacaaaaagaaaggtctgggttagaattaaaacaatgaaagtaccgggaaatttttttgagagaagagaaaacaatatgcttgagcccgttatctgggtggtgtgggatggagtggagtgggggattagagagggtaaagaaaaagaaaacagaaaaaaaattaacagagagaaagaataacaatgataatataataatactctttcctctaagggaggaaaatttgagcaaagaaaggaagttcagtattgttaagtgattcagagagattcgggagaatccaaatcgaagctatttgctctgaagattgggaggccactggtacctttgaaaatgaagctgcagtggaggaaagccaaaaatcatgtgctaggaagtgacagtgtgtggaaggagagagtatgggctacagaactaaattgagcagtttaaaaaggtaaaaactaggaaacagacagcaggggggcaggagggtagagagaa

SEQ ID NO: 176 - DNA, 500 bp, Homo sapiens
  source 1..500: mol_type = genomic DNA
agtgggttttttattccaggaggggaatatatgactttctgaacttaggtctatatttttggcaaactcttattccaactctgcctgtactcttatatcaaatagaaagcaggcagtctttttctccttctagagttgtccaaggacagaaaaaaaccgcagcagaaatatgccacgtacacagaaaaaagaaaggcggatctgataagctggaaaggagaagcctggaaaaagatgtggattatgtaataggcccagaagatgggctgatgagaaaaagcttcttttaatgtttctggaaaaaaatgcaaatattcagcaagacacggtcattatcctggtgaatgggcacattcagtgattccttctatctttggtgcagagattgaggcatcttgggatgcaactgagggagcaaagctgactgcagcctctgccctcctgtgtgtgcagtcaacctggcacatcccctcttgctaccagacccgtttccctttcca

SEQ ID NO: 177 - DNA, 500 bp, Homo sapiens
  source 1..500: mol_type = genomic DNA
ttatttcatattgtctacagaaatttaattactgccacaaaatgttttcttccttttgcaaaccagctcatagttcatataatgactctcctggatgagtcatctgcaggaagtacaaggttttttttttgaatctgctaaggtaaagactttgaagtataaagttaaaagctgcacagctggaagcattctgggaaagaactttaaaagtgactgaaaccactggtattcacttatattttaacccagctacacattagaatcatgtggggagcttttaaaaaatataaatgtgagagccccagttcaaatcaactgaatgacaatctctgggtttagacctaggcacaggaattatttcagagccccccaggtaaacaacatatgcagctaggattcaaaaccactggccaagtctttatcattattaagatagattaaaacaataaggcatcatttagcactactaacgctttattcttaaagaaatgccatttaac

SEQ ID NO: 178 - DNA, 500 bp, Homo sapiens
  source 1..500: mol_type = genomic DNA
caactttatcctcatttccatcatctgactcacacaccaagcccctgaggcagcaacgccgaacatattggtatcagcaattacaggctgactcatccaagaacgtgcacaattaacctattgaacatctctccaccgggcttttcatcctcagtaggaccatctgcaccacattcacccagggcaggagcccagccaacccagtgtgcattcccacgcatttccgctttgatgccaagccagaagcaattcataaccccacagtgcagtgccgcatcagcaatggatctcaagctcagaacattcactctaagctgaacagaccatttctgggttctctgctcctaccatgctaaccctgaaagcaccccaaaacttaagaaagggatttcctactgttgcaatgcttcatctaacagttaacaaaatattaatactatagggcttaagactccaaattccaagttttatttggatataggtttcaccacctggttcag

SEQ ID NO: 179 - DNA, 500 bp, Homo sapiens
  source 1..500: mol_type = genomic DNA
attgatgtagtgagtcttggctggtattcttttcttaaagatagaatagagaatacatcacatatattttgcctcctgaaaagtttgtttcagttgtgtgtgtgtgtgtgtgtgtgtctcctaggacacaatgtaaaatgtgtttcttgccatgtaggagggtgttggttaaaagtttgaaaaacattgctgtagagaaaagttcctcaatcattaatatgtataaaattacaggggaaccttgttaaaatgcagtttcagacttctacttatctatcaatccatgggatagggtcttatattcttcatttcaataaaactcctaagtgattctgatgctgctattccaaaggatcacactttgagtagtgagggccaagaggaagagctatagccacaagcagaggatgactaaccctctggaggaatggcaaatgaaactctagaccctgaatatcctgctcaggataccacagccgcaagaggcatcttcagctaca

SEQ ID NO: 180 - DNA, 500 bp, Homo sapiens
  source 1..500: mol_type = genomic DNA
aaagttgatttatgatatgtgtctcgagttcagatttacaatgtgtgaagaaggaaattaagaaacagtttagatgcaatgtccagtgactggactgataggatttaggatttggaaggagaagaagattgcttgcttttttgctgatttttttaaagggataaattctactctagggcccaacagaaggccatcaatttcaaaataagtacgtggcacagatcagcgtccttcatagagcggtcttgggtcagctcgccgtcaggtgctctgttgagcttgagtgttactgctaattacattctgtaaaggagcttgggctgggccctttcacaaaaccgttgatgtctataaagtttggtacacttgatactggtttttatatctggcagttaacaagaatctgggcttctaccaacttactcactgttaaaaattcaaaagggcccattaaatcgagcccttctttccccctgagttctgaactggttgaaaaatag

SEQ ID NO: 181 - DNA, 500 bp, Homo sapiens
  source 1..500: mol_type = genomic DNA
gacaaaagagtaaaggaaaaaggagctgaaaatatcactgttggtactgacaaagcttatattggagaatgtggatcttttttttttttttttttttgagacagggtctcgctctgttacccaggctggagtgcattggcacgatcagggcctctgctgccttgacctcctgggatcaagtggtcctcccacctcagcttcctgaatagctgggactatgggcctgcaccaccatgcccagctaatttttattttttatttttgtagagatgaggtctcactatgttgcccaggctggtctcaaactcctgggctcaagcagtcctcccactttggcctcccaaaatgctgggattacaggtgtgagccaccacacctggctgagaatgtggattttgtttgcaggcaggtggggtcctactcttgtgcctgggaattacggaagcattcttgcacagccctggacagctctggccaagcctagcccgctgccattgctg

SEQ ID NO: 182 - DNA, 500 bp, Homo sapiens
  source 1..500: mol_type = genomic DNA
ttttggatgataagaactcagcatgttcaaagctgcacttggcatttctttaattcagttagagctattgattccaaactggcctacataaaaagagaacttgttggctcatgtaactgaaaagtccaggaaaatgttcaggcacagtttgatcaggggcttacatgccactagatccgtttctctggcagtacttctggactccacttcctctgttttgagatcattattagaagcactttcccctcacagtggttagaggcctcgtcagctcaagctgtatggactcattcaaatcctgccagggaagaggagggaaaggaattagacagtgtgcttaagtcagtatattatccctacttttccctggaattcttttacccaatattgaaaattctggcatcagggtattataataaacaatgtatagtgtagtgactttataattcttttaatagaaaaggaatgaaatctgtttaaagagaggttctattcattta

SEQ ID NO: 183 - DNA, 500 bp, Homo sapiens
  source 1..500: mol_type = genomic DNA
ctaggtgacagagcgagactccatctcaaaaaaaaaaaagaggcctttaggaaggtggggagacccaagtgaacccatagacaaaagttcagccaggtaggctgagcgtggtggttcacacctgtaatcccagcactttgagaggccgaggcaggcagatcacttgaggtcaggagttcgagaccagccttaccaacatggtgaaaccccgtctctactaaaaatgcaaaattagccaggcgtggtggcgcatgcctgtagtcccagctactcaggaggctgaggcaggagaatcgcttgaacctgggaggcggaggttgtagtgagccgagattgcgccattgcactccagcctgggcgacagagcgaaactccttctcaaaaaaaaaaaaaaaaaaagttccgccaggtagtcaaggccagattgtccaaagattaacaatctcttatcgtactctaggcatatagtcaacaaaaagaacttagaagcaattacagaa

SEQ ID NO: 184 - DNA, 500 bp, Homo sapiens
  source 1..500: mol_type = genomic DNA
cctgatgggaagggggaggagccaggcacggggcctggcacgtagtgggccttcattgaaaggctgtccctcttcccttcgcctttctggtccaggacctgccccagccaaggccgggcagaatgggggtggggggtggagaagcggaggctggagtgaggaggtggggtcaggagcgcgtctatgctgcactttccgctttccgcgctggacacagacagaggctccacaaagcggccaaagaaccaaactttgtccttgcggaagtccgcaggatctaccactcaaccccgatcgctggctccttctactcggtggcccgacagcccacccgctccttccccaggggcgagcgccaacgccccagggtcgtggatacacagcccaccccctggacggccctgatggagaccggctccgtccccccacccacccccattcccagtctgtgaccccgacccgagccactcccggcttcaatacgttctccccagaaccca

SEQ ID NO: 185 - DNA, 500 bp, Homo sapiens
  source 1..500: mol_type = genomic DNA
cgcagctcagtttcctttccctcactgagcgcctgaaacaggaagtcagtcagttaagctggtggcagcagccgaggccaccaagaggcaacgggcggcaggttgcagtggaggggcctccgctcccctcggtggtgtgtgggtcctgggggtgcctgccggcccggccgaggaggcccacgcccaccatggtcccctgctggaaccatggcaacatcacccgctccaaggcggaggagctgctttccaggacaggcaaggacgggagcttcctcgtgcgtgccagcgagtccatctcccgggcatacgcgctctgcgtgctgtgagtacaacctgctccctccccgggcacagatatgacagaggggcttagagggggcccagctttgagatgggttgttcttatgtcacaggacagagtgatctgacatgcacacttccccgccaccctgtcatggaccttgtccttggagttcagagagctggtctcatggcaggtt

SEQ ID NO: 186 - DNA, 500 bp, Homo sapiens
  source 1..500: mol_type = genomic DNA
gtttcatactctgactttctttgccttcagtcttcctttgaacgtgactcctgttctgcacgtatgaggatgttaaacaaatactgttcttctgacacaacctttctgttacttgagtgttttatagtacattcctagaactcctatgtattagaaaagcacaaggagctggaaggctttgctgcacttcataaaaatatggtctctgtagcagacacaactcattccctcagcctggcttaaacatgaggtcaaatctcctttattcctcattttaaatcatcacatggtttaagcttttttcgtatcccgcaagatcatttttcttgcttttgcaagaatcccacttcctttccctgatggatcaaagaattccagagctcactcaccatgactcacccatgccccagccaagttcacagggccgacagaaaaccaggaaagtcgttctgtcctctggccagcccaggccttggctgcattgctgtggtcattgacct

SEQ ID NO: 187 - DNA, 500 bp, Homo sapiens
  source 1..500: mol_type = genomic DNA
agtcatttgtgtaagttcaataagagcctgttctcttcacagcagcatacaatggaaaatattggttatattaccaggttttgactggaatgccaggcttaacgttgctcagaagttgcttctatgaggacgtctcccagcagctgtcagtgtttccaatgagtcatcgccagcccctgcaatgagcctctcaggctggtaagttttgtttcagaaccgcttcctcaagcttcttttgcctttaaaagcttcctcttgccccagcctcccagggaatgcctgtggtctgtcatggctcacacatcctggttgataatccactgctgttctccacggaatgccttcattttgagagctgctcgctgcctgttgtggtttcagttgacggcccaccgctgtgtgcagagttcaccagccgctgtggtgtgcagtgcagcagctgacctgcctgccttgtggttttctaatcccattgaggggacgtcttaggtgttctcacc

SEQ ID NO: 188 - DNA, 500 bp, Homo sapiens
  source 1..500: mol_type = genomic DNA
gcattattagaccattttctggaaaccattaaaatataaaataattttacctgtctgaagtagtaggacagattcgactactttttttttgaaaaaattattaactaaatttaaaagaaatgatcaaagtaaataattcatgtggttaaaaacgtaaaagtactggaattttttgatacatgaaaccagtagtcttctctcccagtccagtttcctgagagaatcacttgcagattctaaaaattttcagtttagctctctggggatgatctccatatctttaaataatatacttttgcctccgtttcttgccttatcagttttagacattgttatcttttgacttcctgcgctgatacatgaagcatcagcctgttttccctatgccccttaactctgttttcttttccttcttaatgtagttatatcaccattattggttcctgtgttggttaccctgtagcttaaaaatttttacttactttttttaatggatcact

SEQ ID NO: 189 - DNA, 500 bp, Homo sapiens
  source 1..500: mol_type = genomic DNA
taaatgccttgatttaacacccttatctacggtggggaaggagctgtgaaaagtggtccctaggcagagtaatcacagccccctacccagtggatgatgactcccactgcctagagcaggacagtcatttacgggatcacctaagggacattttgaaagaggatgtgtttgcctctggcctcaattgtcaccggaacgcgcgcgcgcgcgcgcgcacacacacacacacacacacacattttccccacagggattgtttgcctatgtgaacaagtggaagcagaaatcgctcttccgaattatttaggaaagccaacacgcaattatgcaaaagtgtagataaggttctccgaagcagaaagcagcagcgcgggacgcgggtttccccttctctggcgagtaccagtgctgggaggctgtttatctgtgtcctggtgctgggacaggacgcaatccaattccagctctcggtcggttctgccgctctgtccccggttctg

SEQ ID NO: 190 - DNA, 500 bp, Homo sapiens
  source 1..500: mol_type = genomic DNA
tgtctacttgggtagagaattctgttgttgaagcaaacagagtcattaaatataagatcaataaatataagatagagtgctggttgggaaaaggatggagagatgaatggatagctgcagagaccatgcacttgtttggtagaatcccactgacacctaggagggttttctctccaggcttcataaagcttgtacttttactgtgaaatgctaagcagatcatctgctgagactgaaggggcaggaaaacaattggctcagcaaaagaactgagggtttgaaatagccctgagaggaatggtggaaagagaagaccagggacatgtaaccacagcacagcggacccaagagattagactcattggcactgctgtgggatttttgtccagcagccaaatgtgtgtggtcaagaaggaatttgatacatgtatgtcatagccatttgtttacacatacttttctcaaatacgcaagaaaaaggctgttccttcctctttcgt

SEQ ID NO: 191 - DNA, 500 bp, Homo sapiens
  source 1..500: mol_type = genomic DNA
agggccgagcagaaatagtagccctcgttctctcggcggaagtcgctcagggtgaggacgaaggtgtcccccaacctcttgcccgagaaccgctgggtgtccagcccctcggccgccttgggcttgttttgggagaggtataggaggaaggtgggactggcggcggcgccgcgcggctggaagagccacgagcagcccgacgtcgggttggacagcagcacctggcacttcagctccactgtctcgcccaggttccaggtccgatccagcggcgacacccggaactggctcggcctggcggcgtctgcaggcggcaagcagcgaggctgagcccgcagtcccgcgccccccgccccccgcccgccccatcccctgccttcccgggcgtctcaaactcacggagcagcaaggccagcggcaggagcaaggcggtcactggtaaggccatgacgcgctccccaggacgctgcttggctcgaagctcgggcgcgaggggaggc

SEQ ID NO: 192 - DNA, 500 bp, Homo sapiens
  source 1..500: mol_type = genomic DNA
taatacgaggaaaatgggtagatggcataagaggacattgaatgtactgaaggcagcccaaatattccatgcattagtcacttcggatatccagtggagtgaatgcggcattcattaatgcccaatgtcggcccgggcaaagtccagacagtctgctggcagcaagaaagctaaaggcaagaaggcctgtgtcgattgtcgtctgtacttacgaggctgagaaacagtagctatgaatcagcctgtctgagactctgctgtcattatttgcagcagtaaggaagataatattttaaaaagctttcaggaataaaatgagtcttaaccactagaggaagaatcacagtctgcagctacattgcctagaggcttaatgatgattcattgcaaattagaccaattaagaataccccccatattgtagtcttgagtggcttagataagatcattggttccctttgactcctgggatcctaaaataaatgggatctcagagattt

SEQ ID NO: 193 - DNA, 500 bp, Homo sapiens
  source 1..500: mol_type = genomic DNA
caggacttgccaaggaattgagagtatccccgtgtctctgacccagtctcctcacggtttcccggcttcactctgccacatctaatccatttgccatcgtgtagctgagatgatcttctacaaattcaccctgaccatgcacctccctgtagagccttctatggtcccccactgccctcaaaagccagcattcttttccctggcataggagatactttgatctggcctctctgactcatgctcagtcctgtcctgcagctcccctgactcattgcattccctcttgacacgaagcctgtgcagatgctgttccctcagcctggaagacctcagtctgggtgactcatgctcacgctttaagtccctggtcagacagcacttcttccgggaagccagcctgaccttctcagcagggttctaagacccatatttcctgcctaatcacagccttttgcaaaagtgggtggtagttgtctcctcactggctaggcacacagtag

SEQ ID NO: 194 - DNA, 500 bp, Homo sapiens
  source 1..500: mol_type = genomic DNA
ccgccaccgccgccggggtggggcctgggcctggggccgcgagtctcgttggggcggcgctcaccaagtccactgctgggcctggaccagggggtgtgctgtcgggtactggggggtgctggccgagctgtactgggcgttgtactgcatgtgctgcagcgactgcgcgctgtaggcagaaaagggaatgcccgcctggaaggtggcggctgccaggtcctgggctttgagcgcgtgacatggtttgccgtccctgaccaagacgggcacggccacccggcgcggcgagggcaggggcgtcacctccatacctttctcggcccgggcgcgcttcatcttgtagcggtggttctggaaccagatcttgacctgcgtgggcgtgaggcggatgaggctggccaggtgttcgcgctcgggcgccgacaggtaccgctgctgccgaaagcgccgctccagctcgtaggtctgcgccttggagaaaagcactcgccgctttcgct

SEQ ID NO: 195 - DNA, 500 bp, Homo sapiens
  source 1..500: mol_type = genomic DNA
ttgtatctagcaatttgacaagaaaggtaaaacagaatattaacctcagcacacaagtttagctaatgatctggaacggggagttgtgagtagagaggaggacaaagatgaaagacaaccatttatcccaagtttctttccaaagatgaaaaataaaaaaccctcttagtaatgttttttaaattctaactactttcaagaacacatcaataagatatagagagataacaatcaagttggacattaacttaaaagtcagatgactttttaagcataagtaacttagaactgtaaagtaaaaaacactaaatgtcaatgactttaaagtggatactgaagtaaaaaaaaaaccttctattaaaaactagactatatgcagtaacttatgtagaaagcttagcataaatatttatacaaaattgccctaccatattttattaaaatattacattataaattaagagaaaataattttaaaaatgagttatattttaggcaat

SEQ ID NO: 196 - DNA, 500 bp, Homo sapiens
  source 1..500: mol_type = genomic DNA
agttgtctatctgtgctttaaactcctataaacatatctcccataccacagcatctaactcagagtcacattcgaattgccagcaaatggaagcctcataaacccaaaaggtgaacggcagtgaagtgtatagagcacactttgagtgcacagagtatctttgcagacagtatcttttaagactttcacaatcacatcatgagattattcccataccaaaaagtaggaaatgaaagcctggaaacaagttatatcgacattaaactgctctcaaacccaagtgtacaaatgatttttcttgcaaagaaatttatatcctacacaaagttctatttcaaaatgaattctggaattcaattaaacactcatcttgaaaacaagagtttaagtggaaattcctcactggtattcaagcaaataaattaaataatgatattaaacctacatctaatctcttatcatacatattgaaagtttgctatatagctaccactaagtta

SEQ ID NO: 197 - DNA, 500 bp, Homo sapiens
  source 1..500: mol_type = genomic DNA
aagagaaatgactacagccagagcaacgggatttgattatcgagtagatgaggaggaggaaaggggaggccatgacttgcatgtaatcagacctcactgaagaaagtggagagaacagaaagatgaaaacggaatgcaagttatatgcaatcatacactgatgactttctgaccctggcagtgccaagcgcagacaaccagtcttgtatgattttagcaatcaccatgcccttcatgtctcctatgttgtggtaatggaaaatcttacttggataagatgtaatatgagcaagatgtgtatttagtttgagcccggcaggcgtctccagtggagcacaggcataacacaccagggcctaggagcctgagccccttttccagtaatttgttcactacatgtaggtcggtatcattactccgggccctctgcattctgactgcagccatgaggtctgattaccgtcagcaagaagacgctgacacactcaggtttccagaga

SEQ ID NO: 198 - DNA, 500 bp, Homo sapiens
  source 1..500: mol_type = genomic DNA
agctcaaactctgcctccaccttgccctaaaaaagacattcctgcatcactgggagcagggggcgggctcaggccccagctcagcctggcctctgcccacgggcacccaccgtgaggatgtacacattgccacccatgtctgtgaactccaggtcttctggccggcccttcctcctcctctgctttcgcttcttcttgccagcctgagcctcctgcgcctcccgctccacgtcctctgcctccttcagcttcactaccggccaccagcccctcaggcggcggcagcgaaacagattgcacctcggcccggccccattgcgggccagctgcacagagcagagctcggggccccgggccccacgcaccatgtctggtagctgcaactccagggatcctgcaagtccagagcacaccagattaggcatgggatcaaagtctcattgtgccaggggtgaggaggcaacacaccaaggttgtaaattggggcattgaaagttgtt

SEQ ID NO: 199 - DNA, 500 bp, Homo sapiens
  source 1..500: mol_type = genomic DNA
ctgcggacgcgccgctgtggaacacgacctggggcgcctccaaaacagctcagcgccccaaggagctggaaatcgcgggagcccggcctcgggggacgcagcctgagccctgggggcggggtcgggattggggcggagctacgggcgatcggccaggcctgggggtcggggaaaggagtggaccggcagtgtcagcgtgtgcacagctgtagaagggtgggactgggctggttactggacaggcggttgtggtcagaattttgccaacggagccaaaccgatggtggggttcacagtctgggggcggcttgaagcagtttgttttgcgggcggaccagccctcctaggcggagcggggtcgcgaggatggggcttgcggttgggaatgggccctatggagccctatggaccgaggcgagtgaggccagatttgccgcggccagaagcgctcacccgcgcggcccggatgggagatccgcctcaggtccggcacgtgcgta

SEQ ID NO: 200 - DNA, 500 bp, Homo sapiens
  source 1..500: mol_type = genomic DNA
gcttagcatggttgggattgggactttgaattgggaatacaggagccacttgggatggaattttctctaaacgtggtttatttcatttaccagatcttatcaattaccagtgaatctacatattaccatactgagaaacattctgaggagtgttgcaaatcatctataaggaatgcagaatcctttcaccaaaattgtcattgaggcaggagtcaggggtggtgatgtttgcaatctctgccttaaggaccagagaaagtcaacatacacaaaattgattaatgggtgagacagcatgattggcttttatcctgcaccctttcctgtctccacacacataccctggcctcatggatgcagtacattttcctgactcttgactttggagtagtcacgtgaatctgttttagccaatggcatatgggtaggagtcatagtgggctgattcagagactagggcaagaggcctcctctgcttccacttgctctatgtttctacc

SEQ ID NO: 201 - DNA, 500 bp, Homo sapiens
  source 1..500: mol_type = genomic DNA
ctcgggtcccgtcttcgtactcagccgcgagcctcgagccgcgagctccgctctggtcgccccgttgaaattccgtgccccagcgttcgggggtgcccgtcggctgctccctgggccggaaggtcctgggcggaggaaggccggtagccaaaagtggaagcgccacagtgaagcggcccagggccaccgggtgagaaacctccccggagggcagacggggagaccgaagcacaccgcactaggcatccagactgggcttgggagccgcgcaccctccctacccagatccaggatggctagaattaacgggttctttctgagacctcggctcaggcgccgaaaccggatagatcgcgaattcgctggacccggagacccgacccgcctcccgcgtcaccttcttctttctagctttgggcgcgcgcagcgaaaggcaggagaggcgcgcactgggtgagtgagtcccggccgctgtctgcgctggaccagcccgactgacc

SEQ ID NO: 202 - DNA, 500 bp, Homo sapiens
  source 1..500: mol_type = genomic DNA
cctcctccttctctgctggtttggtaggtcccttggctttggcatcatctggttccttcttggccacctgtcatctctttgggtttagcgtcttccttcacctccacattggcaggagcctccttctctggggtggctgcttttttcttatctttagtctcttccttcttggcttcaactttggattctttgggcttttcgagcccaaacttgacttcagctgaagattttgcctcttccttctcagaggacttcgcttcctcctttgttggggacttggccttttcaggccttttcaggggacttgacctcagctggagactttgcttcttccttcactggggacttggcctcagctggtgactttgcttcttccttcactggggacttggccttctctggagacttggcctcagctggtgattttgccttttcctttgctggggacttggccttctcggggaacttgacctcggctggggattttgcttcctctttct

SEQ ID NO: 203 - DNA, 500 bp, Homo sapiens
  source 1..500: mol_type = genomic DNA
ttaccttgttctatcagttactatgtgaccttggccaggatactcacctctttcagcctcatttccctcatctacaagaagggggaagagttatttcccttacatggtgttttgtgacaatcatattaaatgatgcacgtgaaatgcttagcacagtgctggtccgtcactagtgtacaatacatgatggccatttacattgagcagaaactggaataagttatcaagtactgtgggtccagatggatttatgaatgcattctttcatgcaattttctgcatgtatatgtcattaaaatataatttaaatgtatcccttccaaattttaaggcatagttttcttctaggtgatccaaacacagagaaaatacgatgtttttgcatttggtacacaattataaagatagatgcaacaattctaagtaaaatgatgacaaattaaatccatttgtatattaaaagaatgaaatgccatagcagagtagagtttattttggaa

SEQ ID NO: 204 - DNA, 500 bp, Homo sapiens
  source 1..500: mol_type = genomic DNA
tctctcaattgattgtttacagtcagttacagatccaacttccttctcgcgactgcacttgactgagtgcagtatgaaatgaaagaaagaaaatatatcacacatgataacatgataaggctagtgatttgtaaaactcttgttcaaattgtgtgtatgtgtgtgtctgtttgtacacctgtaacaatataaaaattattccttactgttggttgtaataaaaagaaaacattgagaaacatcatgttacaatataaatgcctccgtttcctcccccaacaccttggaacaggcagactgtctctcccaggaagacctcacctaatgcaactgtacaaccccagggagcctgggtcccactgagcccttctcatagccccctctgtctctgtccttcaccagatggtgtgggcatcctccaatcggctgggctgtgccatccacacctgtagtagcatcagtgtctggggcaacacctggcatcgggcggcatacctggt

SEQ ID NO: 205 - DNA, 500 bp, Homo sapiens
  source 1..500: mol_type = genomic DNA
gaaaaacatttttttggcggaggagggaattgtgtagagttgaagaaatccaagagattgtaaagttcttgtggagggtggagtcagtgagaggaggcagagaaacaaggcgaaggcctttgcgctccatctggtatctgtgtccaatagatggtttcacccacagcatggcagagtccagcaaggatccaagaatatgcaggaatcagggaaatgatgaagacagcactttaaatgggagggatttttaagtaaatgctattaggccaatcaactggaagtctattcatttgcaaacagtaacatgaggcttcctcctcaaaccccaaacacatatacacgcacattccacagttccacacgggctcaagacccaaaccaaaaaaacaaattctatgagaatgcttgatacaagactaataaaaagaagactgggccaggtgcggtggtggctcatgcccataataccaacaccttgggaggcctaggcaggaggatca

SEQ ID NO: 206 - DNA, 500 bp, Homo sapiens
  source 1..500: mol_type = genomic DNA
cagtgtggttaggaactccccagtgtttgttttgccaaattgctctggaaaatagaggcgctttgggaggggagagtgggcgtgaaggagagcagggtgtgagaggggaggagagagactgcggtgacccgatgcagctgtccgcagtggtgtgtgaacaggtgtcatcctgttcttcggctcctcgggaacctccagtaaaatctgttttactcacagtgtttactcaccgtggtttctgaggttggaatttttgtgggggaaatggagggacaagatcggagatttgcagcacagggagcatggggtaaacctagaagtcacccatggaggccagttccatcaggcctcattactggacaaccgctgtgtgtgccctccaaggtggatgagtcttatcaccccgtcttacagaggcagaaactggggccagagtgcctggataacatggcagttaggtgcttgggtttttgagtgagatgggcctgggttcgcatctt

SEQ ID NO: 207 - DNA, 500 bp, Homo sapiens
  source 1..500: mol_type = genomic DNA
agacctcgtgcaaaatgaacaaaactcatccagaacgatgtccacaggcccctgatggctccccaggcctcactgaagcagggaagggtgagcatctcggtccacttcccctgagaatccaaattcctgtttcttttctttcttttttgtctttacttattccaaatatgttcaaaatggaactatgaaatgccatattttatccaaataagtaatttttaaaatgccatcttagaagagcttctaaacatttccaaaggcctttcaaactttctccctgaaaggctttgtaccaggcaaccaaatccttccggacttgttgaatgcggagagtgagagagccagtgagtggtgctggtgttgtctctttgcttcctccttcctcctccccccaccggcccccaccaatctgtccggtggatgctgagtgatcattttgcggatggcttggaacttggcttctcgaggggaagctggtatgagaaaatgagaatctcatt

SEQ ID NO: 208 - DNA, 500 bp, Homo sapiens
  source 1..500: mol_type = genomic DNA
caatatagcacacccagatttctttaaaaaataaggaaacactagtgaagattggaatgaagtgtattgcgtaaggttttataaatttctctagaggaagcaggcagagttggctctggaacttctctacactgtctacaagttaaaaataagctgatgttccaggagagtacggttggatcctgagagtaagacctggtagaataaacagtatcgtcagtgttctcagattccttgaaagcaggaactaggtgatattcttttttttttttctgagacagtttcactttgttgcccaggctgaagtgcagtggcatgatcttagctcactgcctgccgggttcaagcaattcttgtgcctcagcctcctgagtagctgagactacaggcatataccaccacactgggctgatttttttgtattttagtagagacaaggcttcaccatgttgatcagtcttgaactcaaattcctgagctcaggcagtcctcccacctca

SEQ ID NO: 209 - DNA, 500 bp, Homo sapiens
  source 1..500: mol_type = genomic DNA
accttcagacagagaaaacatctctaatttattttttaatatccattttacttccactttgcaatttccatcggtttgtttcttgacaagtttgtctcttttaggacctgcaacatctctgtttagtagtgagcttttctcatttaaaagtacttactgaaagactcccacatgggagtcacatcagtttctttcactgatgttctcctatgcctatcagaaggcctggcacatactaggacttaataaataatctgctgaataagtgaatgagaactggaaatttaaatttttatgtcaatgaatgtgtcatctgctttcttgttttgctgaatcatggggcttaagtttctgccaagcactctttaaatatgtgcttaggacactagcagatttgtccagaattttgcaatctagaaaaaaagcaattttaattttagcccgtgtgtaaatttttagtttatggtttagaattgcattattttgaattacaaatgggg

SEQ ID NO: 210 - DNA, 500 bp, Homo sapiens
  source 1..500: mol_type = genomic DNA
cactatttttggaagcagtctacttataagtgattaagaaatattttcccatgctttccaagatttagatgcttcttatagtaaataacaacaataaaaagcccataattccaattgaaagcaaatcccaaaggaggcttagtagggagacaaagcattggaggtagctagaagtagaaggagaaatctatattacagaaaatcttatgaatgtacattggagtgaggtcttgggctaggtactgccccagatggttaatcattctggcatcgtgtctccttatgtgacagacatggataggaactagaaaaagcagggctattctactatactccctcacctgtatctacataatgacatataatcatttattttgtgggaatttaatttaacagaatttaattgaacagataaaacactcaataatatatcagaaaagacccaacagaatctgagaaatagagatgatttggacttcacaaacatctagagttccatt

SEQ ID NO: 211 - DNA, 500 bp, Homo sapiens
  source 1..500: mol_type = genomic DNA
caacctaataaaatgaggaggcggggatttcattgctcttgtcatttaagcagagtcgtggttctaccttcccaggcccctgccatcctccccatctaaactcccaggagagttggcaacccacttctggaaggctgcccacaccttctctaatctgagaccaattgagaactctaacccagctctaaaacaaattctagtcttctaagaaaagtagcaatgatgttagtagtttcctaattttttataatccagaaatgtcactcttatgtggcagtgaattcgcacattcccaaggaaccaagtgactcaacataacacaacagtcacccccaggatgtaatgtgacacgcacaggcccctccgttccaggagatggtttgcccataatctggggacgaaatcgctggaggccttgcatgtgggtgttgcgttactgtgggagggttttgttggcatcaaggctacctttaatgaatgggctttaataaatcaaagag

SEQ ID NO: 212 - DNA, 500 bp, Homo sapiens
  source 1..500: mol_type = genomic DNA
atgtggctaataaatgcgtttcatgacatgccttaaacaaaacaaaacaaaaaaaaaacctcttgtaacttttaaatattttgatttataaaaaaagaaaaaaaaaagacttccatttaaaaagtttccaatttgtggagataaagcttgtttttgtcctgccttctcccatcctctttctgtgccagctctgccatgggaaggcattcttaacatttttctgagttcttatggttggaaggggactttggctcttttggtgtttctatccaagccctcttttctgcatcaaaggccatcgttcactctgggcctttgaagtcaggcaaaattttgttgttggtgggatttagcatctactcataaactgcatataaatgccagtgcggatatgactcaccaaaaagaatcgaaccttctgacgttcgggtcagacttagcagtcttttatctagagaaagaaaacaaaacttgccttggctctaagtttaagctgttga

SEQ ID NO: 213 - DNA, 500 bp, Homo sapiens
  source 1..500: mol_type = genomic DNA
attaagattccagtgagtgggtaaagggccttcgagacatttgcttagtcaccattttcatttttcttcctcgtggaggttcttcctgcgtgttaaactaccagggcaggatagggattttgtgagcatctgtaggctggcttctgctcccagcctttcattcatcttgaatgttcccgtcctcatggatgaaaggatagcaacaaagtttgccagcagcagagctggtggtcctcttgagattctgtagttttccttcttgtggtccaaaattttgtctcactgttgtttctctgcttttggtacaaagtcatggaaatttacaaggtacagaaagatggcgtttaggccaggcatggtgactcacgcctgtaatcccagcaatttgggaggtctaggtgggtgcatcacttgaggtcaggagttgaagaccagcctagtcaatatggtgaaaccctgtctctactaaaaatacaaaaattagccaggcatggtggcgc

SEQ ID NO: 214 - DNA, 500 bp, Homo sapiens
  source 1..500: mol_type = genomic DNA
tgggaaacctcgaggtgcggtgcccgtgtacttctggtactttgcgtggtgccatcagggaccccagagccacagctgcgtgtgtgtgtggatgtgtgtgtgtgtgtgcgcgcgcgcgcgtgtacggcgaaaggatgtgcttgggggagccgagtacacaacgtctgcttgggcagctgctgggcaggcgttgggcctggaggtatctcacacccacgtatcttccagtcttcaaacacggcattgctctgcctcccgtagcgcgcttcgaacctgcctcgcggacacgtgaacagaggctgtccctgggaagataagtgcgctttcccgtaaaatccgggaaatttgccttgaggaaagtttccgttcttgttacttgtcgggtttctcccacttccacttagccatgtttctgcgatctgggtaatccctttcaagcccaggaggaattctcccgggtccataattgagggtcggaagccgtgggggtgagaaacgca

SEQ ID NO: 215 - DNA, 500 bp, Homo sapiens
  source 1..500: mol_type = genomic DNA
attagcctggtgtggtggtgcacacctgtactcccagctacgtgggaagctgaggcagggaaactgcttgaaccccagaggcaaaggttgcaataagccgagatcacaccaatgaactccagcctgggcaacagagcaagactctgtctcaaaaaaaatttttttaattaaatactgttatgtgtgcacatggggtagaactccactactgaggggaaaatataaaaaagcagttgcacaaaaatttgcagagctctcacaggacagaaaatagttcaagttcgcaggagccagaatacacagcagaagtgctttacgtacacttccagttttaatacctagaatagtaaaaagacatgtattcatgtgcagagcagtaaagaatataataactcctactattttggtgccacaaccaagatttgtgctacagtgccagaagtttatttctacccacccatgatccatcagtacaaatgtcaacactgtaaaaaaataaa

SEQ ID NO: 216 - DNA, 500 bp, Homo sapiens
  source 1..500: mol_type = genomic DNA
tgctgctctgatctatggggaagccaagacctcttcacgttccaagagagctgcttcagggggacggaggccagagagggctctttcatgtgagaacacccaagtgcctagggcccggcaggtgcagactcggggctgagtgctttgcccactacagcacagtgccctctcttgggccaattcagcatgaggctaggcctgtgcccactgcagctgacaaaatgcgggaacagtgccacggctgctaatgccagcagcggtgtgtgtgagaagggaatagtctgtttttaatgcaggctagtccctccaggctggagaagggccaaaaagaatcagatatcccagcttagcgtccaggtcacaccaaagacagcatgagagagaaatcagctcaggaagaaagagcaagaactttcaaccttaccaggagcaaggctgttgtgcctgcgggcacgcctggcagagcctccaggcggaagacagacacgcccctggcccca

SEQ ID NO: 217 - DNA, 500 bp, Homo sapiens
  source 1..500: mol_type = genomic DNA
ttggatttgaggtggcaagaatgacatagtgcatgcctcatgtgcctgggttaacctgtcactagaggagaatgcttgcggagagaactctggagggaggaggctgaccagctgtgccctgacctctccagccttcgtcttcctgcagactgtgaagtcgcatgatcctccccatcccgtttcacacaaatgctgcctttgcccagcaaaaagataaacactcacaaagctattaagacattatccaaaagtgttgagctctctggtagagaattattatgctgttttcagtgtaataatatgtagtagcatttctgagaaaatgctgtgaattcacttttttaagttacaaagtttctttgtaaatttagaaatctggctgggtgctgtggctcatgcctgtaatcccaacactgtgggaggctgaggcaggcagatcagttgaggtcaggagttcaagaccagcctggccaacatggtaaaaccccatctctactaaa

SEQ ID NO: 218 - DNA, 500 bp, Homo sapiens
  source 1..500: mol_type = genomic DNA
cgatacccgcatcagaattagctgaggtgcctctccctgagccggatggggctctgccaaggacccagcctggcaggcagtgggtatctccacccctcaggtcctgtcggcggcaagcgagcagcctgcgcaggtggctggagctgaacagagaggagccggggcctgaggaccaggaagtagagcagcaggtgcagaaagagctggaacaggtgaggccccaggccatccccaggtgtccctggggacgccccgggctgtgctccctctcagccctgcctgtccctccatggccccaggtggaaatgcagatccagctgctggcagaggagctccaggctcagcgccagcccattggcgcctgcgttgcccgcatccaggccctgcggcaggccctgtgctagcgtgttcgcaccaggaacgcaggtgctgggctgtcggggaggcctcaggccacctccaggaacagaacacagttttaagtttgattttttttattt

SEQ ID NO: 219 - DNA, 500 bp, Homo sapiens
  source 1..500: mol_type = genomic DNA
ttgtctgtgtcattccttgttgtatttccaatagcaagagcacatcagatacttggcaactaggcagtcttccagcttctgccactgcgcccgacttccttgttgcatggatttatagctgattgaagcaactgtagccaaagattgagttaattacctacctgccaggagagcactagtgttatttagcccattctcatcctacatatttttcggcatagatgaaaatgaaagcttttgtttatcagatttgcagatgacacaaaactgggagaattaacaagtatgtttatttggtaaaataagttttcatctctaacctaaatcggctgaaatgatgtgtcctaaactagaggaaaaagttaataaagatcaatgtaaataagttaatcttaaactcagtatgcaccagaactgagagaagactgttttaggaggtgttaatggttgtccagtgcccaaaaagccaccagaggcttactgctccgcactcttggcat

SEQ ID NO: 220 - DNA, 500 bp, Homo sapiens
  source 1..500: mol_type = genomic DNA
gggaagagtccaggagaaacgtctgcactgagaatggaaaacacactcctgggacagtagaggtgaagattctcaaggaaaagcagcgatgatggctgagtcacttgccaggaatgtttgattgcactgttatgacagaacttattccaggacctcatttttgtggtttcaacaactcttcatttattctctgaagattgtctttcataccataggtatgagttttggcctttcatcctctttctccctgaaagctctaagggaatcattgtttaaggaggatcaaattctgcttgtgagagcagtccttgcagactgacctgagcttgggaccaggcaccgttgcaatgatggccactcaggcccaacaatgttactatttcacaccatatctttttctacatacagacataccttggagatattgggggtgtggttcccaaccactgcaatcaagtgaatatcacaataaagcaagtcacaaaaaattctgggtttcc

SEQ ID NO: 221 - DNA, 500 bp, Homo sapiens
  source 1..500: mol_type = genomic DNA
ctctggcattagggagcctgttctaatctccctttatcaagtttgagtgatagttctgctcaacgagtattgacagggccgtcctgtttctcaggctttcgtttccctcggttggagaaggatacagtgcattttcacattctcaaagtctgcagttgtttttatataagaagcaatttgcttgggtcacgtcaggtcgaatgggatgcctgcccagctcttggttttaaaggaaaaacatacagaaagacacaaaaacacagcagtttccttcattaaattccactctacctgccatgggcttctagccacaatggaatttcccaccctggcctagcctagcctaacttttatttttagggattttttttcccctttaaatcttatgagctttctttcaagtgaactttgaggtaaggattattaaatgatagagtaattgcctggttaaaaaagaatcagacataaaaaacaaatgcctagtgaccttccataatatc

SEQ ID NO: 222 - DNA, 500 bp, Homo sapiens
  source 1..500: mol_type = genomic DNA
caaactctcccacgtgccctgttcacgatactgagttatgactcagccagttcccaccgctcaacccagaacagcagctgtcggtggggctgcggagcccacaacacagctcacagcagaaggcagagccaggaaaccacggagtcctgcacttgggatgtcgcctcagagaccaaaacagtagaaggattcagaagtgcacatgaaaccactgccgtctgccacatagaaagccaaggggaagctgcgccacacctgtctgacaacaaccctacagggcagagggtctgcacacctgcatgcgcaatgcccagagaaatccaatactttaatggtgcttccccaaagacacggcagcacaggaagagcaggcagcctggcgctggatcaagccccggaaacctgtggtgcgatctgctagcagaagcagctcacacatgctgagacagacaacgcagacagctgggaagcagaacatgtggcgggtccctctcttcagg

SEQ ID NO: 223 - DNA, 500 bp, Homo sapiens
  source 1..500: mol_type = genomic DNA
cgcaggagctgggccacggcagagtaattaagaaaataatgaaattgatggcggatgggggcgctagaaatcctggggcgtctacttaaaaccagagattcgcggtcggccccacggaatcccggctctgtgtgcgcccaggttccggggcttgggcgttgccggttctcacactaggaaggagcctgaagtcagaaaagatggggcctcgttactcactttctagcccagcccctggccctgggtcccgcagagccgtcatcgcaggctcctgcccagcctctggggtcgggtgagcaaggtgttctcttcggaagcgggaagggctgcgggtcggggacgtcccttggctgccacccctgattctgcatccttttcgctcgaatccctgcgctaggcatcctccccgatcccccaaaagcccaagcactgggtctgggttgaggaagggaacgggtgcccaggccggacagaggctgaaaggaggcctcaaggttcct

SEQ ID NO: 224 - DNA, 500 bp, Homo sapiens
  source 1..500: mol_type = genomic DNA
ctttgctacaaagtggagaagttgctctactctggagggcagtggccttttccaaacttttccacttaggtccgtaagaaaagcaattcatacacgatcagcgctttcggtgcgaggatggaaagaaacttcagaaaaactctcgccagacaacccggcagcacttggccccggaacagagaggagagaaagacctgaccgccgcactcagggccacccgccgcactaagtttgagggttccctctgcctccaggcctctgtcgcccgagctcaggctctcctaggtgcttcagggccgggctgcactcgagccccgaggaggccctgctagcgctagcgcggcggtgataaccgagggaggtgggtgagaggtgcggctgtcgaggcaaacgcagagcacccgcccagtcctccaagggccgagagccgggagtcccgaacgccgcttaagcagctccttgcttcccgcagcccgtccacatccctgcgggatttctgg

SEQ ID NO: 225 - DNA, 500 bp, Homo sapiens
  source 1..500: mol_type = genomic DNA
tgtcttttgctttgttttttgttttgcacacaacctctatttgtacaataatcagaaagttatcaaaatatgatgccacatctgtaatcttaaatataagcaggctctctatgaatcaccgaaaaagtcctagccatgaaaagaatctcaaactaatttgtttttttcctgcatgaatagtgactatttgtataaatgtatagagggtaattcaaagctacgaaacttgatgaagtcactcccagagtgaatgtggatagaaaaaggaagaggtctaagtatagaggcctggaacactccaatgtcatcaagtctgtgaagaggtcaaaccacaatagagactgagtcaacaagtaggaggcaaccaaagtgtgtggcgtctggaagccaggcgaagagagtatgtcaaggaggaatgaatgggcaactgagttaagtgctgctgctgagaaagaccagtggatttagcaacacagaagtttagcaaccagaagtcactg

SEQ ID NO: 226 - DNA, 500 bp, Homo sapiens
  source 1..500: mol_type = genomic DNA
aaggaagctggcctgtatcctattagcagtgggaaatcatgggagggtttgaagcagacaaaggctatgatcagattctggtcttggaaaacatccttctggctgctctttggagaagagtcgggagagagccgaaacaaattcaaggagaccaggcaagagatgaaggggatgtggacaagcatgtttctggagagacaatgctgtgtgtttgccttacttcctttttctcctgggcactcagctggactacatttcccaggctcctctgcagtgaggtaggaccatgtgatttagttccggccaatagaatgtgggcagaagtgatgtaaggaacttcctgccctggccaaggaaactctcccatacaatcctctgggctgtttctctttcccgcttgcctcctgcagagggtccaatgcagaactccaaggcctgaggggtggcaaagccactggctggaaggagcctgggttgctgaatgactgtatggagcagag

SEQ ID NO: 227 - DNA, 500 bp, Homo sapiens
  source 1..500: mol_type = genomic DNA
tttgtcactcattaaaaatatttatggagtgcttccatgtgctacatacttagaaaactcaggcagcaagatagagattatttctatcttcatggaacttatagcctaacagagttcattgacattttaaaaagctatgccagtcaataaataagcacaaattgtgttatgcaccataaaaggaaaaaaattacaaagttgtttgagaaagatattggagagcctaatatttatttgagttttaggatacattacaaccaaccgagtaacttttgggttttatgtctgcatgtttatttctcttatctttcaatagaattataaactgggaaggtgaagatttttttgcttatcatgtttatacctccatgtggcagtaaatgtagtatattgaacacggaacactaaataaatatgtattcaataaattaatgatttttctataggtatttgtctccttttgaggttttcttgtttttgttggtgcttggttttgtact

SEQ ID NO: 228 - DNA, 500 bp, Homo sapiens
  source 1..500: mol_type = genomic DNA
atatgtacacaaaggcacaatgtattatttaatattgtttttaaaaagaaaaatatatagttaccatggtattggaatgagcaacaattgagatcctgctgttcagtgggtaaaatgccctgcttcacacataataaatagcaaaccctcattgtttgtcatcttgtagctcattgtcctgataatttctcaagtggaagtaaattaatccatccccccctttaaaggatatagtaggctggaatagaaagagcagtgggtttgaagttaaaagagcctaatctaatccacttgccagctatgtgaacttgaataaggcgtagtttttgaatctgtaaaatagaagtaaaaccatcgatcctgcctgcctccctgtgagacgcacgctgagaatcaaatgtgattgcacatatggactgttttgtaaaataggaagcatggtacaaaggtaaagtactattgggtggggcaagggacatctacattgtctgtcactaggg

SEQ ID NO: 229 - DNA, 500 bp, Homo sapiens
  source 1..500: mol_type = genomic DNA
tataacaaacatgcagtgatcgatggcccaggaatgagtactaagtgggaggaaaggacatggaaaaatgctaagaagaaggctagaaaaagagcctgcatttgaggaaataagatgacagaaatatgaaattaattatccactgataacctagaactagatgatagcaaacattttaaagtcctaaattttcacagtgaaatgtgatattaatctatccacttccttagagacctagtgctgtatctcagcaaagctaaaccaagaacttgaaatgcttactttattcaggcacaccatgcatctcctgtttttagttaggtgcttttgaaaagatgactttcgatatatggaaaagaaggagagagtagtttattcttttttaaaaagaaaagtttcctctaaacttgatgactttaaaaatgttcttagatctttcatgagattgtgtattcaaaggtggcactcctaagcagactgtgatgtggcttcaggcaggg

SEQ ID NO: 230 - DNA, 500 bp, Homo sapiens
  source 1..500: mol_type = genomic DNA
gatgggacttgcagtgacaaatatgctctttcctggagaaattagcgaatatctgaaaggcttatatatttccccaagattagtcaaaacacaagcctagtcgtcacacctttccctcattatcctgtggttgttttcttaaatgttgtgcgtcttcataaatgagtcactctttccaagatctgtcaaaagtatcagtggttataaggctgggaagcataccaaccctagaaagaagtacagaactttcagttataggcaagaatgtaaaatgtccagaattactagcgttttattactttgccaaatttgcattcttacaccattgaatcattcctttttaaggattctttttcctatagttaaacctaggagggagaaaaaggtatttattttgcatgatatattcgtatagttacaaaatctggagcctgtattttttaccatttgaataatgcttctgcttgcccatacatgttgaaagtgttgtttaacttaaa

SEQ ID NO: 231 - DNA, 500 bp, Homo sapiens
  source 1..500: mol_type = genomic DNA
ctctttgtctgctttaatcttggtccccgctccaacttctgttcagctctgtattgaagttctactgtttggccctagtgctctgctaaactgcctggtatcagcttctctggctccgtgttagcctttgcttttcccacagccctcatgtttgtcattttgttctatacacttaggaaaacttgcttgccttactttacctggttcctcacaaggaaaagagcacaggacaagcctgtttccttttgtaaaaaaatcactgtgcaaatggtctcattagcataatttaggagaaaattttaagtcttaccaacagagattgagatttctgctgtggtagctgataggctgaagaagaatttctagattcttagctttgaatgacatttactgaaagagggagaggaggtggcagggggagagagagagagagactgagcagcaagtggaaaatactatattctttctcacttaatgtgttcctgggctccaaaggcaaa

SEQ ID NO: 232 - DNA, 500 bp, Homo sapiens
  source 1..500: mol_type = genomic DNA
tcacagggctgttgcaattgacctcttctctatctctggggactgctggcagcattcagagagctaccggagaggggtctgagctgtctctgtcctggaagtggagcatgggtcaggcagctctttcttctctctctctgttgaaatgaaaccgaaacaaaacttcttaatttggaggcagaggggccagaaaggagatgctcctcatcctctgcaaagcccagcatctctttcccttctttaggggatagagaagtctcctgcctgagtctctgcagaatgaagccagatgacgagttagaacctgagcaaagtggcatgacccgggaaaagcaatacctggacatggtgcagaaagacttcaatcagcatggtacacagacttactttctgtgtgaccttcagtcacatctgatcccatccataaacagggaagaggcaaacagaaaaaaaaaaaaaggaatggtgttatttcaaactaatattacatttaagactta

SEQ ID NO: 233 - DNA, 500 bp, Homo sapiens
  source 1..500: mol_type = genomic DNA
accaatggcccttcgagtaccctcggttcagcaggcacaacgcatctggagaagcataaataggtgccctcctctccacttaggcttcaaagactgtccacgtcagtgattttgtctctctgattgagcctgacatcatggtgagagtgctggggaagctcacagccaccaatactcattaagcacacctacacacatgtggattcatgcaaagcaagttaaacaggctagaggagcttataaacaaattacagaatctcagggttcggtgagattgagagagagtctagcctaacctcccatttgtctggtgcttggatcttccctacaacattccttcaaaatgcttatttattctctgcttgcacacctcccaccatgcagcctcctacagcaactcaatctttggacagctctagctattaaagtcaagtaagaagaagcatttaagcaagcacataaaattggcgcgagcttcctaaaagtttgagaattagatg

SEQ ID NO: 234 - DNA, 500 bp, Homo sapiens
  source 1..500: mol_type = genomic DNA
agttaagtaaacttgaacaatgccaacacttttcacccttagcatgcaatgggggccagtgggcagtcacgttcatctaggcaaagactaagggatcttttcttcaagtgagttaaagggcataacagacacatgatataagacaattaatgtgatttctcaaggaagatactccagccgtgaatcattattatctaagtaaatgggaatttaatgacttttcggacaaggaactcgaaacctttaatttaaaaaacaaagtaaaacaattatcctattatccttcttcccaccatccttagaaatatgtctctctatacaatcctttccagttttacagggggtcactgaacatccattacacagaaatttctttgtggaagatggaaacctaaggaagacccacctcttctttctctctcactgccttccactcccagctgacctctgatttcatcagctatgactattttgctgcatttcccttcagtgcctttact

SEQ ID NO: 235 - DNA, 500 bp, Homo sapiens
  source 1..500: mol_type = genomic DNA
tttttctttgtattatgttgcgcaggttatttagaacctttcttgtcagcctttccccacctgccaccaaccttctctttccaagatagcactacaccgtcagcctctacagaagaccttgggtctgaaaattaaaacttcgggggaatctcaagcagcttctccaaagagtcttgcaaggggcctccctgcactaactggatcttataaattaaaagaatcaacctcaagcataagcagaagacacttagataggacatttccagtaggaatgtaacttttactatgaaaaaatcatattaaaggttaaaaagttatatctaatacttgaggattatttatttaagcgtgcacacttgagaagttaccaggcttcaaactttttcagtcatcccattttcttgtctgaactctaccaatcctcaatttaccccaaatctcggaatgcctaggagaggtctaagagctcaagttcaagtttggccttcactccctcaact

SEQ ID NO: 236 - DNA, 500 bp, Homo sapiens
  source 1..500: mol_type = genomic DNA
cagttatgtcttagagcagcaattcattatcagagggacctggccagtgccccgctctccctgaaaggtgttaattttgtgagttatcaaatgttgttcgtcgcaggtgaggacatgtaaacagcgtttccccagtggcaaaaggactgggctggagttgaggaagtctgggctctggttccagcttttactgtgactggctatctcacccctccggtttcggtctcgctgggactgtagtttccctctatgtttctccaaagcttccttctttgtagttagtcagaagtgctgttgtggttaggaatcattgaaatgtttttccaactgctttttgtgtgtggtgcgagtgtggtgggaggggaagcttctatggttttagtaaaaacagaagcatcttggaagcagaaataaacatattaaggataaaataagatatacccttatataccatggcaactgctagttggtgacagagaaggaaaggtgcaaattctcaa

SEQ ID NO: 237 - DNA, 500 bp, Homo sapiens
  source 1..500: mol_type = genomic DNA
tcgtagctcactgcagcctcaaactgctggattcaagcaaccctcttacctcagcctccaggactgcaggaacacgccaccacacccaactattgttaacttttcttgaagagtgaaaatggtatgttcaaaaggaaaaaagacgttgcttaatatttatacagtttcagttttacaagatgaaaagagttcttgaaattgattgcacaaaaatgtgaacgtacttaacactactaaactgtacacttagaaactgtgaagatcgtaattttatgctatgtgtattttaccacaatattcaaaaaaaggaaaaagatatatttagggataaattatacgtctaggtttgatctaaaataatccacggtggggtagaggttacagaaaaaacaaaggtatatgggggttcattataccagtctctatttttatatgtttgaagttccaaaataaagttttaaataatggcttagcccaacaaaaaatattttttcccttta

SEQ ID NO: 238 - DNA, 500 bp, Homo sapiens
  source 1..500: mol_type = genomic DNA
gttcaggagccgtgtcctctggttaagacagtgcatttttgcttccatatcaggaatttcagtgatatccattctcctcagggattagagattgttaattactttctgtttaaaaaaaaaaaaaagggaacccgcagcactgcagcttggcaggttctctaaaaatagaggatttaggttatttttaaaaaccctcattgagggatcatgaccatgagtcacatttatctccagagtttgcctgctgaaggaaaaccacatggttctgtggacatttaaaccctccctgaaacactgccacctctacagaacaaacagtcccatctacccatccatgaggaaatggagaagaatttgtgcctgtggaatttgaggacccaatttagtttaaaatagatatttcatgtccagaggctgtgaactgttttctaagcacgagctcttactaatgtttgtcatgctgctgtatggctcattttacttattgttaggtttattct

SEQ ID NO: 239 - DNA, 500 bp, Homo sapiens
  source 1..500: mol_type = genomic DNA
acccccccacacaatcccaaaaaaatatacagatctatgccaagcaccagttaagatgcctggcacatggtaggtattcaacatttaatgaatacatgtagaggacttttacttttcactttatatcttttggacaagactttgaatttttatgagcatgtattacttaaatctagatttatagggagtgatggaaaatgtgaaaataaaattttaaaaaggaaaagaaagagtaaagatctagatttaaaaaaggaaatgtaaacaagatgaaatagccaaagataggtctccccaaaactaatgttgagacaatgccaccagcagtgacagtcagctaagagatggttcgcagctcactgctcagtactgaggcattcagcaggggttgtatttaactttcaagttggaaccaaccgaaactgttgggcttgaagagctgtctttatgagtcatcgacggcagaaagcacagaagcactaaagaaaataattcagaaa

SEQ ID NO: 240 - DNA, 500 bp, Homo sapiens
  source 1..500: mol_type = genomic DNA
gggaaaaaaaaaaaaaaaacactttacccagacttaaacttgatttcccagatacaagtttggtctactttctttgatacaaagattttctgaagcatacctttacgttcaacccataaaaatggcctatcctattaatcaacatgagaaagaaaacatgccattctggcttttaagaccatcttcctgaattttagctgacttcgaagcaatcatgtaaactgatctttgacataaaaattccagttacaggaaattccaaattaactaaacaactataatagtgttatgatgtactttgggccaaggtatcagctgcagacttctcataaaaagaaaaaggcactcattagccaagctaataaaaattaccacaaagaaatttgctggagcaaagagaggaatcaatatgaaatgctatataatgaatgtacgacaaatgctctctcaacggcacgtactagcacaaatgggtttttgttctgttaaactttttagag

SEQ ID NO: 241 - DNA, 500 bp, Homo sapiens
  source 1..500: mol_type = genomic DNA
acgaggccactaaatgagtctgctgcagtacacacacaaaaaagttctgtgctgtgtggttagccaaggggatcaagaagcccattgttaaggtattagtaatagggtggaactcagacacacaagaatcccaaaagcaaagtacattccgcaaacgcatgatcctatttcagccaaagtccacactctgaggttaatgaattgggaggcctctgcataaatcaagacatctgtcagcacttacaaataatcacagggccaaggaacccctcatccatcccctaaacactcaggcagagaaaggacaggccaggcaaggaaagtcattcctaaggaccagcccagaggtggcaagagttggcaaggttgtctaaagagaaagctctacacttacagctctggaacagttagggttttggaagaggaaaaaccaccgaacacaacccatgcacagaaagatattctgcccaaaggagggctacaacatcactcgttaaaac

SEQ ID NO: 242 - DNA, 500 bp, Homo sapiens
  source 1..500: mol_type = genomic DNA
gctaatgcattataattagagtataatgagcagtgaggatgaccagcggtcactttcatcgtcatcttggttttggccggcttctttaccacatcctgttttatcacaagatctttgtgacctgtttcttgtgctgacttcctatctcatcctgtgactaagaatgcctaaccttttgggaatgcagcccagtaggtctcagccttattttacccagtccctattcaagatggagtcactctggttcaaacacctctgacaaaaagacagcacagttgttatggttgcctccagccaccatactgggaacgctgcatcccttcactatactcagatacatgtccagccccagcccaagtgatctctggtctggctgccctggccaggaaggcccaaatgcctaggactgctctgctctttcctgttccctagctgctgagcccacatggctcacactgtgatactgcttctcccaggagcatctagggctgtgcaaatgc

SEQ ID NO: 243 - DNA, 500 bp, Homo sapiens
  source 1..500: mol_type = genomic DNA
gaaacaaaaaccaagaaaaaatttaagatatataaataagctatgtaggacaatgaagtctaatatatgcttacctagaattctggaaggagaagagagactggaacagagaaacacttaaagtacaacagctcaacatttcccaccacagattcatgaagcccagtgaatcctacgtaggataaaaaaatgtaatgcccatcaagatgcctcatgatcatgctccagaacatcagggtgaggcccttaacccacatcaaaggtctcaccgcagaggagtgtttaatttgtggcattttgaaaaaaattaaaaggtagaacttaaatcttggacaggtaaaatagcatatgacagatgagtggtaagagcggaaatgttctaaggaggtgaacaactttagactttgtgaaagtatgcaaagcaaacatttcaagttgtccccagatttcttttatagctttccaggatagaaagaattcatacactgcatttggttgtt

SEQ ID NO: 244 - DNA, 500 bp, Homo sapiens
  source 1..500: mol_type = genomic DNA
gtactcacagtcatgcctggcacatagttaagtgctaaataaaaggtaattgttattattattttcttttgtagagcatttgatgaatttctgtccataaaaaccctctgagagaagtcatgaaaacaaataagtctgttgagctttacatatgccggtcttagccaaatttgtctgaccacaagatcctttgatctccccataaaacattttctatcactgggggagctcaagtcctgtagagctcaccatgggatacactgctccatgacgactgtgtctctgcctcgtctacttccattgctcatccaggaattgagaagactttatcatttaagccatgagatggctgaggaagaaaaaaccagatgcctgtttaagtcacctttagatttccacttcttcttccactgaattgtccttgaaatttcctttggaaataaattccaaggtaataaaaggcctcagtgcaggtagtgtttttttttgttttgtttttt

SEQ ID NO: 245 - DNA, 500 bp, Homo sapiens
  source 1..500: mol_type = genomic DNA
cccactcaaaaaaataaaaattttaaaagccattctatattaaagcagaagggaaagagatattggtaagaatccagctggccttttgtgatctgtgtcagcctttcttttgatctcatctgctgttttaagcactttacactgtagccccacgagaacactttgcactcactaagaagcagtcccctttgctgcgccccccccccaccactttgcttatattctgaaagtcttttgtttcctattccactgctcttacctctaacacactgcctctaacacaccaacctgcagttgtagttattacacaccctccttggttctttcatctctctatcacagcccttgttgtggtttagccaatatattttagttccacagctaaattttcataccctctatgactctctaatcccctgccacacttgcctactataatacattatatatataacaaatgtttgatacgtatttattgaattccattccagaactaatgc

SEQ ID NO: 246 - DNA, 500 bp, Homo sapiens
  source 1..500: mol_type = genomic DNA
tatagtaatgttaaaatgtcatatccagtcaaacatttgtttgtgtatgtgtccttgcaactgttagaaatacttgtagtgaaagatgtcagacactgaggacatccctttgaaatcaaaggagctctctctttgattcagtggtttccttttctctatatagcttctctttctctccctttctttagtgcccacgaccttctagcataattcccagtctttcaagggcggagttgccccatccggcaaggtcctaggatcccggcgctgtgggtgcggctcacacgggccggtccactgcatactggcaagcactcaggttggaggccgggttctgcacgctggcgtagccgaagctggagtgctgctttgctttcagtctcaggctggccaggctcgagttacacgtgtccctataaacatacggaggagtcggcggcgcgtaaggacaggcaggcgtcggcaccgcggaattcagcgacgggctactcaggttgttc

SEQ ID NO: 247 - DNA, 500 bp, Homo sapiens
  source 1..500: mol_type = genomic DNA
tgtgaaggcttctgccaggcatatgggacaatgttttttcaatctcaagggcatcctgttaatgtatgtttttggaaagtgccggaacacagccattgctcctggattcggattttcccaccaatattaattcctgcttgagagcaaaactcaggcccgctattaaaaagacatctctttggtccctaattgagaataaagttccctctaaaagttgtattgctcttcctaaatcaatataccaatactcgcaattttagaaatatatagtgactcgggagaatgtgcataaaatagatacgtttaaaaaagcttggcgcttaaaactaaccctagtcactatataggtgctgggctttccctacttttgggggctgtctggaacatgttatgtgttttcttgaattactccgtgttttgaattcatttgagttagcagtaaaaacaggcaaacaaacttgctcaatttgttttgagtgctaaatcccttcactttgaaa

SEQ ID NO: 248 - DNA, 500 bp, Homo sapiens
  source 1..500: mol_type = genomic DNA
agaacttgcactccctagccgagatagcgaagtcctcagcgctgtggctgatgactcattagcagtgagccacaaagactctctggaagccagccctgtgctagaagataactcttcacacaaaacccctgattctctggagccaagtcctctgaaagaatccccttgccgtgactctctggaaagcagccctgttgaaccaaagatgaaggctggaatttttccaagtcactttcctcttcctgcagctgttgccaaaacagaactcttgacggaagtggcctctgtgcggtcccggctactccgagaccctgatggcagtgctgaggatgacagtcttgagcagacatcgctcatggagagctcagggaagagccccctttctcctgacacccccagctctgaagaagtcagctatgaggttacacccaaaaccacagatgtaagtacaccaaaaccagctgtgattcatgaatgtgcagaggaggatgattcagaaa

SEQ ID NO: 249 - DNA, 500 bp, Homo sapiens
  source 1..500: mol_type = genomic DNA
ctctctatcttgaaaatatcctctcttggaacccgctattttttaaattgccacatttctctttcctttcttgcaagattaaaccccgcacgcaggctacacccactcttgccatttctactctaccaacccttttaataacctcttcagaatcaaaccatttgtgttttgggagcgggatgggggtgggaagataaaaatgatgactttcttcttaaaatagcaatttaaaagcacgataaaatttaaataataactagagctgtctgaagagaacatttcttttcaggcaaatgtgaaattaagtaatctgtttcatgttgcggtagacatttttctgaatggctcacacagaacataaaccttaaaagccaacagcatactgtggggggaataatttctgtttaccctcagttcagtgttctgtcccattaacagctctacctctaaatatgcatgacatttcctttcaaaaattttctgtttaatgtttcaaatgc

SEQ ID NO: 250 - DNA, 500 bp, Homo sapiens
  source 1..500: mol_type = genomic DNA
catgcattatccacaacctctttccttcttcttttttgtttactgctatcattattcatcggataaacacatccatgtctctgaggtctagactcatgaactctggaggtcaagcacctgctctgttcatccttttggatgagaaacatttacatgcaacggggcattgcttggctggagaaacaactcttccgactcagctaacctgtatttctggaaaaatcagtgagtctactagattccgtaaaatgccattcctgctgactcactccctgcactgggccagtctgttcacctccggtgagtctgaacatagttttctcatctgtgacattacaaaatgcagatggctgcctctcaaagtcccctggcttctaaacttctctggatacaatgcccataaaggaggtttctaccattacttttttacttctctacttctctattattttccaagacttctaggacttgaatagatgctttgaactctaccttgtgtg

SEQ ID NO: 251 - DNA, 500 bp, Homo sapiens
  source 1..500: mol_type = genomic DNA
ccccaagcactgcagcgtttctcccaggaggctgggcgagtccgtagcggaagtcggagcggcagagcagtgattgggtgcggccggcaccgtctctgggcttcgacttccgggtgagaccgtgaaggtgtggcgcgacgttggagaccggggcagcgccatgtaccacagtggatggaaggatgcgcggtgcggcggggcagctgtcctcttctccccggacccagcgcctggagagccagccctgcagggtgggctgggcgagccaaactgcgttcctggtgcagggcttcgggtctccctaacagaccttatacgctgaccggcggccgccatggcagtgtctctttgctcagacatccagggacgaccacattcgtccaacagcggtcgctccaccaatcctgggagaagcgaatcgttttctccgcgtgccctgtcagccgctcatggtgcccagagaggaattttagtggcagcattccggctgtcacgccacc

SEQ ID NO: 252 - DNA, 500 bp, Homo sapiens
  source 1..500: mol_type = genomic DNA
cacaagataatgtgttttatataccctgttatagatacagtgggaatcaacttcactcacagcaactttggattggcttttcatctttatttggtggcaatttgtaataataaagcaacagaatgtcttcatgtattttatcattctatctcttaattgaaacatttctgctattttatttttaaataagccagaatggaaggcattgtagtaatactttttcagttatgtaaaaagaaagcactttaaccacagcagatatagcattcttagtactgtgaattagtaatcgttttaaaatatgtaaatcatattgtattttattggtgggttattcttttgttgttgcccttagtacagtagtaaacttcttgaattattgttcaaccctttggagatattgaataaatgtacatattcttctaggcattcatttagttgccagtctgaaaatattgtttgaaaaggtaagtaagaaaacggtcaaagatgccgaaaga

SEQ ID NO: 253 - DNA, 500 bp, Homo sapiens
  source 1..500: mol_type = genomic DNA
ctgaagtgtgtgagcatttcaggtttaactatattgttcacctgaaataagtgaatacatgtaagtgctgaccccgtaaagagttagatatccctgataggaggaatttctgacatagtgtcaacaagttcttgcagatccagatcaagccagctgcaactggggtaacagaatcctttcacggtgttacgaatggatgattttcagttagaggctattagttgaggattacagtgccaggcaaaatgatgaagttcaagtactttggagaaaaattcatctctgtgttgccatttaccttctagacattctgaaacaaatttggccatgagctagaatttcctgtaaaattttaacagttttaaaggagtgtcttactgcacaacaaggaatgccttggcatgagaaaacatttttggaaaaggaagaatcatgggagatttttatcaaataatgaagaactagaagggaggcgggacattgtggtttgaaaaaatggc

SEQ ID NO: 254 - DNA, 500 bp, Homo sapiens
  source 1..500: mol_type = genomic DNA
tggtggtgatgagcgggccaagagtggctgcctccctgatgtccctgccatgtgtcccacacaggctgtggcatgggagacaaaaggccacgctgaagtccacagggctctaaggcagcccctgcctcctccgcctgtgatttgctagtgactgtgagtcattcactcatttcttccatctgataaagctagtggacatgaaggggaaatggcaaagttttcttatcatcttaggagccagaagccaagtctactttcaactgcttctctgttaagtcctccgtcagggagcacttatgagggctcagcgtttggaagagaaagtgcccgattgtgtagacaccacagcaaagggggaagaagggagttaacacaaggaaaacctgttagagaagagaaggaatgtgttagatgtttttctcacctgtcacgctctatttccttacctttgaacaatttcatgtgttatacctcatggcagaccttaaaaggcaggttgt

SEQ ID NO: 255 - DNA, 500 bp, Homo sapiens
  source 1..500: mol_type = genomic DNA
gttcaaagtgacacactaaccaacatgggagccacatgactttctggcttggctactgcccttcagctgaactttggcttagaacacaaggctcccagaggcagcctggcacatgccgccgcgtggagtgtccggtggcattttccgttgctagggcctctgttgcttcacagtctagtgaggggcagctggggatcagtgacagggagtcacctgctcaccccacctctggggacagggaaaggaattggctgctgtggtggccgctgcctttctgagcttgtgctgggactccctgtcccctccacagttgattagttttgcaaatgtgtgtgtcacgcgttatgccaagaaccacagcagggaaactcggacccccaaagggagtttgtgctggaagaggtagagaaggaatgtgactcttggctaagaggacacaaaggcaagggcaggaaggaaggaggaaaaaaaaaggaaggaaagttattacctctgggtag

SEQ ID NO: 256 - DNA, 500 bp, Homo sapiens
  source 1..500: mol_type = genomic DNA
tattaaatcgttgctcaaaatgacaaaccttgcatgtgtgggtgctgggctttggccctaagcagtctggctccagagttcgtattcctaatcagtagtctacgctgcttatgctgttagtctattataagactctgacagtcctagacggtatttccactttgtaagattcagcttcttgactggtcaaacaggagaaataaaaatttgtgaggtagtggagaacatcaaagcagacaatgaatggtgagcacattagtgcttagcacgtggtagtgagttgatgctaaacttatgttggttccctgatatttaaatgcctctttctaatcaacaatagataatgtgaaatacatgtacacattgtttcaaactaattcagattcttcaaaacacatgtggatagcataaagggagggacctttcacatttccagatttacttataatcatgatcccttgccccacttgccagacactgtaaccacttctaacaatggt

SEQ ID NO: 257 - DNA, 500 bp, Homo sapiens
  source 1..500: mol_type = genomic DNA
ataggttaaagaaagtagattgggaatacctaagccagggaagggaatagggaacaggaggacaaagctataatactggagaaacattgggaggttagagcccaagaacacttgccttgtaaagaccaagatttaatcagattgtagaatgtccctggtttcccataccttagcactacaccaacagggcttcagtataattgatagatgcaggaggcagataagggagggtccctagagagtctctgacctaccccacatgtgtttacatcagatgcttttgtgcaaatgagggaacttacctaggaccttgtctggacatgcctgcaatggactgggggcctgactgcgcactaggaattcatgccttatgcagcgaggagaagcctggccatttcagctcatgtgtggtggcctggtgttcgttctgtgaggtgggagcctgttggcaggacctgctcctttttgatgagagctttcttttaataaattttactctt

SEQ ID NO: 258 - DNA, 500 bp, Homo sapiens
  source 1..500: mol_type = genomic DNA
agtgaggctgttccacggtggcacaggacacgcctgcagctttgtgcctgtgaatctcaggagctgttttctggaaagttccataactcagcaaaactgactcacaaacaacagaaacttcaaggctgtcctaagatatgggtggcagaagaaaatgtgccccaggcatgggcttgtgatgccggctcttcctcctggcagagctccccagaggaaggctgggctgggcagtcagccagacgggaaagggggctgaggcgtccaggctgcagagggtgccggggtggagagcggaagagagagggagtcggtgccttaggaggctgcgggcgaggcgagggcagagtgcactcgctgggggtcaccctgccccccaggactcctttcacaggacagagaagctcctggtgagcggggctgctgaacgcaggccccagggcctgtaggacccttagggagacgggtggctctgcgtgtgggtgtggagagaggcctgtggg

SEQ ID NO: 259 - DNA, 500 bp, Homo sapiens
  source 1..500: mol_type = genomic DNA
gggtttctgatgatgagttgggatttggttttcattcttctggcctcgtagatgagtggccagtttcatttcattgattggctctatcttcagtttatgtgctcattctttccattggaaactcctttaactcttctgctgaaaatgttctctagggttcaactttagggaaatcttagcaaattttatttattactctagctattatgtttattttcataacagcttttctgaaggaggacatctaacacatctaggtgttcataatgtgagcctcatttgtattttcagagaaaagttttatcttgagtttgaatgaactgtggaattagctgagttaagagactctcatttttgctatccatgaggcagaaaagtggtgtgaaggatatatgacttcagccaattgactactgaccagtctttctattgtttaggccataggaaatagggcatttggagacaggtgctaaggaaatgagtagcacttttgtgtgtgt

SEQ ID NO: 260 - DNA, 500 bp, Homo sapiens
  source 1..500: mol_type = genomic DNA
ttggaacataatgtcccttggaaagagttctgtggtttttctctaatttaaatttgaggccagactgatgaatgctatgaccagggattatgtcatagaacagagaaatacagtaatggctcacatattagaaatagaccacaagctagtatctgtcacagtgttgctaggtactagatagttctttgtaataaatgaaagttgtggaagtttcatatcgaactatatctagtcagctttctgcgatggtttgaaattaaaataattactttaattgaggcaatactcagaaaaaaatggttccttcagccacccatgaatacttctcttatccgaatttaagtcattcttctgccacaaactttctgtatgatctcaaacaatttactatttatttaaatgaaaatactaatatcagctttcttctccataaaactattcagaagaacaaaaaggatagctgtgaaaacttttaaaaatattttttcttcttttatgtt

SEQ ID NO: 261 - DNA, 500 bp, Homo sapiens
  source 1..500: mol_type = genomic DNA
ccacaccttcagtcactctctgctataatccttgccagatctgtcatttcagtgcacaagcttgcttatgttgcctcccagcttgagaactgacactgactccccattgtgcaccatgtttagcaaggactgttcagcctgcattgtgaagccctctccagggaggctcaggtggtctgtctttctcatcccccctcgccctatgcatatcatcagctgtggccaaccactgctctatgctctgcaaatgggccacacaatccatttctgtgttttaccgtctctactgttcctgctacatgtattaccctccctcacctctgccaagatcacattatttttttcaaatgctgccccctccttaaagaatggtgttatttacaaatgtcatttctccttcttttgaatttccttgacatctttctctttttttgtacttttcaaacacttacattctgccttgtattataattacttatgttcttagctaagttccaatg

SEQ ID NO: 262 - DNA, 500 bp, Homo sapiens
  source 1..500: mol_type = genomic DNA
cgactccatcagcataggcaggaaagtgggagtgaggaaaggcttagagttttccagcctggctggggtcagacaatttgcctggggaaatagtgggagctgaggttgaaaagaccgattggcttcacgtttgtggcaggccttgtccaaaaagcaataggaagtcgttgaaaggttttgtgcaggggagcgacaggattaaggcactacttagtaggaagtcatatcaaaagcagcaacctgacaaatggcaaatacgacagaaggaaaaaaaataacaggaattttcttcacaatgactcgactttgaggtaataaatgcctgagccacattggaagcaggggtctcagaaggaaggcgcagatgggaaaggcttttctgggcggtggcgtttcaatgcaaggagggcgcttgaatcactgacagacttcaagttaagggagttttcgtggctgaggttagtaagtcacacgcacagctctccaaaggcatgtatggg

SEQ ID NO: 263 - DNA, 500 bp, Homo sapiens
  source 1..500: mol_type = genomic DNA
aatgataatctggatacaaatataaagcccattctcatgtttaaaaaatcagcttggcaatatttattgctgattttagcaccgttcacatctaataatgatgagtcttatttacgatggaatcatgaatactgtctctgattattcctttgataaccaccctttacttccttttacaactctactctcttagctctcagcaaacttaattttcttttttctctaatttctttttctcttttctttgccacttctgtctgctctctaccacctgtttctcaaagttctgttattttccagttcatactgttttccttggaacatataaatgtcttccattcctttaaaggcagtatctcctcatatgactttcaaatagacttctcctaatctccaaataaattcttattcctttactgtattcccaacagcctcaaaaatataaataggtaatacctatagataaacattaaactcaaatatgttcactcccttcatgc

SEQ ID NO: 264 - DNA, 500 bp, Homo sapiens
  source 1..500: mol_type = genomic DNA
ttcttgctctttggatttagtaagtgtgatttaagatttcagtgccttggattcccctttgcaaggtgacaactgtggtggagtcacttctacctgagaatgttaattcactacatctactctttattaaggtgaagagaaagttctagtaatatcaaatgtgattgcctgtaatatgagaaatgaaaaagaaacttttgcaaattgaaatctgaaggaaaataaaattttggattctgtaagattgtctcctctaaataacattgtactatatataattcatttaatttttagtccgactgtctgtgtgtgtgtgagagagagagagaaagagaaacagaattgaatgtgtgtaaagagaacatgaattttctggtactacttatttagcaaagggttgaaaagccactgtattcagaataagtatgatgaaatgaggttggaaatttaaaataatgaaaaagttttaaaacaaccatcataattaattcaatagaata

SEQ ID NO: 265 - DNA, 500 bp, Homo sapiens
  source 1..500: mol_type = genomic DNA
tcaaaaacagatgaatggaagaaatgctcagcttcataaggaataagtgatgttgacagcatgattttgttttgttttggatcccattatgccactttgtgacttttcttgggggggcaggggctatgtttggctgtgtcagagggatgagaaagagtggcttccttcttgaaataaaatcatagctgcatagagccaattacttccagaaaaggagaaatgaagtcgtagtagaggaggaggctgaagacttaggggctttgatgaagctaaagagcaggtaccatgggtattaggaactggaagaggtgggagaaaagattacaggcagagagaggaattgtatgtggaaacattgtgggtggagcagtgctgaataatgttgaagtcaacattatggtgatgtgagtgggcaactggcatgaaatggatagagagatctctgaatggaaaatgggaaactaaaagacttgagtatcagagggtaactaacgttaaga

SEQ ID NO: 266 - DNA, 500 bp, Homo sapiens
  source 1..500: mol_type = genomic DNA
tttgccaaaacctcataatttgggaaagagacaaataatgagaccacgttagcatggtgtggtgagttaggcataaacaatgttgctgtgggattgtgtgggaagctgctggcctatttgaagtagctggcaataggaaaaactaaatcctcctttttactctttataagtgtgacttttctcctgaggaatgtttgttttagagaaaacccacaggtaagagcacttcaccatctcttcatcattgccagggcatccactgtctaaagctttaattggtattggggcctgcagaaaagccataagtatatgagaaactgagggaaacaaggtggaaagaagggatatgaggctggggtgtctgtaagaaaattcagggcagctgttattcttattcaactgatgtttcatgtataatgctaagctcagcaggttcttccttaaatcaggggttcttaaccaggggttcgtgaatgggctttaagggtataggtgaactc

SEQ ID NO: 267 - DNA, 500 bp, Homo sapiens
  source 1..500: mol_type = genomic DNA
tgaaaacattagcagaaaagaaagggcaaaatcaagtgctgtgaagggcgttatagctgttttttatgtctaatttattttaaaaggaaggaagaaaaatttcgaaataagtaggacaaaatgttaattttttaaaattaaattaaattttaataattgacataattgtacatatttatggagtacatggtgatattttgagacatgtaatatatagtgatcagatcagagtaattggcatatccatcatcttaaacatgtatcacttctttgtgctgggaacattcagtatcttccttctagctatttgaaactatagagtatattgttgttaattatggtcattctacagtggtatagaaactagaatttatttctcctttctagctgtaattttgtatcctttaacaaatcttcccccatccctatctttctcatacccttcccagcctctagtattctctgttctacttttttcttatatgagatcaactttattt

SEQ ID NO: 268 - DNA, 500 bp, Homo sapiens
  source 1..500: mol_type = genomic DNA
tgagcagataaagacgaggagctgcaattggtggtaagaaggaacaggattgttgtgtcataggcataaatgtatcttagctatttttaaaatatagaaataattattggttcctgagaagaagccgatggttagttggtcagtggattacttcctgttgaacattagatgatataccaaatgctgggttaagtccaaaacagttttacctcagatcagtctgacggctttgaggaaaggaggaggcagtcacatcttatgatttttgcgaggaaatatcatttctgatattaccttgagtttggaagatgaaagaagactatgtgaaatattaagctttccaaattatagattctttggccatgtgaaaaaacaagcatcattcttcatggcctcaccctgtattagctgtgacttgcataaaatggctaagcttctctacacagtcctgatgacttgttgaggttgttctccaaagagaaaataaagtgactgtttca

SEQ ID NO: 269 - DNA, 500 bp, Homo sapiens
  source 1..500: mol_type = genomic DNA
gtggaagagaacacataattgtggacttgagtagggtctattctgtctgtggctgagtttaataaagagttatttcatgtggcaggagatcctctgtatatgggcaggaggaggatttccaagcatgcaggaaagatgggaagctgcaaataatttttgttagggaccttgaagtgagctacctctcacactgtaaataattataacatcttccatcaaccagctttcagaagaccactgttgcgctggtcctatttaaacctctctggaagaaatcagggaatttccactggcatttttatttggtttatagtctcaaattgggtttaggtgcaaataacacttaccttgaagaatttatctcagtcttacttacctattttatatgatttttcctccaatcctgaacctaattgaaggagcagcattctcacaggtattatttctcaaagagaaattcataatagagtacgcaaatccctgaaaatgaccgagataag

SEQ ID NO: 270 - DNA, 500 bp, Homo sapiens
  source 1..500: mol_type = genomic DNA
gagagattatgacttgaaatctgttttaacaagagttatctggtgggcaagaggtcaagtcctggaaggtgaaaaaagaaagaagaatgagaggacactagagtctctggaatgagagctaatgttgctagcatgttattatattgagagttactaactctcaataactcaagaatcattgccaggcacagttctgagtgttttacatatattaactttcttaattttcacacctctgtgaattaggtattatgttttattctcactttacagatgagaaaactgatcacagagagtaattcaatcgtctaggttacatggtcaattagtgttagagccagactttgatattacgtcactctagctccagaatccacattcttaaccagtgtgtcatatccctctcaggaaggagccaggtctaagaggtcagaaaattctcaagattggcactaagggttaaaatcttatgcgaaatcagagcattttgttcactactg

SEQ ID NO: 271 - DNA, 500 bp, Homo sapiens
  source 1..500: mol_type = genomic DNA
gcagaaatcacccgtcttctgcgtagctcacgctgggagctgtagaccggagctgttcttattcggccatcttggctcctcctgaagatatttttaaaaaatagattctttcaattttgggggagcaataactttaaaaatcatattatattgacaaaagcatacatatggatgatagctattcaattctggagtggcttttttaccatcccgtatttcataatcagaataactttctaaaaaacaatttttatcttgccactctcaatttaaaaccatttaatcttagctccatttattatatgtattctcccttacaattaaaaccaacttatgatttaattcctgaaaagggctttgtacatttctattttctgcctttgctcagatatttccttcttcccataccttctatttctatctgccagaaccttatacatttttaatgactaacttaaatgctacctcttcgtgactattttcccaagtatactcattag

SEQ ID NO: 272 - DNA, 500 bp, Homo sapiens
  source 1..500: mol_type = genomic DNA
acgcagaagctttgactaaagcatcttcacaacttacatcttcaccactttcttggcaagtcatgattatagttataaatttggaatgaaaaataaagtaagactctttgctattctgtgattttcaaggaaaaaataagctgaatagaatgtatgtgctgacataaaaagatattgttcatatacatttttttgccactgcctctcaacttgcttctttcggactgctcatgatagaggtttaaaagctttgattctgaacgcgcagccctgttttattgataaaaataagccctaatatttttttcctttgctttatctctttttatgtgggcagctgataaattccagaattcctacgggatgttctaatggaatagcaggttgagctgccagcagtgtcagtattacaagataaaaacataatgccatgaacctatatatcaaatgttgtgttgcaaatgaaacactatctacttcatgtaaaatcagcttcttag

SEQ ID NO: 273 - DNA, 500 bp, Homo sapiens
  source 1..500: mol_type = genomic DNA
ttttgttaatgtacatgatcggttatagaagacaacctcaatacagcatggaataggagaacattttaaaacatctgcatttttactgttttccaattctcatcaggaatcttgttggcccctcaacatgtaatctgacatgacctaaataatacccacatttggagtggccaaaatgtcaaaagatttcaagatattacaaaaacaaaaatatccaaagttcaaacatatttttacatgtgtggtccaccaccctaaattttctgaaactaaacatgaagatcattttcgtgaaaataataaattatgtttttgctagcttccatttatatgaaatcatttaacacatattattttagcatacctattacttttccagcacaatctaggttcttcaggaaatttagaacaaacacaagagccagtctctgaactctaggagcttttatttcagcaggaagattatattgtgtgcacacaacatcaaacatcataaggca

SEQ ID NO: 274 - DNA, 500 bp, Homo sapiens
  source 1..500: mol_type = genomic DNA
aaataataagtttttgaataaattgtgtggcaggaatagaataatcctaagttgtcaccaaaacagagaaatatataattaacttagcaatcattatttcccacatgtatgactcatttcctaagttctttcatgttggtttccaattgtcccccacagatcacctattctcccccatccactttctctttcctccttttttcctgtaacccttagtatgacctgacatcatatcctaacatttttttttgttgactcactgcccccataaaattatgagttccaagaaggcagggatgtcaagaggctggggaaatagctcatgaacaagaagaactgtacctggcacatggtagaatttcacgcagtatttgttgaacgggtaaagttagcaaattagaaaatacagataaaggaacattatccttacctcttcccaccaccactatgagatgatatcacctgcaaatatctgtcagacatttctgtaagtgtaacta

SEQ ID NO: 275 - DNA, 500 bp, Homo sapiens
  source 1..500: mol_type = genomic DNA
aaagtcaggagtttaagaccagcctgggcaatatggtgaaaccccttctgtactaaaaaatacaaaaattagctgggcgtgggtgtacacacttgtagtcccagccactcggtaggctgaggcaggagaatcacttcaacctgaggggaagaggctgcagtgagcggggatcatgccactgcaccccagcctgggtgacagagcgagacttggtctcagtaaataaacaaataaatactcaaacatagggatcttcctgttcatagcatcctgtttcttctcagctctgcctcctagcagtacatccaggcactaagctatgccataacagatatgaactattaaagtgagtaaactgtctactttattttccaagatgagcatggtttcacgttatactgtctcaaaactcctagatgctaatattatcaagtgattcagacaagaagcagaacgctgaaaatgtagaacaaaaggcagatcttgataacagaatgaga

SEQ ID NO: 276 - DNA, 500 bp, Homo sapiens
  source 1..500: mol_type = genomic DNA
acttgccatcctgcaaagacctgaggaaccatcctttttctcagagtcctctcaagaaaaagaagtctctgcaacttggagcaatctctaagtagctgtctgagccccctggaagagggctgttgtgggcagctgcattcagtgtgagcaacctggagtgggcctgtcctcctgctcgttcccaggttcaggcctggaagagggagttggaggcatgagagaagccactgtggggagagcacctggttcttccaaggctcggggcatgtgtggtccctggctgacttgggtgtcctctggtgtgtgcggtcagtcttcttctgactgtggatgccaaaggggaggcccttatctcttagcgcatgactcatctcttcgcgcatgactcatctctttgtgcatgactgtattattctcagcgtgtcatgtggttcctgtgcataactgagctcaatgaatatttgctgatttcagggagtgtgttagcctaggatgctacc

SEQ ID NO: 277 - DNA, 500 bp, Homo sapiens
  source 1..500: mol_type = genomic DNA
gaacactccattgctggttcttgtatgacctataagctaataatttttcttaacattttaaaataattgagaaaaaaatgcaaagaagagtaatacttcatgacacatgaacattatatgaaagtcagatctcagtgttcataaagttttattggaacagagccatgctcatttatttatgtgttacctatggcagccttcgagctaggatggcaggttgagaagttgcaagagaaccacatggcctgtaaaagctaaatatttactctctggtcctttagagaaggtctgccagaactcctatacttgagattccttttccattggatgtctcagacctaagacatgtttggacttgctaactcattcagcagctgttatatcacatgcctacagcatgccagacacactgctagacacaggtatccaaagatggacatgacaccttctctgttaggagggaggagctcacagcctagagggtagcatgggcctgtcca

SEQ ID NO: 278 - DNA, 500 bp, Homo sapiens
  source 1..500: mol_type = genomic DNA
ggttctccatgcaccacatttcaatgattcatgctacttcctgggccacagttctcctccataaccgcacatcctttttcacagactgtgagtgatttcaatagtatatgaaaactatgactcagaggctggaaatcaaagggttttctttgaaggccggaaaaatttcatctcaaagaaagtgcaacaaacgcacaaggtagtctttttctctgaatagagacatgggtttaaaactaggaatagtaaatgacacaggcacagagacgggaaaaaagccactgttgtagatatcttgaaagtgcatttggctcacggagggtctccagggaccacttaagcccatcatttccatcccacctattgaagcttattgattagtacagtcgcaaaacccttcccatgtgttctctgtaaccaaagttctctaagtaaaaagcaaagcccaggaaacagctttaaaaggagaagtttacctaaagatgagaaatactaactgg

SEQ ID NO: 279 - DNA, 500 bp, Homo sapiens
  source 1..500: mol_type = genomic DNA
aagaaatttcccatgtctgtatcataaataccttaaaaaggggggacaaaatgtaaaaaaatgcttttcagacattggacaatagataggaaaacatttttactcagagtagttaagcaaattagatgagttttattaatgaattagttttctgtctgtagttaatatctggacttcaacatagggagaagaagcccaaacagagactgaaaatcttattgagttgaacactagaggacagagatgactggagtttgtggggaagaataccagaaaagagggagctaagcagagaaaattctccaaaaatctgtgtaaggtcttccgtacctttctttggatagatgctgatttgtatgtacataggataaaactctacagaactgtgcaaagaacaactgctgaggacctaccagctgaacaaatcccattgctcccacatagctgggaaacatttgagtacctgccacccggagtggagagaacatagtaaaaactga

SEQ ID NO: 280 - DNA, 500 bp, Homo sapiens
  source 1..500: mol_type = genomic DNA
cagtgtgcaggtttggatatactttctttctggaattaaatcaaagtcagtctctggcctgtggtctagagggcagaaaagtttagtcatagcttggtccaactcctgagcaatgatattaagcttatgatttctgaaatgtttatgttagctctagccatgccgtttactgcaattgttgacactaacactgttcggtccagatgagagaacaagatcagcaactgagattgttttgcactgtaagttctactcacagatgttctcatactaatgaaagccagagtgtattgctttctctgatcacatgaccagatagccaaggttgttgcaaacattcaggacagctttattttccaaggttaacagttactggggaaaaataaggtgaaaataatgtgtaagaggtaacttgctttcttgagcatatttcagaggcccctcaaaacattatatttaaaaaagagtgctctttttagtagtgtctgctttgcaattac

SEQ ID NO: 281 - DNA, 500 bp, Homo sapiens
  source 1..500: mol_type = genomic DNA
catgggactggaagctcgagtcccaggtcatttttctgccactgggaaatgttttgagctctgccagcatctgctcacgggccacaagttgaaagtgattttacattagcaacagagattcaaacaaggaacatccaacaaatcctggtgacttgcagcagtggttctcagtgtgctgtggaccagtagcagcagcattacctgggaaatggttagaaatgcaaatgcttgggctccaccccattcctacctactgattcagaaactctgagggttgagcccaggaagtggttttaaaagccctccaggcgattcagatgcaggctaaagtttgagaaccactggcctaaggaactctggcagtgggaatgaagaaaatcattgcagggttcttaagaaaacccaggtgtggctaaacagatatgcctgtccccatttcccacctacccccagcccccaccaccatgatctaagaaagcaaaagctcattgaggcaggtg

SEQ ID NO: 282 - DNA, 500 bp, Homo sapiens
  source 1..500: mol_type = genomic DNA
tcacctgggatgacattggtgtcatggatgtgaagctcaagtttattcggtggcagtgcaacacgatgctccagtgctgatgccctagagccagaccccctgcattgacttcctaaccagctccacctcttactaagctctgctaactcgggcagcttagcctccgtaatgcatgaaggttttttcatctataaaatgaagctagtaataattccccacggggttgttgtgaggatagaatgagatgatccgtgggaaacacgtggcaccgctgcaagcacacagtgagggctcaataaacattagctggcatacttaacagaggtcaggggttctcaacttggttgttcattggaatcatccggaaactttttaaaaatactgatgcttggaccccaccccagaccaaatgaaactaagtctctgggatgggcagtttttaaaaaagctcttcagggccgggtgcggtggcttatgcctgtaatcccagcactttgtga

SEQ ID NO: 283 - DNA, 500 bp, Homo sapiens
  source 1..500: mol_type = genomic DNA
ttgctgttttgtggaaaattttctttctcgaagttgtccagctgtgagtcagtttctttgcctgagaacattgtctgcggcagcagcagagctatatttttccttcagcctctatcactttttttatccccgcaaaggaaaaagttagctacattatctgacttgtggatttgattttgggtttgtaattggctgatgaaagctctcctgactggcagtgggagggaaaataggagaggagaagaggatttccattgggaagcagtggtccctactgcccagaggggccgtaggtagtggttgccctcagttttgctggggcagtagttgagttgaacatgcacagtccctgggttttctccccctggactgccctatcctttaagaagtaatggactgagtgttgactctgtgctgagtactgttatgtgctttatgtattctttctgtccttccaacaaccctgtgaggtaagaatgagtgcccctatttgaaagctt

SEQ ID NO: 284 - DNA, 500 bp, Homo sapiens
  source 1..500: mol_type = genomic DNA
acagtaaatgttggaaacagaaaaaaacaggcaatatgtacaaatatataacttctctaatatgaatattaaaaagaatttataaataatagaagcatgctgattgttttataatattttcaaattcaaattaagaaaaagataatgaagctgtattcaagaatattagaagtattgtgaatatatataggactgaaaatgattttgtataacagcaaaaagcaaaattgaatggcattctatttaaaatgctttcttttttatatttaaatgtattattttagagaaaattcatcatttaataggtggctagcaaactgtttcaaaaagcaagataatttacaattgagtatagtatatcagcatttccatattttgcatcatcttgatttaatatttctggtgcttcagcaacgctagtgcccattcttggtaaccacatcaccacagaaatgtaatatatgtgttccgtatcgtttcctgcattatgtgtgtgggtt

SEQ ID NO: 285 - DNA, 500 bp, Homo sapiens
  source 1..500: mol_type = genomic DNA
aagagttgatgaaaactcgaaatagcttcaagccccagtctgtgttcaacatttttcagtgagcggaaggaagagagggagtttttcataaatcagaatccggtcacctggggatcaatacacagtgctattgacatatatgctggaatgttaattttcagacatagtacatctctggccatccttctggtgaaggctaatgctgttcacttaaatcaagttttttctcatcggaactgccggtaattatccaatccatctaaaaggcacgctcccttttaacattaaccacagtgtcagattgcatcagccacattgtgttctggtgactgcttctgcagagtgatgaatgtgcgtgtttggagttcatagtccgactgtctgtttgggcagtgggcagttcagtgaaacaaatgatcaggaagggatctatttatttgggacgaacattctccttattgatccagtcacttacatttccaactctctcaccttgccac

SEQ ID NO: 286 - DNA, 500 bp, Homo sapiens
  source 1..500: mol_type = genomic DNA
acagcacccagccctgaatatccctctttttaaaaataccttttcaaatttcaccaacttaagacatgggagcttttaaacccaaaacactttatttcttaaattactcaagatacgtcctcaaaacacagaacaatcaaaagtcaactggactgttttctaaagcagaaaaatgcttttcaggcaataatagaaaaactaaactagtaaaagggtattaatccaatcagttcagaatttgtaatataattttgaaacggccacttcatttgagaaaaaatatctttggttgctatttttcaggatctcatttgtaaagcaaagtcaattttaaaacattttctctccaaaccaaagtaaagcattaaggacctcccaaagtaattcttatatatgaaaaaagtatgtttatgctattttatgtagcataggtttatcatgtgttacacatttttattaccttattttacttgttagtaaagatataaactataaagata

SEQ ID NO: 287 - DNA, 500 bp, Homo sapiens
  source 1..500: mol_type = genomic DNA
aaaaaaaaaaaaaagaagagtggacatttgtatgtttctcagcctatatctcacctttcatctttcaccaaagcttcatgattctctgtaaaacctgtctggtttcctaggaagccctctggactgcaggtgacctaggattgaactatgtttctcaaagccacaatccggtctctgtggtcctgactcagctggatttatgtgtagagggagggaaagaagaccacagcatcgtaaatcaataaagggctttaagcacatcctatgtgtcccagagtgacttaagcaaaatgcctgttgaagtcagtgctggcattatcagaactgttcacctcatgtctagaccacagccagacatttaataacactaatgactaagtgtactaagtccatgccacaaaccatgcactgaactaggggcactttatacagattccttcatttaactcgacaggccatcaagtggatacaattgccctgttttctagataaaactgaaa

SEQ ID NO: 288 - DNA, 500 bp, Homo sapiens
  source 1..500: mol_type = genomic DNA
gaaaaatgtaaagtcacatgttttagggtcatctcgttagactacaaagtcaacagacctggaattccgttcaactgaacatatatgattaatgagtgccaacaacaaacattctgctaggcttcagggctttctttcttttgagatgcagtctcgctctgttgccagactggagtgcggtggcacaatctcaactcactgcaacctctgcctcccagattcaagcaattctcctgcctcagcctcccaagtagctgggactacaggcacatgccaccacacccagctaatttttggagttttagtggagacagggtttcaacatgttggccaggattgtctccatctcttgacctcgtgatccacctgccttggcttcccaaagtgctgggattacaggcatgagccaccgtgcctggccagggctctcacataaaagtgattcaaacacaacagtgcacataggagcttacaattcagtcaagggaacatgaacaata

SEQ ID NO: 289 - DNA, 500 bp, Homo sapiens
  source 1..500: mol_type = genomic DNA
aacttaagaggctttgtgggttttgttctggtctgaggaacgttgtgggtgatgtaccatagcaaaccaaggccactgcccactcaggttgagaagataactgtgcacaccccatcagctttttttgttttgcttgccttgcctcctcccaggaacctagtaatatggaggctgaaatagacaaaaaaggctcaagttgacattgactttgaacttggaggtattgtggtggggtagaagcatcgagtgaacgggctgtagcttttcctgccctagtttattatgtgccatgattcaggctgagagctcaggtgttccctcagaatctctgaatccttcaggaaacgagaaatgtttgctcttcctcctaagaggaagtgactcaccaaatttgtactaaccttagttaggctgggtagtacttcttcccctcaattgtggagagtcattctttccgtgtttatatcctttacttagtaaaatgtggcatggctcttgtg

SEQ ID NO: 290 - DNA, 500 bp, Homo sapiens
  source 1..500: mol_type = genomic DNA
gcatggtgattctgacctggacagatttgtgaacgtcatctacaagtctttgccatctaatatctgatgagatttagggatttttagcctaatatcttgaaagtatccttggagttttcagatcctcactttgtccaaacttgctgtcctgttcctgttttcacagaaacttcaggtgtcctcacaggctgactaggaccaaggtatacctatctgaccattatgcgggccagtctgaggtcactgccctggggctgagacctgtgtcactgatttactagtgactcactgtgtattaccgcagctggcccttgactctgcttcctcagctgtagttcagtatgaactcagaaaacttgtttgtgacccgaaattagttctgtgttcatttcttactcttactcatgcacacatgactcatgacttagtccttgttttaaacttgtgcattagggtagctctgaattatgtcctccttctcctagaagcagaacctctta

SEQ ID NO: 291 - DNA, 500 bp, Homo sapiens
  source 1..500: mol_type = genomic DNA
ttgcttttgcttttagtcataaataatgcagatttctgtgtgttactatgagactctcacacctccctctaagcataaagctgaccgtaaacaacctgtgggaagccgcttgtggtttcagtggatacccacactcttctatccgtgattttaaaatacaaagatgtattagtttgctaaggctgctgtcataaaataccacaaactgtgtggcttcaacaacagaaatgtattgtctcacagttctggaggctggaagtctgagatcaaagcgttatgggatctgttcctttcggggccggtgagggcgaatgcgttccaggcttctcccctggcttccggtggtttgctgcccatcgttgttgttccttggctggtagaggcatcacccggatccctgccttcatcctcacaaaatgatctccctgtgtgcctgagaccgtattcaaatttcccctttgtataaggacagcagtcagattgtagtagtgccctcccta

SEQ ID NO: 292 - DNA, 500 bp, Homo sapiens
  source 1..500: mol_type = genomic DNA
ggaagacgttttaaaaagaaatttcattttactaactgccacactgcatagcttttctagggctgtggttagatttacgggagagaggcaccagagtggattacaacacaggactgaccttttaccacccggctgaagctcgaaaaacaaaaccaaatcccatcttactaaccatacctgcgtcttttctgggaaataccccagaatacaagtttgtttgttttttaagatggttttccttccctgagagaacaatcctgaaacttaagtcaataaagttctcatgctacataagcattttgcctcctcgggtcagacttgaggccttttcccccctttcttctcgaacatacatcaagtgccttagatcacggtgcatcctaggcaggttatgccattttaatctcataaatatgaaaataaaagacataatcagagcaaaaacaggactttttatttttaaaccaaaggaagccaaaatagcaacagagaagaaagga

SEQ ID NO: 293 - DNA, 500 bp, Homo sapiens
  source 1..500: mol_type = genomic DNA
ggaaagctgtgcagaactgatgataaatttaatttgtttgcagcaaagtccaagagcagatgctatggcactagtaccccactgtgaggccttgcctatcaacacatctgccaagacttgcttttcactcaaaaatccaaaaggtttcatccttctatgttttctgtctctggcagctgaaccagtgctgtcacatcacaaacaacttcttttcttaatatacacatctggcgttggcagttggactaacttcataagagcacatgatcatcactcattacaagattaaaaagtaccctatggcatcattgatgttttttaactttgatcttttgcagttgtgattcatctcggttataaaacttccctttaaaggaacatagccgatgacttattagaaccttcatcttaagtagcgtaaacatgaaaatggtacacatctttacaaaatgccatttattttctttgccagcttatcattttaagacatgacatcatac

SEQ ID NO: 294 - DNA, 500 bp, Homo sapiens
  source 1..500: mol_type = genomic DNA
atttctccccctggatctagtcggcagccaccaagggctcaccactctattaaaatgacacggccgtcatttcagtgaattgcagtatgtctggtttggcaatctgcagaggtgattaaggatccctgtgaaagagatgaggtttctggtgctgagaggagcaggtctactctgtgtaacagtattgtggcggaaaagctctgacaagagagggtacaacgtccttttggacaccagatcatggggccatgcaagatgttatctgggcttgttggccttggaaaaaaagatggtcttggaacaatttgggcaggaagacaatgggattctttatttcttggcacaggaatgaatgaatctttatcccaaatgcaaagcaggcattaaattcaaggacaataaatggtgagaccagcattccaggaacaatcccaggctttctctgtgtgctcacagtgaaaacagtcccacagggcttcaaagagacatgtggatttctt

SEQ ID NO: 295 - DNA, 500 bp, Homo sapiens
  source 1..500: mol_type = genomic DNA
acatgtcataatgaaaaagtagccagggtgaaagaggattaccctcaaagggaaaaaactaggctgctgactttttgacagcgtctttaaaaccttcccacacatagtgaaaacctttcaatgattttctgtcagtttctggatagaggcaagaacagcatagcctacaattctgtgcctagcctttttcggggccactgtccctgcagcggtctgagctccatggctttctttcagtttcttgtatactgctgtctttcctcatggctggggacttcagacaggatgttctctttgcctgaaatattttctacttttcccctcctttaatctagttagctaccactcgtccttcaggactctgataaaatgtccctttcctggaaagcatagtgaaaatttgttagtttctgtgtttgtttgctttcctgcccaacatctgacctccacgtcctacttaaggggactcttataaattatatcctttgactgataaggtt

SEQ ID NO: 296 - DNA, 500 bp, Homo sapiens
  source 1..500: mol_type = genomic DNA
agtgggaagacttgttaatagaaaaaaaaaagattatgggccaggtgtggtggctcacacctgtaatcccagcactttgggaggccaaggaggctggatcacttgaggtcagaagtttttgagaccaacctggccaacatggtgaaaccccatctctactaaaaatgcaaaaatcagctggatgtggtggcacgcctgtaattacacctgtaattacacctataatcccagctactcgggaagctgaggcacaagaatcactttaacctgggaggcagaggttgcaatgagacaagatcatgccactgcactccagcctgggcaacaatgtaaaactgtgtctcaagaaaaaaagaaaaaaaagattataatgaagctgaaaaaattttattgcctagtgatatcatagctgtcataatgttgcaaggcaacacattactcgcatgtttgtagggatactggtgtgaacaaacctactgcactgccagtcatataaaagt

SEQ ID NO: 297 - DNA, 500 bp, Homo sapiens
  source 1..500: mol_type = genomic DNA
actatttaagtttcggtgacaactcttccattttaaccaagaaaactgagactctgagaacttaagtaaccatgtccaaggtcacgtaatgagacagtgatgtttctggaattcgaaaagggctctttcacatacattgcatggtctcttgggaagttagagcttagacagtgacgataacagtgatgagctcacctgacagattgctctttttcctctgcagagacttgcttcaacaccaggaagaacatgaaagggtgactcataattcccagcagcagtgccagttcatgtgctgggattctgaccacaagcctaacaatcaggtcagggagtcagatttctgttggatttagaaaagcatctatgtgtttatgaaagaaacccactggatttttaatagttctgcagctcttggaggctctacatctaccctttctccccagccaagagcatggctatgggagaaggaaggcaggcagcaggcaggtaagtgtgac

SEQ ID NO: 298 - DNA, 500 bp, Homo sapiens
  source 1..500: mol_type = genomic DNA
tcacaaattgtactcgaccaaatactggaaagctcgagggtgagtagcatgcccctgcaagcctgtgatgattcatggcggcggagggaaggctcctcgtggactttcatgtttgcttttaagcaaccctcaaccctaagcgctggtgttcattttcagccgcagagaaacatgacttggggtttgattgtgaatcaacgattgggtgaagttaaaagtgaacacactgattctttaaactccaagttaaacatgtgctgctcctcttctagcactggatgagtcactgtcctagtgactcactgaaggattgtggtggaaatagaaaacagatcccataagaatttgggctgggttactgttgatcctttatgtcctgtgaagagggctttataatgctgaaactagttgtttccccacagacatttcttctcattaatgtattatttattgattatttgctgtatgtgaaacatgaatgaatggggagtggggaataa

SEQ ID NO: 299 - DNA, 500 bp, Homo sapiens
  source 1..500: mol_type = genomic DNA
gtctctactaaaaatacaaaaaattaaccgggcgtggtggcacacgcctgtaatctcagctactcaggaggctgaggcaggagagttgcttgaatccaggaagcagaagttgcagtgagctgagatggcgccactgcactccagcctgggtaacagagcaagactctgtctcaaaaaaaaaaaaaaaaaaaaaaaagacaaggtctcatcctttcctggttgggtcttgagaaatcacctctctgagccacacaagattccctccaaaaacagtcccacatctagagggcacagagccgtctctgcccttgcaccccttccacagtgattgtggactctgggatgaagggacagctgcacccatgcccccttctgcctgttctcacatccttccaatcctagaccacccctcaccctgttctcttgggaaccccagctgccctcagccccagaccccccgaaccatactcccactgggacctgggctgccttaatccgag

SEQ ID NO: 300 - DNA, 500 bp, Homo sapiens
  source 1..500: mol_type = genomic DNA
gatttgacaacagcatttttaagtctttgacggcttgaagttggcagcattttcttccgctctgatgtggtttgaacagaagcatgtttatctgttatttatgtaacagcctgatgaaaaaatggggcatgtgcttcccttctatttgtcttctgcattaacctcattttgaggtcaggtgaaaatgctataggtactgattgcagcacgttatcagcattattgcttaatgtgccatcaaccacaagtgcaagtgggctcaggatcatcgccgcggtcttcccaggaatcatttatctggggctaactccgaaaaaatcatttagaattgtgacatttaaaaataaagattaaaagttctgaaaggagcagaagtcatccacacagggccctcttggcaccataaatcaaagtttgttagagctgcaaattggaagagcataacacagaggtgcaaccctttgatgtggttatgcaactcactggtctccaccacttac

SEQ ID NO: 301 - DNA, 500 bp, Homo sapiens
  source 1..500: mol_type = genomic DNA
tagaccacttctatttttgagtactattctcacaacgtagactgtgattttttggcaaacaagcacaaaatccagggttaaaaaagataaaatgtatctagcataaagcatcttttaaatggaaatgccaagttctttataaatttgaaaaatttattcattacccggcttctaggggagccccttatttccattttttttgctggggctatctgtttcaccccactaggctttccaaatggctgtccacagatgctgagcctttggtcacctccgagtggtgtttggaaagagtactggggaactgggctgctttttggcctccttgcacacaattcaagtcagagcttttgatcttaaggtaatatagagcttggaaacaaaaaatctgcatttagtttggaatatctgaaaatgatagtggttaggaaaaaggatgttaggcatggtttgtgtgcaggctattataggtacttcctttccaaaaaggtgatatttag

SEQ ID NO: 302 - DNA, 500 bp, Homo sapiens
  source 1..500: mol_type = genomic DNA
attcaacataatttcctctttttgagttcaggatgattggttactccacatagaacatggagtggaaagctgtatctttgtgacttttatttagatagcacaaaatgagcctgatttttaaaatgtgaacattcaaacctggctaactaatgataaaaaagggagtttttcatagaactctacaactctcatttcctcaaaacaagaattaatgcattctttcacatgcggtcattacaggaagggggggtagccatttactgtaaatgcctttctgatgcaattctactacctctttcaaagacagaattcatccaagaagccttagtcacttcttcaagaaaaatgccaccgcgctgaatgtacacagactaaaccacatgcctaaggaaaaaagatgagctgattccaccattagaacacagttcgggagaaaagtggcagagagagagagctcatagcttgtcagagcagatcaagtagtatgtctgaaaatccgc

SEQ ID NO: 303 - DNA, 500 bp, Homo sapiens
  source 1..500: mol_type = genomic DNA
tttctccttcaggctccagagagccatccaaaggccagctgctttctttttgcccttccttcttccgattaaatagaacaaatcccacttcatacacatttctccctccatggaacctgctggctaatcagcaagtgcttcgtttcttcgggagccaggcttcaaaccccagaaccgcaaaagaacctgcctgcttgacttacctcgctggacaagagggcttagtattttggaataaaatgccttgtaactcttctgggagggagaaaataacctttcctttattccagataaatatagagcagtggaaatacaaagcaaagtaattatgtaataggttagccttctatagcatttttttgctagtcagtatacaaaatgtttgatataacgattatttaatgctaaaaattctgcaaagatatgtcccactaatttcattttttttcttttaatcaaagggctgagatcttgagaggttaaatagctcgttagagatc

SEQ ID NO: 304 - DNA, 500 bp, Homo sapiens
  source 1..500: mol_type = genomic DNA
acgcttggtgcccgcgctcctaggccaggggtgcgcaaggcgcggggcggggcgattgattccaggcgggtcccgcacacacctccctcccccaaccccactgccccagggacaggattccgacacattccttaacgactctctaagtctgggctggcggtcacagaggttggctggcgtttcctgcagaggccggtgacactctttccttccgccttcctccaaccccacccccagctccgcacacacccggcctcgccgcgaatccatccagagggtgtttgctctgcacttggattcctcaggaagcctccttgagctcccgcgggcgccgggcgcaccctccttccctcccgccccggcgcggggcgcggcgcctgctcgcgcactcagcacccgggctgcgcggcggaaacccctggcccgcctgcccgcctgcccgcctgcccgcagcaccctgccgcgcctcggcgtgggcctgcggaggggcgggggcgggg

SEQ ID NO: 305 - DNA, 500 bp, Homo sapiens
  source 1..500: mol_type = genomic DNA
tacacggccaccaccctgtccctgacaccctggatacacggccaccaccccgcccctgacgccctggatacacggccaccaccctgtccctgacgccctggatacacggccacctggatacacggccaccaccccgcccctgacgctctggatacagggccaccaccctgtccctgacgccctggatacacggccacctggatacacggccaccaccccgcccctgacgctctggatacacggccaccaccctgtccctgacgccctggatacacggccaccaccctgtccctgacgccctggatacacggccaccaccccgcccagactgaagggtgacaccagaggcaaaaagagtgaactagattcacgtaaatcaacatgaataaacttcaaaacagaacagatggaaagactggaaaagtccacgcactaatgttcattcaggcagaaagagtgagggtccctcccagaatccagtccagggagactccttctct

SEQ ID NO: 306 - DNA, 500 bp, Homo sapiens
  source 1..500: mol_type = genomic DNA
gcagtgagccgagattgtgccactgaactccagcctgggtgacagagtgagactctgtctcaaaaagaaaaaaaatgaagaagaagaagaaaactagaagcctaggttagggatttggctaaagccacatgtcagtgccaaaagagagaccagagcctgagtctcttgactctcagactggcacattaattaagtacctacacggtactcaagctcttgggacatctaggacgtctcagtgcatctgggatggggtgactcagccttccactgcccaggctaatcactctccagtgctagattgtgccattcataatgaagaggttgcaatttggaaccatgactttggggagaaaatgggctggaaaaacaacactggtctttgcggtcagctagacctgggtttgggagtatcacctgctagtatgccctcccataagctgcttgaatcactccaagcttcagtgtctcatgtcaagtgggagaggaatgtgtactcc

SEQ ID NO: 307 - DNA, 500 bp, Homo sapiens
  source 1..500: mol_type = genomic DNA
gaggtcttgattgatgaactttgaaatgtatcagcgacagggggaaaagatgtcaggcactcagcgagcgacggctggctattgataaaaccaatctctcgctcaaattcgtaattcatggccttctccttggagccccctcagagaaaaagttccctcttttggaggggctttgggggggcaaggcctaggaaaaaggcgagcgcagaggaaaaaaaatctatcatagaatatcgctgctagggtgttttttttctaattcactgattacagccgtatggggaccgcgctactattaaactattgaattcatggagacaaggttgaaattggaccgaattggctgtcacatgattgcttctgcccaatgacaatttgggctttaatcaaaagaagccactgtctgtttgattgatccaaaaaagtcgggaaggaacgcctcattgggggccagcgaggctttatttacacttttttcagagcaaaaatacatatatgtt

SEQ ID NO: 308 - DNA, 500 bp, Homo sapiens
  source 1..500: mol_type = genomic DNA
ggtgtgggtggggatgtcccggagtacgtgggggcgagggtgcctgcgtgcctcctgatctgcaaggatctatctagtgtgtgtgcctgggagtgtgtgtgtgtgtgtgtgaatgtgcgcgagtgtaagccctgctgtcggtcccgccggtggctgccctctgcctcccccgcacactccgcgcattgtttgggactgtcgggaagacgcctcgcacctcacaaatcatttaagcacctcagtctgacgcctgcagtcattaacaaagtaatccattaatcttcaaagttttgacacccgagggccctgcgtcccagccacataagttctgttaaagcaggagaaaggagcagaggaagagaggagatgagagagggagaataaagagagagggaagaagagagagtttgagagatggagaaagagaagacagaaaagagagaagaaaggaaagattttggttgggaaggggtcttccttttctttcccttttcctcctt

SEQ ID NO: 309 - DNA, 500 bp, Homo sapiens
  source 1..500: mol_type = genomic DNA
cacttttcctaaaagcagttcctggatctcaaaactgatctctctcggtctgttttccttcctgtctgtccctttccctctttttcctcttctccccctttctccctccctctctcttctgtccgcctccccttctcccctcagcctctcgcccccctcccagtgtccagcccagagtctgcgccccgggcccattgttagcaggctattccacggcagctttgcatctggctccggcgggaagcggaaaacgggaggcggctctcgaagcttcccgaccttcctgcgccatcaacttctcaggagtggctggagaaagatgcatgtgccaagcgagacaacaaccccaggtccatgtgtccaaatccccgtagccagggcggcggccagccaaagaaatgccgccccgagcaggcgcgtgcggctcctggcattctgggtttcatacccgtagggctcgggtgcggtgagtatttccgatttccaggaagtctgttgga

SEQ ID NO: 310 - DNA, 500 bp, Homo sapiens
  source 1..500: mol_type = genomic DNA
tgactctccccagttcagtcctccgtttgctggagacctgggtgagcctcagtccctttcaaactgtttcgctccgcgtgcagatttttggagcaattctttcctcctgacgcgataacagaccgcgaagcatccccggaggagaccaggagtccgattgctcccggaaagtgctcggcatcctctgcgcggctggctaataccgaggtttaggcgttagttggtccgctttgacccgaggaagagcatggagcagaagaccgccctgcgttatcccccggctgggccgcggggcacctgtgcgctcccgctgcgccttgggccgggatgtctttgtttcttccgtgcacagcactcggcagcccctgcgccctcagcctgcctccgcagcagctgggaaccgggcagcccagctggcccgccgcacggcgttaccagagctgccgcagccgcctggagccccagccgccatcctgagaattcgccgagcttccaggcga

SEQ ID NO: 311 - DNA, 500 bp, Homo sapiens
  source 1..500: mol_type = genomic DNA
atagcctggccaggccccatgctggagccagagggctgctgcgtccggcctgctctgccggctcgcctcggcctgaattccacgcagacccacgtcttcggccaaagaaccccttcttaacacggatattattcagaataaaaactttatttctttttgtttctcagaatgtgagcagcaaggaatgaagaactctcaaaacaaatctagtatttttcgcgtttacagattttttttttcagttttgccggatgttacaaacctaaatcactgttttcaaaagctggatcttctctggttttattgtatcgttaccgtttaaaggaattatatttctctttcaaataaaaaaaattctaagtacgccaatacacaattgaacaaaaggcccaagaacccttctgaaccatcagggtacagaattctttaatataaatacgaacggatggggataaataatatttaaaacttagattattcaatgcttgcaaaaaaatata

SEQ ID NO: 312 - DNA, 500 bp, Homo sapiens
  source 1..500: mol_type = genomic DNA
aataaatctgactgttcaccagcatacacacacggaaagacgtacacttagtcatccttgcacagagagcccctgtttcaaagcgcctttgattttttttctcactctttacaagaagtgcaattaaaaaaaaaatttaaaattaaaaaaagtaatcgcttcccctcgggagccataatgtaagaacaaattcacattgaaaactcgactagaaaatttgttcatataccctgtttctgatcaaagagtggagaaggtaaagggtgcagggccagtggcctatcgaggagcaggaagagataaatatcgctatgatacagccattccagcaaccaagattgctacgtcacataaactataaaaacgccttaccaacgaggggggaaaccgggaaacggagtgcggggcggagaagagagaaaaggaaggaaggaaagggcaggaagaacctaaaaaaaaaaaaaaaaaaaagcaaccaaagaaaaaaggtgggtgggggg

SEQ ID NO: 313 - DNA, 500 bp, Homo sapiens
  source 1..500: mol_type = genomic DNA
agactctcctggcgcgtagccccaagcccactatcacaggtgggtgagcttgggtgcttcctgaattcttccctgagaaggatggtggccggtaaggtccgtgtaggtggggtgcggctccccaggccccggcccgtggtggtggccgctgcccagcggcccggcacccccatagtccatggcgcccgaggcagcgtgggggaggtgagttagaccaaagagggctggcccggagttgctcatgggctccacatagctgccccccacgaagacggggcttccctgtatgtgtggggtcccatagctgccgttgccctgcaggccatgagcgtgcgggtcatagtcgggggtgccccctgcgcccgcccctgccgccgtgtagcgcttctgtgggggtggcgggggtgcgcagctgggcagggacgcagggtaggaggcggggggcagcccgtaggtaccctgggggggcttggagaagggcgggggcgactggggctcat

SEQ ID NO: 314 - DNA, 500 bp, Homo sapiens
  source 1..500: mol_type = genomic DNA
acgggacgctgttgaccagcgaatgcatagagttcagatagccaccggctccggggggcacggggctgcgacttggagactggccccccgatgacgttagcatgcccttgcccttctgatcctttttgtacttcatgcggcgattctggaaccagatcttgatctggcgctcagtgaggttcagcagattggccatctccacccggcgcggccggcacaggtagcggttgaagtggaactctttctccagctccaccagctgcgcgctcgtgtaggccgtgcgcgcgcgcttggacgaagcctgccccggcgggctcttgtcgccagcgcagctttcgcctgcgaggacagagagaggaagagcggcgtcaggggctgccgcggccccgcccagcccctgacccagcccggcccctccttccaccaggccccaaaggttcctgcatccgtcaggtcccagagagaagtaggaactaggtgctatcctctctcctggtggg

SEQ ID NO: 315 - DNA, 500 bp, Homo sapiens
  source 1..500: mol_type = genomic DNA
taaaacagtgatactccctcatttagccaaggagcaaatcacagccttctcgggggaaaggacagagaagtagaacccccggtttgccttcctggtctggattttctgtttagagctattaactttctgactcatttactggtccctttggcctatcggacaacagcctccctgtgggccggtctcagcatctccattctcttcacagtaactgaaatgtgggaaacctaatgtacacactcatttccctcccacactgtctgacaataattaggcagtagcttcaactggccacttttttctctctacccagaggagatgggcagactggaaacctcaaactggaaggccttctctgcccaaagaagagatcccattgaaggtatttctggtggggaggcctaggcccttcatgctaggtcctattctttagggttccctatgtcatcaagcagccagccccagcttttgtccactaatcttgtacccttctgtcttcc

SEQ ID NO: 316 - DNA, 500 bp, Homo sapiens
  source 1..500: mol_type = genomic DNA
attgttgataatggactcctttagatttcattattaagccaacaatcttaccaacatctgcaaaacaggcacaattaattttccagaacctcgattaaaaattacagcatcgcttatccagagttattgtcagtgatcatgagccctggagcattgtttctcttttggaaataggaagctacacataccatggttgaaagtaaataaaggataaagtaaaacttaaaactgaatagcaatttagtgtatccgtttccttttcttttactgaaaacagttcctattacatttggcagtgtcaatgtctgccattacaaattttttagataccaggcttgtgtaaaataaaatgtcaggttaagaaaattagacactcgaacagcaagatattagataaaacaaaattaagctgattttgcacatgcaatatttctagtgacttgctaatccattatcacgttataccagcctgctacttagttaagcctttttatcaagtt

SEQ ID NO: 317 - DNA, 500 bp, Homo sapiens
  source 1..500: mol_type = genomic DNA
ttgaaactaacattccttagaaaatccactgaaatggaaaacaatgttcactccacattcaaggacatttctggggaatgccaccaccacacgcccatcccctccatctccttcattttcaatgcattaggaattcttggattttggcaattcctgaaacaaacaaacaaaaaatctgataactcttatttagtgtaaaaaaaaatccaaaggcattttaaaaaacaggactaaatagctaattaaaatcacgtcatttcagaagaacttgttacattcatctaggaacattcatctagggctacagttatctgggccatgtcctggcaaactgtacactgtgagcagccactgtgggcaggagggtgaaaggaatttaagaatgattcatcacatcttctgctccaggagatgtggcaagccaattatctttgcagaacattaggtgcattttattattagagcgaatttttcagtcttggcttttaacatcctgtgtg

SEQ ID NO: 318 - DNA, 500 bp, Homo sapiens
  source 1..500: mol_type = genomic DNA
aaataaaataaaatgactttagacataatatgaaaaaaaacagttttacatgttccaatttctccctatatgttttcccatccattgtgcattttactgttgtccctaagggtttgaacatttgatttatatcacctctctggtccctctgagtctatccacagaccccaggttataataatataagcttgacttccttcaactccacccggttgggggcaagggtaaggcatggtacctgcagcctgactgctgttttgttttgttttgtgacagggtcttgctgtgtcgcccaagctggagtgcagtggtgtcaatcatggctcactgcagcctcaaacttctgggctcaagggatcctcctgcctcagcctcctaagtaggttgttgggactgcaggtgcataccataacacctaatttttaaatttttaatacaaatggggtttgatttttaaagtttaaaatttttttgtacaaacagggtcttgctttgttgcc

SEQ ID NO: 319 - DNA, 500 bp, Homo sapiens
  source 1..500: mol_type = genomic DNA
gtctttttgatagagaagaaaggaggaaaccagtcgatcaggcagttacagtggttgggtccttgattgaattctttcaaacaaaagaatagcctaaaaaatcaagtagcaggcacagataaggaaacttgcatggggggcttgcctaactatgcacatagccacacagataagaaaggcaatgcaggtgacttacccagacatgcttgcaatggaaaattctgtcccctgacacatgcactggaaggggaacaaagcactatggagtaacttaagctaagggcctgcatgtgcattaggaggatggggtggagctaccagaaatttgcaccttatgcaaatgagacgcccagccctaaacaggttcttatataagcctttgtattcatttgtaaaaccggcaaccctctttcggaccccctttctgcagcagagagctttcttctttggcttattaagcttttgctccaacctcaccctttgtgtccacattccttaat

SEQ ID NO: 320 - DNA, 500 bp, Homo sapiens
  source 1..500: mol_type = genomic DNA
ctctggggtggggctgccctccccaccagcaccccaagggctaaaaggttgaggggagaacaccatcatttgtacagggggatcctggaagatgaggcctgagaaagccctgcggggcccctcaccttctccctagctgtggccaagagtgtctggccttgcctgcctcaggaccagcccaaagtggaggtgagaggtgagccccagcccccaggggaagggtgatggtggtcttggtctcagcatggttctggtagaggtgggttattttgaagatgatgaaccttaagcctctttctgatcttgctttaaataaatacttctgaacaacagcaacaacagaatagtgttgataggaaagccctccactccaccagaaccacgcggccttctcgtcctcccctcctccacttccttcctaagtcactgctccatgagctcttccacaggagatttacaaaatagaacacaaacaatccagttcccgcctctcactctga

SEQ ID NO: 321 - DNA, 500 bp, Homo sapiens
  source 1..500: mol_type = genomic DNA
actcctcccaagactcgtggggtgcggcagcccctgggaacacccagcccttcaaggtcaaacacagcccccgcccctcactctggggtaccctgccagaataagccccgacagccatgtggagcagagccttcttttttgtaagtggaagttccaggctggcttttcaaatccccttttaacctcagtgctgtatttcaaaattcattccagttttcctgtagtaattaacaaaaataaatattttaatttcaattaaagtgagggtctcggagaagaagcaggaactgagtttcctgagaggccccgctgaggctttgttgatatttcttcctgcgacctctgctcggaccctgggagctcacaggccgtatcgcagctcttatctttggggaccagttaaagcataactgcgccaggcacagagttgtcctttcaaatgtgccggcagtgggacggagacccatgcgtcaagtctcctctaagttcacatgggattc

SEQ ID NO: 322 - DNA, 500 bp, Homo sapiens
  source 1..500: mol_type = genomic DNA
cccagcaattttttttttttcttgatacagagtcttgctctgttgcccaggctggagtgcagtggagcgatcttagctcactgcaacctctggctcccaggttcaaacaattctcctgcctcagcctcctgagtagctaagattacaggcacatgccaccacgcccagctaatttttgtatttttagtagagacggagtttcaccatattggtccggctggtcttgaactcctgatcttgtgatctgcccacctcagcctcccaaagtgctgggattacaggcgtgatgagccaccgtgccgggccaccagggcctaatcttgtttgtgtagtgtctctaattccttcattttgaccacagctcttacgcaccctgtatatagtaattatccatgagagggagagtttgggaaatgatacccttgtcaagttccctcttacattgtactaaggttggtctgtgtgatgattcatgtacggagaattgatggtatgtaact

SEQ ID NO: 323 - DNA, 500 bp, Homo sapiens
  source 1..500: mol_type = genomic DNA
taaactctcccattttctccagatatttgggattaagaactagattacttgctaaaatctttcaaagacctctttagccatgagaagcggcagtcagtcaatcacaagaaaaactgatttccaacaaacaaggcacaattgtgaacatcgccttatctttattgttttcaaacacctcattgaagagacaagttaaatgcactaaaacatcaagaaattctctctacttctgcttgcaagtaggtctggcattaacaaataagatcttaaaattgaaagtgacttccagtggatacagaactaactatgatttttgtaattaggtcatatttatgtggtcatatttgagaagatatttattttttcctgtgcaccttgataaataaaagacttaatctgtcatctatttaacttactgactcaggttaatgtttatagatactctctagctgtataacatttatgaacatatgataagaaaacattattatacatacctg

SEQ ID NO: 324 - DNA, 500 bp, Homo sapiens
  source 1..500: mol_type = genomic DNA
cgattttccaggtgccgtccgtcacccctttctttgattaggaaagggaactccctgacccctagcacttcccgagtgaggcaatgcctcgccctgcttcggctcgcgcacggtgcgcacccactgacctgcgcccactgtctggcgctccctagtgagatgaacccggtacctcagatggaaatgcagaaatcacccgtcttctgcgtcgctcaggctgattgctgcagaccggagctgttcctattcggccatcttgcctcctcccccggaattttcttaattgtaagtatttggagtcaaagtaaatttgatagacttacagttgtattttaaaaatattactcccatgttcatgtatctagtctaggggggagatgaatttggacatgtgacagtgacacagaggatggcctgttgttgcttaccaaatgctagggtatgcatgtgccagcacctaatagtgcctgtcacatgacaggtgttcagtatataactga

SEQ ID NO: 325 - DNA, 500 bp, Homo sapiens
  source 1..500: mol_type = genomic DNA
gctgtagatcggagctgttcctattcagccatcttggctcctccccaaattatatgttgattcttaagcatagtgttaatttgacaattttcagatcctaatagaagtctttttgaaaatctgaagtagtgtattagttaaatgttattctgcaattattcaaatgacattataattgagatacatactttagagctgttcacatatactaagccaattgtgaaagaaataaacatttgtccaattttattaaattgatggtagaatcatatatctagaaattattgtctacattaaaaggtggttgtgaatactataccctacaagatctttaaggctctccaaaaaaataccacatgggcagtttaacatttcaaaaataatatattgaactaagacaaatttgtgctgacatatgtaaactatcattcagaaactgtcaaacacaaaagttactatttgaggatacgaccattctttcttaactggaagctttctta

SEQ ID NO: 326 - DNA, 500 bp, Homo sapiens
  source 1..500: mol_type = genomic DNA
tgctgtgaaactattctgtatgatactgtaatggttaatacgtgttgttatacatttgtcaaaacctgtagacaaagagtgaactctaatgtaaaccatgaacttttgttcataatattatatcaacattgggtcttcaattgtaacaatgtactacataaatgcaagatgttaataatagaaaaacctgtctgctggagcagtaaggggatataggatctctctgtactttctgttcaatttttctgcaaacctaaaactgctctaaaaaataaagtctattaatttatttaacaacaacaaaaaaaagttccaggttctaagtagctccattagcttcactggtcagaaggaagggcctctctgaagagacaacctttatatctgacctgaaggacaagaatatgtttcccttgtgacatgcagataggaggatttctagtaaaaagagagctggaaaagggactctgcagtgaaaagctgcatgtgcctgaggaaca

SEQ ID NO: 327 - DNA, 500 bp, Homo sapiens
  source 1..500: mol_type = genomic DNA
cttcatttaatactttatactattggctgtacaagtttaaagcactaaaggatggagaatttaaatagatttattttgcctcaatactcaaatcctgcctcatattcatgacatgttttgaagaaaaatccaataattacttgtatgtggaacaacgccaagacggctttcactaggaaaacacaagtccagcctgaaagaattcatgaagtgcctgtgacctgacgttgaggatcacatgggactgtcgtcatcatgatctcgtccccaggctgccccggcggaactgtccggtcagcgtgactgtttggctttctgcagccatcagcaccgcacgggctcaccagcactttgctcctgagggcacagccggagcccctcctcactgcaggcagacgcagcctctgctgccacgaagccacacagccctgcgcttggcatgcggctgctttttctgtgccagctcacgagtgccaccggcacagtctgtgtcacctggc

SEQ ID NO: 328 - DNA, 500 bp, Homo sapiens
  source 1..500: mol_type = genomic DNA
taggtaaaagtgatttcatctcttaagatctgaatgtcgagaacttttttacaagttccatatacatgatacacagttgcagccaaccacaaattaaacaccataaaaaaagttaaaatgaaaacacagaacatacttaattttttattttgaaattccctattccctctatacaagaacctttgctgaaacagtttccacaaaggcagcagtgaattttcagaacatttacattttttccccctcagcaaaaagataaatcacagtgtaaattatgttgttctgctgtcatctttggctggggttagacccagaagttggtgactagcaaaccaatatagccaaatgttgctagtgctccttaggcctttaagctataaactcagcaaggaatgtctgcattttatctctttaaggtaccaccaggggggtatgacagcattaacttccataaacttttatagacaaatggaaaaaaatctacaaaatttgctagtaat

SEQ ID NO: 329 - DNA, 500 bp, Homo sapiens
  source 1..500: mol_type = genomic DNA
ggtttcttctttcttgttgctctgccttctctagggaataccctattccaccttgtcaaagatggagcaatgccacctctgcattccaatggaagaaatgggaggaagtggaagacacaaccttcccttttaagggcataacctggaagttgggctcatatttcaatggccagaatgtggtccaatggccatacccagttgcaaaagaatctgggaaatgtagtctgactggaaggtgactcatacagctaaaattcagggaagaaggcgagaatggataatggaaaacaaataggaatctctgtcacagtcagaagtcgaactgggattcaaacccaacagtttgacttcaaagccagaactcttaaccataatcttcattatgctgttgttttagaagaattaaatgaggtccacagttggtaaggtctttctctacagtttgagacttcattaacacatgtatgcacatacatttttgctaaatggatagattatag

SEQ ID NO: 330 - DNA, 500 bp, Homo sapiens
  source 1..500: mol_type = genomic DNA
tattattacaagttgcatttttccagtttttaaagtaactggcattttacatgtaatttaaaatgatttgtttcttaaagcagaaacttttctaaacaaaccattatgtagacattaaatcggtgagcctagaaatcaataatttatttttaagcaaatgagaaattattttgtgcttttatttgtacatttgcacatttatagttaaattgtaatttgcgatacagagggtattagttgtgaattgtggttttcagtatcacagacacatttgttgctgtggttttgcaatatcattccctgatgcttttctcaattgtggttttcataatcattgtttgatagtcatgtagctgtggtttggggctgctatatccatttggacagagataattgcttataggtttttccgtctatttattttataacctcagtgaattaaactagaaaaaaagaaaaactgaaccttaaatatcattaatattctcattaaaaataat

SEQ ID NO: 331 - DNA, 500 bp, Homo sapiens
  source 1..500: mol_type = genomic DNA
atttttttcttttaccaatgcatctctttatgattagtaaatgtgttgtgtgtgcagttttattgttattttcttcttcaagctgttgtctctagtaatgtgtttactgccttatatgtccccaactccagtcacactgaagtgtattggctatgggtgcaggaagaggtggacatcactttttttttttttttttgcaaatgaatgtcattatctgctctctagtagttaatatagagcttgaaaaggagaaactcaagtaatttatttttgtataagattaggaaaaggcactcttctttataccataaaagtagagttttcataaaacttttagattgcttgatcttttcagagcgtagtgcataaatgtttggtctagatcaggtgccaaataatttgtggtgaagtataatgaaagggtgaattaagaggcagaatgttttcttcttgaaaagtgaagcagatactggaaattagcatgcatgttgaaagtaaaa

SEQ ID NO: 332 - DNA, 500 bp, Homo sapiens
  source 1..500: mol_type = genomic DNA
aaaactcattgcaggctttgaatcccagcgacattcattccgcaacatactaaccacatcctggtgatcccagcttcagagaggagaacacggggacttgagttcactgttgcggtgaagtcctgctctggccccaggcagaagtcaagatcaaagctcacactgcaaatattgtgctgattaaaaccaaactttctgcttttgatgtgggccaacctccattgctggtaggaacaaaggaggagtatagcaaaaagatactagcagtaagtataaaaccaggatgcactcaatttaaaagacagagaaagaaaaaaagagagcgatgaggatgggggtagacagagaaaggaagaacgaaagaaagaatgaaagaaggaaggaaggaaagaaaggaaggaagtaaggagggagggaggaaggaaggaaggagggagggaaggagacaaggaaggaaggaaggaaggaaggaaggaaggaaggaaggaaggaaggaaaga

SEQ ID NO: 333 - DNA, 500 bp, Homo sapiens
  source 1..500: mol_type = genomic DNA
cagttaatttttgtatttttagtagagacagagtttcgtcatgttggccaggctggtcttgaactcctgaccttagataatccacctgccttggcctcccaaagtgctaggattagaagtgtgagtcaccgtgcccagtcaaaaactgaagtttaaagaggcttaataactttctctaaagggtggagtgcccaaccctacctgcctgactctgaatggctctggtcttgggattcctctgttcttaatcactccttcgacatcaatgaattatcaatgatgcgtacaaaacgctgtttgggagacaccaagaaggattagcaatgtgatgcctactatttttggagttgcaggaaaagctaatggcaggaccagccagtactagggagtcagaagagggtggctgcctgtagccaggagtcgagtagttcctctccccagtgaagaagggggaggtgtggaaggtgcaaaagttaatacaggaagaatagaggaagggc

SEQ ID NO: 334 - DNA, 500 bp, Homo sapiens
  source 1..500: mol_type = genomic DNA
cagaagcacccagatttcacaagaggaaatgatgaggcatttttctgaggtgttgaaattgtgccctttgtcagtcacaaaccaaccaaaaaaaaaaaaaaaggctttgaaaattcctcaaaggtaaaaggtagcctttcttctctcatagttctgatatagtcccaaaaggaaacaaaagcttgcataattctagccccagtgattcttctttccttcttattaactacaaatcttcaccacattttttcttactaattagtcacatgcttaagctcctgagtcacggagttgtctactggttatagcttgttctagctcttccaccctcaaatggaacttgcaaggaattaggccctctgaagatcgcacattcaagtcatgaaaacaagccaacaatgaaatcaatcactgccgagaagggtggacaagcacaagcattaagacccactactgttgagtcagggccttcagatatgctgccaatgggaagaagagag

SEQ ID NO: 335 - DNA, 500 bp, Homo sapiens
  source 1..500: mol_type = genomic DNA
accagccatctgtacatcaaaagcatttgccttcataccattgtcttactgtattcttagaacagtattccagaactcaaagcaacagagtctctgtgttcagactggttcttctcgtaaacaaaggaaaaaatggtcattaattttataggggcagaaagaaaagggacaaggacttcgggaactaaaggttctgtctacatggggatttatgatactattctctcaatgatagatctggaagtttgattcaccatgaaaaaaaaaccacacttttaaatgcttaattcctgttaaacttacaaagaaatttgacatgccaaataataaacaaagaattcaggaaccagagtggtgagaatgatgtgatttgagtgaagattttctaaaggcttaataggatttcttccctttctcttattttctgtaccacctaaattctaataacagaggacagttaactttctgttattagagctctaatccagtcacaaaaagag

SEQ ID NO: 336 - DNA, 500 bp, Homo sapiens
  source 1..500: mol_type = genomic DNA
aaaaaattaaagagagaaaagaagagaaaaagggaagggaagaaaaaagaaagagaaaggaggggaaggaagggaagggaggggagaggagaggagggaagcgagggagaggagaaggaaggggaggggtgagatggtgaggtgtggaggaaaagttaaatattaaatttgaactcaattgaacatcgacacaaacaatggtcaccaagtcccagaacaggttgtgtgtgccccttgaggcgttcatccagcactgtttcagagaaatccctatttcaatctattcctatacgttagttattgaaaagcaatagacaatcacaaaaaacaagttgacctttttgtgttccttgagccaaagggccctcatgactgggcctcacaccgaataactcgttacaaaaagagctagggtcccagactgcgccaaagcttcaggagactgctcctcgtctgtgcacagatgagtggccaactctggagcccaggttgttgcttcc

SEQ ID NO: 337 - DNA, 500 bp, Homo sapiens
  source 1..500: mol_type = genomic DNA
aatcccttaatttctaagatcgctcattgttctgttggaaacagagggttaggtaagtgtctaagacagagccagtgcacaagtgagtggtagagagagtgataaagcatctcctattttgaatgagatcttctgtctcttctcatacatatcccaatccacaacagcgaaaaagtaatacgtagattcattcattcagtgactcagcaaatagtaagtgccatgcattttccaaaacattaataatacaattgggagcaaagcagacaaatgtcccttgccctgatgggagaacacaggcattaaataaaataagtagatcaaaatatagtatatactaagtgatgagaattgttatgggaataagtaaagcaggtaaaaaggaatgaaggccctctgtgaaggaggatgctgtttaaaataaggcgaaggcaggcatcttgagacagttgcatttcaacaatggcctgaaggaagtgaagggcacctgagagaaacat

SEQ ID NO: 338 - DNA, 500 bp, Homo sapiens
  source 1..500: mol_type = genomic DNA
ataagcctaagcagagtgagttccagagagaaagggaaaaagatttaagagataatgagaaaaagcatctctttagagaagttttgctaagaaggggagcagggaaatgtggtatcaaggaaaggagttttgaagatgggaggaattacacacagacttcatttgcaaataaaaatattggtatgggagataaagagtgctttctgaggcaccatccttgagttggtaagagggaatgggttctggtacaaaaatgcagagaccggccttgcacacaaacatggattgttaattcacactgagagagaggtgagtatatagggcagatacaggcaaggtagacgtggtgcagggattgggagaaaattgccttctgctcccttctcttctctcagtgaaataggaaacaagatccagacactataggtcactgtgcagtcacatttttttggattcaaggtcctggaatgagtgagttggaaagatggagtgtggtggtt

SEQ ID NO: 339 - DNA, 500 bp, Homo sapiens
  source 1..500: mol_type = genomic DNA
agtggcacaggttataagggattttgctgatgactgatctggaattgtacaagggagggtgagggaattagaaagaggtgaagatggggtcagattaggtggtatacagagcagtattggggaagtatatgggagctaaaggatgagctgggtgtctggggcttttgtagtattttacggacgtggagatcaagggaggatcttctgcaagacaccagtggtgagattgtgaatgtcaggggagatagggtgtggggtctttcttggagcacccagggctctgaggcattctcttctccctcctgccaatggcagtatggaaagcaaggaagaaatagtgttactataaacaattaagcatgagccccctcctcattctagccaatgtttttgctttcttcattcattatacaaataccttttcagggcctcgtaaacctgaatactagaatataatagtgaggaaaatgtcagtttcttctctcatgtagccttcagag

SEQ ID NO: 340 - DNA, 500 bp, Homo sapiens
  source 1..500: mol_type = genomic DNA
ttttgcatactggcagcgacaagttgagacttgttcaacttgacacagtcctgtggtcatagcgaatctttctaaagctctgatcagtcaagaagggggttgtatcaatcctcagaaccctgagtggaactttctacaggatttattaggagaaaaaccttcccggaagctgcagaaggacaaatacagaatccgtgtctgggagaaacctcgtggcctggtctccattatttgagatgagttacatcttggaggtgaggacgtgcctcgtggtctaaagcttcggcacaagggcccaactggaattccacttacgggtatgactgtggggtatatgctgtacccattgaattcccagagggatttgttaagtggttgtgttgctgttttgcctggttaagagtggcttattcttgttgcctcatctatcttgagtgcagaatttttgcataaacggcttctcttgaaaaatagaagtccgtttttgttttgttttgttt

SEQ ID NO: 341 - DNA, 500 bp, Homo sapiens
  source 1..500: mol_type = genomic DNA
tttttctgattaactttccttttcctctgtcttaaacaccttcccccgcccctcgccacctccatgctgtgtttctgtggctggagcttttctgcactggaaaggaggagttctcccctctgttctgacatatctgatccccactagtttatatgattgctggtctgaaaacctggtgaattctcactgcccacatcaaatcaattccctgttctttagttgttttttttttccgcctcctgagcggtaggcaggcactctggctggattctggagcctgtgtttgccatgcctgggccttctgcctgcccaagatggacacgtttctctggcagctttgtcaagagatctcctggactataagacaccctgttctttcctcctgtttgtgtgagtggccctgcatttgggcagagtattggcagaatatctgggggaagtggaagactttggatagttgccggtccaggtcgtctggagaggcagtggcaggcctgctg

SEQ ID NO: 342 - DNA, 500 bp, Homo sapiens
  source 1..500: mol_type = genomic DNA
aagaggagttttaagcttctaatacagcaaaaatgatacagaggctaacgacagagcaggcccatacaaagcagccccctgaccatgcatctcacaccagccatctgtttgaaaacacttcacttgacatgtttccctcatttttgagaaacccccaaagtcactctcctgttacctaccatacattttgcaaagacagtgccatgccattaattagctattggttctagtaaatttaaacaatagaaacattgtctactttctcatccatagacaatgtgaactttgttcacataagcatatccatatttaaggggaagaatagaaaaaaaaggaggagaaaggagggaaagatacctaaagaacaagattccacctaaatataatatttaaagcatctacatcaaaatgcccttttccaattaatcaaaacttgcattctttgccacccccaattactgaggttggtttattcaaagcactggggtcgcatcgtgtca

SEQ ID NO: 343 - DNA, 500 bp, Homo sapiens
  source 1..500: mol_type = genomic DNA
cattctagtaattatgtgaattaggtccttctctattttattatttccatcttactgactaggatactgagtaccgaggcttcatgtggctaagtaccttgcccaggatctcgtggttaaatccaatgcttaaagttgtattgcaggaatctgacatccacatgctcaataaaaatgctgtcataagcagtcagtaactgatagaaataaaaatgtcacttttttgagttttcaaaggcaaagtaaataagaaacttctgagacatttagactttgagaaatctgttaggatgagcctgaatcgcagatgaaggtagtagaactctttattgtttgaatggagggcctactaattctgtttctgttcaaaacttagacactatttctataatttatagaaaaaaaccagactttcacaattgagtttaacgaaaatacttaacttggtgtaatttatttcatttaggtagttgtggtggtgggggaaatatcctattgtt

SEQ ID NO: 344 - DNA, 500 bp, Homo sapiens
  source 1..500: mol_type = genomic DNA
tagggtcagactaagactcttttcatattaaataatagaaaactagtagctacagctctatgttgtgtcttcctattctcccatgctatgtgttaccctgtccacagattataaatgacatttaacatttttctgttttggggacttctgttgcctagtcagctcaattaaatttcgtaaaaagttattgagcaattccaatatgccagatatttgccagtccatacaatataacaataaataaagcagaaactctagactgtagggttttctagctgattggaaagacacgaaaaagtatttaccctgtagattgatgaatttcataatagggttaaatatagatgggagcacagaagggaggaacttttgttagttcagggatcaaagaaaacttcctgaaggacagcatgccccagtgaagtgctaaaggacaaatagaccttatcagatgggtcaggatagagaatggtgtgggcaggagagcatcatgagccaag

SEQ ID NO: 345 - DNA, 500 bp, Homo sapiens
  source 1..500: mol_type = genomic DNA
acatcgagcaatatcttagagctaacggtggatgcaaggagaggctgcatgaaggccgtggaagagacagggaggtctgagtccttgaaataccattcagccgtgtgaacttggaccttctccccatcatctctaagcctcattctcctcacttgtaaaagagaaagtgagatttaataagctttccaccttattcctgttttagtaatcaccaattttattatacagctcactattagcggtctgacagccagtcatctctaaatctaatctctaatatgcaatatcctcatcttggaaatagggataacattaatgtccttgaaacattgacataagaattagatagaaaacgttcgtataccttgcacttgcttataacagggacccaacacatcatagccatagctgtaattagcaaaataaaggtcgataacggaaaactaaaatcagaaatgcaattcctcggggcatgagactccatcctaatgaatttcctg

SEQ ID NO: 346 - DNA, 500 bp, Homo sapiens
  source 1..500: mol_type = genomic DNA
ggtgctgactcaggggcctgggtgagccccttcggaagccagagcttctgcttccttgtctaaaaaagggaaaggtggtgcgtggagtgaaggagagggctgagctctgatcctggccagagagaaatgcccaatgaacagaggggtgtgaatcactggtgcctggctcccacacccaggagagctgagaaaggagttgtgggttaatccaggccatgcacttgcagcggctccagctcagctccgccttcagcacgctcaaagcgattggtaggacagcgggtgagtcggggtgggctgtgcacagagagctgagcctgaacacaggccaggtcgtcctagcaggggcaggacatgggctgctgaaggaaaccagtcctccttcaggcccagcaggctctgggatttgctgccctggctggagcctcccttggggacaaacagagcaggacagggaggcaaaggggaagccagggcctctggatggagcgggcagttgg

SEQ ID NO: 347 - DNA, 500 bp, Homo sapiens
  source 1..500: mol_type = genomic DNA
tgagcgccctgggtgctggtgcccgtggtccagagaaggacgtgactcacccaggatacccgcaggccccagagaaggacgtgactcacccaggatacccgcaggccccagagaaggacgtgactcacccaggatacccacaggcagggtccggcaggtggctggatgctggatgtctaacgcgggccccagcgccctcgtcgggccatgaggcctcctcgtccccacctggtttgctcctccctctgcccctccacccccacccctacccccggccccttcctcctgacccccctgcaccctggccccccattcctcaggaaccgcttcccatgcaaatgcattcagaacacatgacgtttcagaaacatctatttgtatatatttagactccatttcaaaagaattattcaaaatcggagccatttggatagatgggtgtggaacggattgtttcttaaatgttcacatcaaaaataccatgttttctaagtggatta

SEQ ID NO: 348 - DNA, 500 bp, Homo sapiens
  source 1..500: mol_type = genomic DNA
tggcacatcctgaaatctcacttaatcctcttgtcactcatgggctctaaaagttgcacagcaagttcagccacattctataactgtgtgagctggttcattgactctattcatttatcaccaagaatccacaatagcagggaaatctacagaacactagtggagcccactcagtcaggagaatccaggaagcctcctaggggaagggctgtgagggatgagtgggagtggagcaggggagcagacatggaaagagaattccaggctgagtagcggggaggacccagcctgggaagttgtctcaacatgaggttggaaagaccagttctagaaagaaataggctaaataagagtgaaggcaggccaggcacggtgactcatgcctgtaatcgcagaactttagcaggctgacacaggaggattgcttgagcccaggaattccagatcagcctggccaacatagcaagaccctgtgtctacaaaaattttttaaattagct

SEQ ID NO: 349 - DNA, 500 bp, Homo sapiens
  source 1..500: mol_type = genomic DNA
tagaataaaaaagacaacagtaactgttggcaaggacatggagaaattggatccctcaaatattaccatgtgaaatggtgcaattgccttgtaaaacagtttgggagttcctcaaaatgttaaaactcaagttaccatatgactcagcagttctactccgaggtttctacttgagagaaacacaaatatatgttcgcacgtacttgcacaggaatgtgcatagcagcatgattcatgcagccaaaatgtggaaacaacccgaatgtctatctgctgatgaatggacaaacgaaatgtgatgtgtctatccaaacaatgagatattattcaactggaaaaagaaatgaagtgccgatacatgctacggcatgggctaagtgcaaaaacattacgccaagtgaaaggagacagccagcaaagatcacatacggtatgctccacaacaggcaaatctatagagacaggaagcggattcgtgcttgcctagggccggtagagtg

SEQ ID NO: 350 - DNA, 500 bp, Homo sapiens
  source 1..500: mol_type = genomic DNA
ataaaagaaattatctttcatttgagggtaccagcaacccgctctccagctctaatcctcttcatcctccttctttttttttttttttttttggttgttaaaacctgagctgctgccaagctgatcttaatagcatgttcacaaagacagatggatttttttcctaccttcattagccactgagtgttgttttccatgatgttctccagcacttgcagcctctgcaccgagtcatcgtattcgagcggcgcgtccctctgcacagcattggacacgtaggggctggaggaagagcggcagttgtccatctctggcaggaggaaagtgtagctgcaggacccatgctggacctgatattgcttctttcctatgctgtccatgctcttccgaaagttgttataggctgcggccaagacaagatcacagctcagagtaaagaaaacaatctgccacattctttcttcagtaataaaccagcagcttagcaaacttgagggcaa

SEQ ID NO: 351 - DNA, 500 bp, Homo sapiens
  source 1..500: mol_type = genomic DNA
atttttttattaggaggatggttgcatctcaaatctcctgttaacagaggtgtttagagatgagaatttaaatttaaacataaaaatgtttcatggcctaacctcattttatacatttatcctgctctggcaattactgaagaacttggtgcaaggatttctctgttacatatccttacccactttttgaaaagagataaacaatctctgattatgagagagactcagtttttgtacctaactagtcaaaataataaatcatgcattgtccaatcaagtaagtacagctacatttgccatgtgcagtctatttctgcagtagtactatggtcaaaattcagatgccaggctgactgagtcggtgctctccatctaagattttgatgaaaggaaatgattttcctaagcaggcctccacagaaatgtgaagagttgggaaagaagaaaggatatctatctattaaatgcctgatgtatcaggaagcagggtcagttaatac

SEQ ID NO: 352 - DNA, 500 bp, Homo sapiens
  source 1..500: mol_type = genomic DNA
gtaaataattaacaataaacaattaacagtaaacagtatcaagcacttttcaaaaaacacagcacagccattgggcatttttttatcctgaaaagaaaatacacattattattcacatgatcattgctaattctggaaggttctgcaaatctagaataaagttgaaaacaaaagataattatttcacagtttatctatttagtgacataatttatcccagttggtaaataaacaataatgagctgactagttcaaatgaacagaacaccttctagccaacttctcacggagtctcaggccagtccctgtaaaatgttagtgactcacaccagtgtctctgagaaaagcccagtgtcccaggaaaatactgtacgtagggttactaaaaacccacatttcattttcatcaccaccattctgtagtatatgctttatttacaatttattttagttttatgaacaaatagaatactgtccaaatattacccagctttattcat

SEQ ID NO: 353 - DNA, 500 bp, Homo sapiens
  source 1..500: mol_type = genomic DNA
ggcctacggagcagttaccttctacggcaatttcaagggtggatggtgcgagcgccgctggggcagctggcgttctggttcttactccgtgggaaaatggccctgagcccgactggcttgaggcttagacaggtgaccccgcgaagcgggtgggcaggcgcggccgaggggcgggaggcgggcagcctccgtgattggccggcggagggggcggtgtagcgacccgaggagggaagaggactccaagcgccatggccgctgccgcccgagcccgggtcgcgtacttgctgaggcaactgcaacgcgcagcgtgagtgcggggccggcgggcgggcaggggaccgcagggtgcccacgcagccccctgggtgtgacccgctcagatcctgcgcagtcttctccgcttactttcaagaattcggagaatttggataccgccctgggctcccaccgcgcgccaggcggaacagcgaggtcacagagtgcgcgatgcagcctct

SEQ ID NO: 354 - DNA, 500 bp, Homo sapiens
  source 1..500: mol_type = genomic DNA
acctgtgacagagcctgccgagatgacagactcatgtgagtggacagagaaaaggaagacccagggctggcttcatggatgcacatcctgtgcagtggcccagggttctgagctgagaaggatgcccagcttgttttaatgctctgctattgccatcttgaaattcttgccaattttatctttgaccttgtgttttgcaaatgaagtctgatgggacggtggacatgagcagagcagatacatgaaagaaaaaagctttatatttcagtacctttaatagcattcccccacagccccctgctttttgaacaagaaacctcacatttttattttgcactgggcctggaaaattgtgtaggccatttaactgtgggtcagtggcaatgaggcaggatgaccatataatttactgtctaaactgggacacttctgagggtgaaagggagtgctattaataatgacactgggaaacagatggaaactgggattgttcctggcaa

SEQ ID NO: 355 - DNA, 500 bp, Homo sapiens
  source 1..500: mol_type = genomic DNA
ccgccgggaaaggatggcgttttaatagacaggcagcaagttcaccgaggctgaagaatgaagccccttcagggccggcgggtcttgagatcaatgagcccaataagaaaaccaagcagggtcatgactcagaaattaaagaacacggggtcaggagaagaggtcagccacgacacaggcagcggcccgtctcctcccgatcctccaaaggcgcccttctcctagcctcctccgacctcagggatctgcaacttgggattcaaagcccccgagagggcagaacgaccatccaaaacgaactgcgccagcgagtgctgccgccctccccaacggccctggaagaccaccgccccgggccccaggcgcgtcctgtcccgtgcctacctccgacaccacctccaagagcgccaccgcggagcgggcgcctcctggacgctgcggggccactcgggctcggtaggccactcgggctcggtagacttcgggcgggccctgagggc

SEQ ID NO: 356 - DNA, 500 bp, Homo sapiens
  source 1..500: mol_type = genomic DNA
gaaagtcccctggagctgctgagttccttcaagatttggtaagtctgcagatgaggcctgcgggtggagcgggcgcctaagctgcggatcactcctgcgggcgctcgctctctccacgccgccgcccgcgcgcccgcggcagccacgagcgtcccgggcggggaaacgcgttgcctcccggcggcgcctattactagcagctgcttctgcttagcccttcgaggatcggtttgccccaacccacggcctctcccagggttcggtcttctcccgcccctccctcccttccccgcctctcccccaagctcctcagtggccgcggcccgtcaacactgtcgcgcagtcactggcgcaggttcccagctctcagctgggggtttcggggggagggagcagaaggaatgagacagaaggaacgggaggctttaagcccaccgagggaggttagaggaaggcgctgtggctgtgggattaggaggccacagacgggaaccgcgccg

SEQ ID NO: 357 - DNA, 500 bp, Homo sapiens
  source 1..500: mol_type = genomic DNA
ttcttatttttttctaagtttaccttcagtcaatcccttacagccatttttcagggtagaaggattctttacatactcctgtcaatcactcctgacccctatgaaatgatatgattgtttttttctgtctttttattcctcagttttaatttgcatttctcctgaatatattacttccctttagtattgcagcctttgcttcttcagtcctccctaatcctcaggatcaggaggaaaacacaacccaccctctactcccactttcagacctttggccgcaccatatctcaaatgctttaactctgttggtatttataaaacatctgcttaacacgtatcttcataattgcttactcttaatctttaaatgaatttatttggagacttcagaaaaaatatttgactactgatgcagttaacttaatggttagatgtctatttaggattactgtatcttattagatcagtttttgaaagttatactttcataactaattgtc

SEQ ID NO: 358 - DNA, 500 bp, Homo sapiens
  source 1..500: mol_type = genomic DNA
ttgagtccatcagctggtgagtcaactccgcaatcgcatcctcacattcctgctgcatgagctggcagaagccagtagaacatgtgctcattccaaaggaaacacaaactcactgccttcagcctcccagaatcatcagtcttacagaattgaacaagtagagaaggtggccaaagtgaatttgagttgcccatattcttctatcactctctttctctacaggatggtgactttacgtttgtcttacattttacttttcttgagataaagcttatacatatatatgcctcttaatgaatgcagaattatttcttatgcagtgggtttttctccatccatctgtaagctgtctctgatactgagtgctgggctggatgacgtgatgccagctctatcacatgcccaagttaagcctgaaggctctgctcttatgtaaaatgagcactactggattagtgtccctgttagatgtgataagaggaaatagaaaaatgagaaca

SEQ ID NO: 359 - DNA, 500 bp, Homo sapiens
  source 1..500: mol_type = genomic DNA
atcacaacccattaagcaagaggagaaaaagcctgagtgtaggatctttagaatgaagccacagcaggagcagcaaaggttggtttaattatgttaaaagcaaccctaagaccggaaaaagcttttaacattcctagcacataaaaatagttggtcttgatgttttgctgctgagcaattggggaaatgagtgtttctattgtggccaaaagcctgcatatttcttttatgactcatctcatgtctgaattatgaaagtttggcatgcggaagggcatgaaagcctcacatcttcatttccagttaacccctgtcagtataaagttgggctgcactttaggatgaaatcgtgtgacaattcaactcagagtatattttctaggactgtttggtatttggaataaggaatgatttctcatctctaaatgttttctaaaagtagacataggctgggcgtggtggctcacgcctgtaatcccagcacttttggaggctgaggc

SEQ ID NO: 360 - DNA, 500 bp, Homo sapiens
  source 1..500: mol_type = genomic DNA
ggcttgcttgcttgctttttttttttttttttttttttgagagacagggtctcactatgttgcctgggctgggctcaggtaatctccctgtcttggcctctcaaagtgctggcattatgggtgtgagccactgtgcccagcatgaagggtattttaaataaaggaaatcacttttaaaaaaaaagttctcctaaaacccttttattaaaaataaaaactctgaagtgggtagtcactcttcacttgatcattttcataaatctaggttttttaaatcattgtctaaagtggggtagagtctaggaaaatcaaatttcagtcaatcccttcagttctctctttcactgtgtttaatgagaatgagaaaaataaggcattttctctttttggtttccttttttgttttcctccttctccctcttctaacagtgaaaaggcagcagaaacaaggaagacgataaattcaaggctttgataaaccacactgcaagttagcacgc

SEQ ID NO: 361 - DNA, 500 bp, Homo sapiens
  source 1..500: mol_type = genomic DNA
cctgccacacgtcgaagacttcccagccggccggcggcgccccctgcgggtccagggtccgcgcgtccagcagtaggggcgaaaggcaagggaagagctgcacgtggagcggcccggctggtggcccccagggcgctgagggcgcctggcgaaagagccgcagctccgcgcccaccagctcttctttgtctgagagcatggacacatcaaacaaatacttctgtctccggagaggagtgtgcgagagatcgtctgcgagataaaaaataattacagtcagtttcacttaagggggagatcagcccggtgctcttcggccgccccgggaggaaaagggcggggagtgggggcaggtcggccgggcagtccagcttgcccggcccagggcctgaccaccccggctccccatctggctggtgcatggcgcggggaagggggcgcgccaggacgggccccctccttcgcgtcagctccggactctcagggcggaagtcggtggc

SEQ ID NO: 362 - DNA, 500 bp, Homo sapiens
  source 1..500: mol_type = genomic DNA
tacctgctggtggggatccagttgtcctgtgaggaatgccatctgggtttagattctcactagattgtccttcttccattgccaaaaatcaaactaaaagattttgcccatccttttcttcttcccaaggcagaagggtgcattgcagaatctccaaaccactgaattcttttcgtggactagaggccaaaataaagtcttagagaaaagccagaagtaatgaagaagaatctttgctaaaaccaatctactcttatttaacttttttagtcaactgtgacagtactatcattttcattctaatcatttggatttaaatcttgaagaagccctggactcattcatctttgttggtttccacgtccagtctgcctctaagtccagctgtgcattcattctgcagatatttatttcatacctactaggtgcttgaggtaaagcagtgagcaaaccaggcagatatccccctgccttcttggagcttgcattctagtgatctt

SEQ ID NO: 363 - DNA, 500 bp, Homo sapiens
  source 1..500: mol_type = genomic DNA
aaggaacaaaggcatgaagctctgggatcatggctgggccaagttactgacagtactatttgcatagttctggtcactttccaaattacctctcactcagcctcaccacagcccttatccacagagccacctggggtggaatgggaggggcttttcttatccccatccaacagatgaggagactgtgactcagagaggtgaatgacttgggcaaagtctaacaacagtaaccacagagtaatgatttctaagctactaattaactttctaaccatctacccataaggaattggcctgtaggttgaaaaggcattcctgagtctctgtataccacacaccaaggattaatattccaagtaatcattttagaatttaaaagtgcaatagttaaaataaagaaaataagatactggacacgtctattaaagaaaaacatcagaataaacacatcagaagactgactcattgggcgtggggatcagattccttctaaaagtcat

SEQ ID NO: 364 - DNA, 500 bp, Homo sapiens
  source 1..500: mol_type = genomic DNA
ttcgagagagtgagtcgggaaagaaggggagtgggcaaagggtgagatgtggggtcccggtccccgcctcgctggctgccagttccctctgcgtttcctagtccgcgtgcgtgacacgagatagtgcagccctggcatggggcttggcatctggcggccgcgagataaccagggcccgtgcgatgggaaacgtgccgttggcagcccgccacccctccatcgtgacctcagtctgccaaacagggttcgtgatgctcagtttactagggaggagccgcggctttgagatctcgcccagcccgaagcagcggagactggccaggagcccggctgtcagacctcggagcgcacgctgcgggcgggggctcggtccacgggggagggtcaggggacgcgggactcacccttgaaggagtcggggagccgctgggcttcggagtcccgtgtgtgccgcttctcggccatgctgcccgagacgcagtcgcactcccccgtcctcg

SEQ ID NO: 365 - DNA, 500 bp, Homo sapiens
  source 1..500: mol_type = genomic DNA
gctgagcgccggcaggttggaccagcgctgcgcgccggaagtgcactcgggacgccggggttctggaggagagaccacacgccgcaaaagtggcctccgaatgcgcccggggcctgccctcggcgacactgctggctcggcggccgcagcctacctgaagtagtccatcttgcagaagatctccttgttcttgatgtagcagctgttctgctgcctcagcgacgtgcgacacacggagcactcgaggcaccgcacgtgccagatgaggttgttgacctggggacggggcggggacggaggtcggctcagcgcgggcctctttcactccgggccccagccttcccggtctcatttacagtcagaggcgctgaagctcagaaggtgcatgcgattcccctatttttctcccgtaatactgagactcagggaaatggaaataaactcttcttatttttcagacggaacccgggggctcaggcagaccctaagtcttgcccaaa

SEQ ID NO: 366 - DNA, 500 bp, Homo sapiens
  source 1..500: mol_type = genomic DNA
tggaagttacaaatatggaaccataactgccctgtcccctggtgactctaacgagtgaccaagtttatcaaaaattggtgtattaatgcagatatagctttgtagcataatatctcacagctgtgttgaacttacaagttgtggcctagaaccccattgccactgtggtggattgggttgcagggtagattcctgggtggattcctggctgccagggcttggggcaagggctgcattgtaaaggaggtctgtctgaaggtcctggtggtagcagccttctaaaagggtatgttttcaaggtggtgttttgtctctaccagagctccttaccacatctgtctgtcagtatgtccagttcccagcctatggagttgaaggcgcagcagtgtctcagaggctggtctaaatgtcagaactgtttttgtcattagttttagcatggagcagcatcaaggggaaactgctgttcttagaatgtgctgaaaatgggcacagcctgt

SEQ ID NO: 367 - DNA, 500 bp, Homo sapiens
  source 1..500: mol_type = genomic DNA
aaatgctgactccaggaatgcggaggaggaggaggactgcatagctcatcactgggggccacttgactggagcagctgtgctgcaaaccatcacctctcttccaccttttttgcatattcctcttgtaccaattttgaacaggaaatagtattttgtaaagtaagtgtactggcaaactaggcccaagtcagatctttgtggcttgagttctactttgtggcaatttcatgaagtcatgctcttttattgctgaatggaaggggatttaggaatcatcttgtcctgggatcctcaggaggaaggcatgtttagtttgaaaaagtatattcggtattattactttaacaagtggggaaattgaggccccaaggagaatgagacttgaccagggcagcatatctagaaagtaactgccaagacctgggaaccttggttctccttccacattttaaatcccttgtgggatttagacgctatacagaatgtcagagagaagaca

SEQ ID NO: 368 - DNA, 500 bp, Homo sapiens
  source 1..500: mol_type = genomic DNA
ggatttgttccacttctttgcagcgattaaacagtcagtttgaactggggaaagtatttgacctttagtctgtcctaaaagaatgtcatcaggctgtttatacattaaaaggctctcataagatatgtactcccagattcataattttggaacttctctcctatggtacacacccttgtatgtatgcacacctggctctcactgagtcacttatgggaaactgaagcaagtttttctattaataggggaaaaaagacctcataaaagagtcaaagtaaatgagacttagagaaatgtagaagcatgactatgcatcactgggcctttgcttagtttttattcatcagccatggagaagaaaggcatgactctttcctgcctcccacacccaccggacttgtaaagctcgacttcgatgatgcattataaagtggtgcacaggattggtttttaatgagatttttgccattggagcaaagcaagactgtttccctgccagc

SEQ ID NO: 369 - DNA, 500 bp, Homo sapiens
  source 1..500: mol_type = genomic DNA
ccagacgttaaagagatttgtgaagagtaaaacaatattactctctttactcaaaaatttttttgttttgggaaatgtagttatttttcataaaaaaagttattttgttagcatgtaatgggcttattactttctcaattaataaatatttttaaattttcctagttttaatttctaatattgttagctgttgctagatatgacccacatacacaaaagatcaggattttcagtaatttttaagaatatgaaggggttctgaaaccacagaaaatttgaggagcactgactgttgttcatctgtcttatttaaatcttacagcatcctaattccgttttcctactttaattgtcttcatagaacttatccttatctgacattatgtcatatatttatttgcgttttatctgttttctccataagccagttatttgcctacttgctctcagatccgttctctatctttcctcagcaaaacgtgtttcccaggctcctttgc

SEQ ID NO: 370 - DNA, 500 bp, Homo sapiens
  source 1..500: mol_type = genomic DNA
gacagccggagtgcgcaacccgcacttctacacgcgcgcgccgggcaacatagcgcaccgcgggtacacgcacgccgaccggacacacgcagtctcgtacacgcccaacgagcgcacacacccgcactccatgcacgcgcgatgggcgcacacactcgcatccctacacgtgcacacacccgcgctccaattaccgcgctagcgcgcaaaagagccgcaacttccgagtgggactcggcatgcgggggcagtgcccggtacttcaccatcagtcaccttcgcgtccgcctcctcccctgctggttgcacctccagccgcagagatttccggctggggcaccagaactgtccaggccgaaagagctgctcctccgtcacaaagcgcagttgcacactgtactgcaggcgcgcggggacccgggccggagccggggtcgcagccatggtccaagcgcctctgctcctgagccctagcagtgcctcccccgcgctgctctggg

SEQ ID NO: 371 - DNA, 500 bp, Homo sapiens
  source 1..500: mol_type = genomic DNA
acacctataatcccagcgctttgggaggccaaggcaggtgaatcacttgagctctggagttcgagaccagcctaggcaacatggcaaaaccccatctctacaaaaaatacaaaaattagtcaggcatggcggtgtgcacctgtggtcccagcaactcgggagactgaagtgggagaatcgcttagcccgagaggtcgaggctgcagtgagccgtgatcactgcactccagcctgggtgacagagcaaaaaccctgtctcaaaaagaaaaagaaaaaaaaatatatcagctatattcttaaacatgaaaaagactagtaggaaatatgccggtatgtttcttttgggtgataggaatttgggtgtgcttttatatctctttcaacttttcaaattattttcaatgagcctgcattactttttacttttaaaatgaaggaagagattatcccccctcaaaaggcaaaagcaaagacccatacccctatccctatccccaaca

SEQ ID NO: 372 - DNA, 500 bp, Homo sapiens
  source 1..500: mol_type = genomic DNA
atgcaaaacctttttttcctccagatccctaactgagacacatcagttaagaagcatagacttggacacttcgtgaatattatgtgaaatactgattaattagtgtaacgcatctgcataaataagcctgtcctttccctctgtacatgatccaggaaaatttctccttcttactgctcgtgagtggcacacttcgtgatgcatctctgtttataaacatttgtaatgtggttgtgcttttgtgttttgtatagctccacagagaaaaggaacataaatgtgacaatagtggatgaactaaaaagcttgacattgtcttgagtggaaattggtacctttcccacttctctttggaagtccagagcatgccagttacgtgttcattatatgtttacttccattccttgggagtaaatagctacttaaagtgatggcctccactccccacgcccccaagcccccaggagggccaagaaaggaaaaaagaccagcaaagttaa

SEQ ID NO: 373 - DNA, 500 bp, Homo sapiens
  source 1..500: mol_type = genomic DNA
caagatgtccttcaataggagaatggataaacatactgtaatatatccatacaggtggaatattatttagtaataaaatgaatgagccaagaaaccatgcaaagatatgcatgaatattaaataaatatttctaactgaaagaagccagcctgaaggctatactgtatgattctatttatgtgacattctgaaaaaggcaaaattgtagagataacaaataaatcatgattgtcaggggcttgtgatgagatcggggcagttgaataggtgaatacaggggaattttcagggcagcaaaactgttctgaatgatattgcaatggtggatatatgatgctattttttcaaaatccacagaactttatattacaaagagtgagtcttaatgtacacaaatttaaaaaatcatttgaggtcagtggatcccaagatgaaatacagaatgtgaaatgaagaattgaactgtgatatcgtttggctctgttgacctaaaagttat

SEQ ID NO: 374 - DNA, 500 bp, Homo sapiens
  source 1..500: mol_type = genomic DNA
tctcattagtactttgtgggtgtcaagactttcgttaaaattccacttcctttaatgtggtcaccttggcatgctttttgaatgagtttagtggcttagggaggattggtttttccaaatactaggcaagaatgcagaaagtaattggatttggtatacttcgtagcatttcatcggattgctttgagaagagctcttaaagaaaggctttatttaaatcagaacaaagagggagattcagctggaggcactgatgagcttctatgggattctatgactaatgctgcatgtctataccaggcttccatgtagacggatattatgacattagtgtgtgtaaactccacagtgctgagggaggaggggaagatggtcaccccactccatttaagaaagtttgtaggaatgtagtgagaatccaggaggctgaatggattttatgttgcttcatgaacaagtgagcagaaaacttcagtttttgggtgattttgtatctcaga

SEQ ID NO: 375 - DNA, 500 bp, Homo sapiens
  source 1..500: mol_type = genomic DNA
acttagtgaccaaagggaaaggaagagtgacgatgaccttggtttaatttttattttcatttattttaatttttaaactgacaagaatcgtgtatatttattgtgtacaacatgctgttttgaaatatgtgtacattgtggaatggctaaattgagctaattaacatatgcactacctcacaaattaatttttgtggaatctaaaaaggttgaactaatggaagtagagagcacaatggtggctaccagggcaagggctggggggagttggggagatattggtcaaaagtacaaagtttcagttaggaggagtagttcaagagatctgttgtacaacataatgactagagttaacaacaatgtattggattttcgaaaatcaggaaaagagtagattttaagtgaccttggggtttccgatgggtttttctagttgggtggtgacacagcattcctgagagaggaagtagaaaaagaggggcaagtctgagggaaaaatg

SEQ ID NO: 376 - DNA, 500 bp, Homo sapiens
  source 1..500: mol_type = genomic DNA
atagcctatttttcctatgtcctggattttttcatttttagttgtatattatcattgtagtcataattattacattattatttgtatgaagataacctaggatgagtatgatacacttccacattaacttctttcttgttattgtttggtaatgtgtaagacaaatctgtagtgatcagaatattctaaccattggcaaaatctgaaaaagtaatagcaacgatgagtctttcagttactggtaactagaaaagtcaaatttatttcatttttgggtggcaggggtttcttggagtacttgacatctgtgatatggtgaagtggtctcattgtgtggggtaacacctgaggtttgttgtctcatggccacggagattaaggacatggacacccaaagggtgaggtttagagcagaaatttaataggtaagagaaagaaaatatctttctgctacagacaggggtcccagaaaaaagggttgcctttttacagtttggata

SEQ ID NO: 377 - RNA, 20 nt, synthetic construct
  source 1..20: mol_type = other RNA
tgagtcacggagttgtctac

SEQ ID NO: 378 - RNA, 20 nt, synthetic construct
  source 1..20: mol_type = other RNA
gaaggaaagaagaatcactg